European Patent Specification EP 4 232 463 B1, published September 3, 2025. Title: INTERLEUKIN-2-FC FUSION PROTEINS AND METHODS OF USE. Applicant: GILEAD SCIENCES, INC. The sequence listing filed with the application follows.

SEQUENCE LISTING (265 sequences)

SEQ ID NO: 1 - protein, 128 aa, Artificial Sequence
  source: /note="Description of Artificial Sequence: Synthetic polypeptide"
  VARIANT (33)..(33): /replace="S" or "G" or "A"
  VARIANT (36)..(36): /replace="G" or "A"
  VARIANT (37)..(37): /replace="G" or "A"
  VARIANT (40)..(40): /replace="G" or "A"
  VARIANT (56)..(56): /replace="G" or "A"
  VARIANT (57)..(57): /replace="G" or "A"
  VARIANT (63)..(63): /replace="G" or "A"
  VARIANT (67)..(67): /replace="G" or "A"
  VARIANT (69)..(69): /replace="G" or "A"
  VARIANT (102)..(102): /replace="G" or "A"
  SITE (1)..(128): /note="Variant residues given in the sequence have no preference with respect to those in the annotations for variant positions"
STKKTQLQLEHLLLDLQMILNGINNYKNPKLTRMLTFKFYMPKKATELKHLQCLEEELKPLEEVLNLAQSKNFHLRPRDLISNINVIVLELKGSETTFMCEYADETATIVEFLNRWITFSQSIISTLT

SEQ ID NO: 2 - protein, 128 aa, Artificial Sequence; identical to SEQ ID NO: 1
  source: /note="Description of Artificial Sequence: Synthetic polypeptide"
  VARIANT (33)..(33): /replace="S" or "G" or "A"
  VARIANT (37)..(37): /replace="G" or "A"
  VARIANT (40)..(40): /replace="G" or "A"
  VARIANT (56)..(56): /replace="G" or "A"
  VARIANT (57)..(57): /replace="G" or "A"
  VARIANT (67)..(67): /replace="G" or "A"
  SITE (1)..(128): /note="Variant residues given in the sequence have no preference with respect to those in the annotations for variant positions"

SEQ ID NO: 3 - protein, 128 aa, Artificial Sequence; identical to SEQ ID NO: 1
  source: /note="Description of Artificial Sequence: Synthetic polypeptide"
  VARIANT (33)..(33): /replace="S" or "G" or "A"
  VARIANT (37)..(37): /replace="G" or "A"
  VARIANT (40)..(40): /replace="G" or "A"
  VARIANT (56)..(56): /replace="G" or "A"
  VARIANT (57)..(57): /replace="G" or "A"
  SITE (1)..(128): /note="Variant residues given in the sequence have no preference with respect to those in the annotations for variant positions"

SEQ ID NO: 4 - protein, 128 aa, Artificial Sequence; identical to SEQ ID NO: 1
  source: /note="Description of Artificial Sequence: Synthetic polypeptide"
  VARIANT (33)..(33): /replace="S" or "G" or "A"
  VARIANT (37)..(37): /replace="G" or "A"
  VARIANT (40)..(40): /replace="G" or "A"
  VARIANT (57)..(57): /replace="G" or "A"
  SITE (1)..(128): /note="Variant residues given in the sequence have no preference with respect to those in the annotations for variant positions"

SEQ ID NO: 5 - protein, 128 aa, Artificial Sequence; identical to SEQ ID NO: 1
  source: /note="Description of Artificial Sequence: Synthetic polypeptide"
  VARIANT (33)..(33): /replace="S" or "G" or "A"
  VARIANT (37)..(37): /replace="G" or "A"
  VARIANT (57)..(57): /replace="G" or "A"
  SITE (1)..(128): /note="Variant residues given in the sequence have no preference with respect to those in the annotations for variant positions"

SEQ ID NO: 6 - protein, 128 aa, Artificial Sequence
  source: /note="Description of Artificial Sequence: Synthetic polypeptide"
  VARIANT (33)..(33): /replace="S" or "G" or "A"
  SITE (1)..(128): /note="Variant residues given in the sequence have no preference with respect to those in the annotations for variant positions"
STKKTQLQLEHLLLDLQMILNGINNYKNPKLTRMLTAKFYMPKKATELKHLQCLEEALKPLEEVLNLAQSKNFHLRPRDLISNINVIVLELKGSETTFMCEYADETATIVEFLNRWITFSQSIISTLT

SEQ ID NO: 7 - protein, 128 aa, Artificial Sequence
  source: /note="Description of Artificial Sequence: Synthetic polypeptide"
STKKTQLQLEHLLLDLQMILNGINNYKNPKLTGMLTFKFYMPKKATELKHLQCLEEELKPLEEVLNLAQSKNFHLRPRDLISNINVIVLELKGSETTFMCEYADETATIVEFLNRWITFSQSIISTLT

SEQ ID NO: 8 - protein, 128 aa, Artificial Sequence
  source: /note="Description of Artificial Sequence: Synthetic polypeptide"
STKKTQLQLEHLLLDLQMILNGINNYKNPKLTAMLTFKFYMPKKATELKHLQCLEEELKPLEEVLNLAQSKNFHLRPRDLISNINVIVLELKGSETTFMCEYADETATIVEFLNRWITFSQSIISTLT

SEQ ID NO: 9 - protein, 128 aa, Artificial Sequence
  source: /note="Description of Artificial Sequence: Synthetic polypeptide"
STKKTQLQLEHLLLDLQMILNGINNYKNPKLTRMLGFKFYMPKKATELKHLQCLEEELKPLEEVLNLAQSKNFHLRPRDLISNINVIVLELKGSETTFMCEYADETATIVEFLNRWITFSQSIISTLT

SEQ ID NO: 10 - protein, 128 aa, Artificial Sequence
  source: /note="Description of Artificial Sequence: Synthetic polypeptide"
STKKTQLQLEHLLLDLQMILNGINNYKNPKLTRMLAFKFYMPKKATELKHLQCLEEELKPLEEVLNLAQSKNFHLRPRDLISNINVIVLELKGSETTFMCEYADETATIVEFLNRWITFSQSIISTLT

SEQ ID NO: 11 - protein, 128 aa, Artificial Sequence
  source: /note="Description of Artificial Sequence: Synthetic polypeptide"
STKKTQLQLEHLLLDLQMILNGINNYKNPKLTRMLTGKFYMPKKATELKHLQCLEEELKPLEEVLNLAQSKNFHLRPRDLISNINVIVLELKGSETTFMCEYADETATIVEFLNRWITFSQSIISTLT

SEQ ID NO: 12 - protein, 128 aa, Artificial Sequence
  source: /note="Description of Artificial Sequence: Synthetic polypeptide"
STKKTQLQLEHLLLDLQMILNGINNYKNPKLTRMLTAKFYMPKKATELKHLQCLEEELKPLEEVLNLAQSKNFHLRPRDLISNINVIVLELKGSETTFMCEYADETATIVEFLNRWITFSQSIISTLT

SEQ ID NO: 13 - protein, 128 aa, Artificial Sequence
  source: /note="Description of Artificial Sequence: Synthetic polypeptide"
STKKTQLQLEHLLLDLQMILNGINNYKNPKLTRMLTFKFGMPKKATELKHLQCLEEELKPLEEVLNLAQSKNFHLRPRDLISNINVIVLELKGSETTFMCEYADETATIVEFLNRWITFSQSIISTLT

SEQ ID NO: 14 - protein, 128 aa, Artificial Sequence
  source: /note="Description of Artificial Sequence: Synthetic polypeptide"
STKKTQLQLEHLLLDLQMILNGINNYKNPKLTRMLTFKFAMPKKATELKHLQCLEEELKPLEEVLNLAQSKNFHLRPRDLISNINVIVLELKGSETTFMCEYADETATIVEFLNRWITFSQSIISTLT

SEQ ID NO: 15 - protein, 128 aa, Artificial Sequence
  source: /note="Description of Artificial Sequence: Synthetic polypeptide"
STKKTQLQLEHLLLDLQMILNGINNYKNPKLTRMLTFKFYMPKKATELKHLQCLEAELKPLEEVLNLAQSKNFHLRPRDLISNINVIVLELKGSETTFMCEYADETATIVEFLNRWITFSQSIISTLT

SEQ ID NO: 16 - protein, 128 aa, Artificial Sequence
  source: /note="Description of Artificial Sequence: Synthetic polypeptide"
STKKTQLQLEHLLLDLQMILNGINNYKNPKLTRMLTFKFYMPKKATELKHLQCLEEALKPLEEVLNLAQSKNFHLRPRDLISNINVIVLELKGSETTFMCEYADETATIVEFLNRWITFSQSIISTLT

SEQ ID NO: 17 - protein, 128 aa, Artificial Sequence
  source: /note="Description of Artificial Sequence: Synthetic polypeptide"
STKKTQLQLEHLLLDLQMILNGINNYKNPKLTRMLTFKFYMPKKATELKHLQCLEEELKPLEAVLNLAQSKNFHLRPRDLISNINVIVLELKGSETTFMCEYADETATIVEFLNRWITFSQSIISTLT

SEQ ID NO: 18 - protein, 128 aa, Artificial Sequence
  source: /note="Description of Artificial Sequence: Synthetic polypeptide"
STKKTQLQLEHLLLDLQMILNGINNYKNPKLTRMLTFKFYMPKKATELKHLQCLEEELKPLEEVLNGAQSKNFHLRPRDLISNINVIVLELKGSETTFMCEYADETATIVEFLNRWITFSQSIISTLT

SEQ ID NO: 19 - protein, 128 aa, Artificial Sequence
  source: /note="Description of Artificial Sequence: Synthetic polypeptide"
STKKTQLQLEHLLLDLQMILNGINNYKNPKLTRMLTFKFYMPKKATELKHLQCLEEELKPLEEVLNLAGSKNFHLRPRDLISNINVIVLELKGSETTFMCEYADETATIVEFLNRWITFSQSIISTLT

SEQ ID NO: 20 - protein, 128 aa, Artificial Sequence
  source: /note="Description of Artificial Sequence: Synthetic polypeptide"
STKKTQLQLEHLLLDLQMILNGINNYKNPKLTRMLTFKFYMPKKATELKHLQCLEEELKPLEEVLNLAQSKNFHLRPRDLISNINVIVLELKGSETTFMCEGADETATIVEFLNRWITFSQSIISTLT

SEQ ID NO: 21 - protein, 128 aa, Artificial Sequence
  source: /note="Description of Artificial Sequence: Synthetic polypeptide"
STKKTQLQLEHLLLDLQMILNGINNYKNPKLTRMLTFKFYMPKKATELKHLQCLEEELKPLEEVLNLAQSKNFHLRPRDLISNINVIVLELKGSETTFMCEAADETATIVEFLNRWITFSQSIISTLT

SEQ ID NO: 22 - protein, 128 aa, Artificial Sequence
  source: /note="Description of Artificial Sequence: Synthetic polypeptide"
STKKTQLQLEHLLLDLQMILNGINNYKNPKLTRMLTFKFGMPKKATELKHLQCLEAELKPLEEVLNLAQSKNFHLRPRDLISNINVIVLELKGSETTFMCEYADETATIVEFLNRWITFSQSIISTLT

SEQ ID NO: 23 - protein, 128 aa, Artificial Sequence
  source: /note="Description of Artificial Sequence: Synthetic polypeptide"
STKKTQLQLEHLLLDLQMILNGINNYKNPKLTRMLTFKFGMPKKATELKHLQCLEEALKPLEEVLNLAQSKNFHLRPRDLISNINVIVLELKGSETTFMCEYADETATIVEFLNRWITFSQSIISTLT

SEQ ID NO: 24 - protein, 128 aa, Artificial Sequence
  source: /note="Description of Artificial Sequence: Synthetic polypeptide"
STKKTQLQLEHLLLDLQMILNGINNYKNPKLTGMLTFKFGMPKKATELKHLQCLEEELKPLEEVLNLAQSKNFHLRPRDLISNINVIVLELKGSETTFMCEYADETATIVEFLNRWITFSQSIISTLT

SEQ ID NO: 25 - protein, 128 aa, Artificial Sequence
  source: /note="Description of Artificial Sequence: Synthetic polypeptide"
STKKTQLQLEHLLLDLQMILNGINNYKNPKLTGMLTFKFYMPKKATELKHLQCLEAELKPLEEVLNLAQSKNFHLRPRDLISNINVIVLELKGSETTFMCEYADETATIVEFLNRWITFSQSIISTLT

SEQ ID NO: 26 - protein, 128 aa, Artificial Sequence
  source: /note="Description of Artificial Sequence: Synthetic polypeptide"
STKKTQLQLEHLLLDLQMILNGINNYKNPKLTRMLTAKFYMPKKATELKHLQCLEAELKPLEEVLNLAQSKNFHLRPRDLISNINVIVLELKGSETTFMCEYADETATIVEFLNRWITFSQSIISTLT

SEQ ID NO: 27 - protein, 128 aa, Artificial Sequence
  source: /note="Description of Artificial Sequence: Synthetic polypeptide"
STKKTQLQLEHLLLDLQMILNGINNYKNPKLTRMLTAKFGMPKKATELKHLQCLEEELKPLEEVLNLAQSKNFHLRPRDLISNINVIVLELKGSETTFMCEYADETATIVEFLNRWITFSQSIISTLT

SEQ ID NO: 28 - protein, 128 aa, Artificial Sequence
  source: /note="Description of Artificial Sequence: Synthetic polypeptide"
STKKTQLQLEHLLLDLQMILNGINNYKNPKLTRMLTFKFGMPKKATELKHLQCLEAALKPLEEVLNLAQSKNFHLRPRDLISNINVIVLELKGSETTFMCEYADETATIVEFLNRWITFSQSIISTLT

SEQ ID NO: 29 - protein, 128 aa, Artificial Sequence
  source: /note="Description of Artificial Sequence: Synthetic polypeptide"
STKKTQLQLEHLLLDLQMILNGINNYKNPKLTRMLTFKFYMPKKATELKHLQCLEAALKPLEEVLNLAQSKNFHLRPRDLISNINVIVLELKGSETTFMCEYADETATIVEFLNRWITFSQSIISTLT

SEQ ID NO: 30 - protein, 128 aa, Artificial Sequence
  source: /note="Description of Artificial Sequence: Synthetic polypeptide"
STKKTQLQLEHLLLDLQMILNGINNYKNPKLTGMLTAKFYMPKKATELKHLQCLEEELKPLEEVLNLAQSKNFHLRPRDLISNINVIVLELKGSETTFMCEYADETATIVEFLNRWITFSQSIISTLT

SEQ ID NO: 31 - protein, 128 aa, Artificial Sequence
  source: /note="Description of Artificial Sequence: Synthetic polypeptide"
STKKTQLQLEHLLLDLQMILNGINNYKNPKLTRMLTAKFAMPKKATELKHLQCLEEELKPLEEVLNGAQSKNFHLRPRDLISNINVIVLELKGSETTFMCEYADETATIVEFLNRWITFSQSIISTLT

SEQ ID NO: 32 - protein, 128 aa, Artificial Sequence
  source: /note="Description of Artificial Sequence: Synthetic polypeptide"
STKKTQLQLEHLLLDLQMILNGINNYKNPKLTGMLTAKFGMPKKATELKHLQCLEEELKPLEEVLNLAQSKNFHLRPRDLISNINVIVLELKGSETTFMCEYADETATIVEFLNRWITFSQSIISTLT

SEQ ID NO: 33 - protein, 128 aa, Artificial Sequence; identical to SEQ ID NO: 6
  source: /note="Description of Artificial Sequence: Synthetic polypeptide"

SEQ ID NO: 34 - protein, 128 aa, Artificial Sequence
  source: /note="Description of Artificial Sequence: Synthetic polypeptide"
STKKTQLQLEHLLLDLQMILNGINNYKNPKLTRMLTAKFGMPKKATELKHLQCLEEALKPLEEVLNLAQSKNFHLRPRDLISNINVIVLELKGSETTFMCEYADETATIVEFLNRWITFSQSIISTLT

SEQ ID NO: 35 - protein, 128 aa, Artificial Sequence
  source: /note="Description of Artificial Sequence: Synthetic polypeptide"
STKKTQLQLEHLLLDLQMILNGINNYKNPKLTRMLTAKFGMPKKATELKHLQCLEAELKPLEEVLNLAQSKNFHLRPRDLISNINVIVLELKGSETTFMCEYADETATIVEFLNRWITFSQSIISTLT

SEQ ID NO: 36 - protein, 128 aa, Artificial Sequence
  source: /note="Description of Artificial Sequence: Synthetic polypeptide"
STKKTQLQLEHLLLDLQMILNGINNYKNPKLTGMLTFKFGMPKKATELKHLQCLEAELKPLEEVLNLAQSKNFHLRPRDLISNINVIVLELKGSETTFMCEYADETATIVEFLNRWITFSQSIISTLT

SEQ ID NO: 37 - protein, 128 aa, Artificial Sequence
  source: /note="Description of Artificial Sequence: Synthetic polypeptide"
STKKTQLQLEHLLLDLQMILNGINNYKNPKLTGMLTAKFYMPKKATELKHLQCLEAELKPLEEVLNLAQSKNFHLRPRDLISNINVIVLELKGSETTFMCEYADETATIVEFLNRWITFSQSIISTLT

SEQ ID NO: 38 - protein, 128 aa, Artificial Sequence
  source: /note="Description of Artificial Sequence: Synthetic polypeptide"
STKKTQLQLEHLLLDLQMILNGINNYKNPKLTGMLTFKFGMPKKATELKHLQCLEEALKPLEEVLNLAQSKNFHLRPRDLISNINVIVLELKGSETTFMCEYADETATIVEFLNRWITFSQSIISTLT

SEQ ID NO: 39 - protein, 128 aa, Artificial Sequence
  source: /note="Description of Artificial Sequence: Synthetic polypeptide"
STKKTQLQLEHLLLDLQMILNGINNYKNPKLTGMLTFKFYMPKKATELKHLQCLEEALKPLEEVLNLAQSKNFHLRPRDLISNINVIVLELKGSETTFMCEYADETATIVEFLNRWITFSQSIISTLT

SEQ ID NO: 40 - protein, 128 aa, Artificial Sequence
  source: /note="Description of Artificial Sequence: Synthetic polypeptide"
STKKTQLQLEHLLLDLQMILNGINNYKNPKLTGMLTAKFYMPKKATELKHLQCLEEALKPLEEVLNLAQSKNFHLRPRDLISNINVIVLELKGSETTFMCEYADETATIVEFLNRWITFSQSIISTLT

SEQ ID NO: 41 - protein, 128 aa, Artificial Sequence
  source: /note="Description of Artificial Sequence: Synthetic polypeptide"
STKKTQLQLEHLLLDLQMILNGINNYKNPKLTRMLTAKFYMPKKATELKHLQCLEAALKPLEEVLNLAQSKNFHLRPRDLISNINVIVLELKGSETTFMCEYADETATIVEFLNRWITFSQSIISTLT

SEQ ID NO: 42 - protein, 128 aa, Artificial Sequence
  source: /note="Description of Artificial Sequence: Synthetic polypeptide"
STKKTQLQLEHLLLDLQMILNGINNYKNPKLTGMLTFKFYMPKKATELKHLQCLEAALKPLEEVLNLAQSKNFHLRPRDLISNINVIVLELKGSETTFMCEYADETATIVEFLNRWITFSQSIISTLT

SEQ ID NO: 43 - protein, 128 aa, Artificial Sequence; identical to SEQ ID NO: 1
  source: /note="Description of Artificial Sequence: Synthetic polypeptide"

SEQ ID NO: 44 - protein, 133 aa, Artificial Sequence
  source: /note="Description of Artificial Sequence: Synthetic polypeptide"
APASSSTKKTQLQLEHLLLDLQMILNGINNYKNPKLTRMLTFKFYMPKKATELKHLQCLEEELKPLEEVLNLAQSKNFHLRPRDLISNINVIVLELKGSETTFMCEYADETATIVEFLNRWITFSQSIISTLT

SEQ ID NO: 45 - protein, 228 aa, Artificial Sequence
  source: /note="Description of Artificial Sequence: Synthetic polypeptide"
ESKYGPPCPPCPAPEAAGGPSVFLFPPKPKDTLMISRTPEVTCVVVDVSQEDPEVQFNWYVDGVEVHNAKTKPREEQFNSTYRVVSVLTVLHQDWLNGKEYKCKVSNKGLPSSIEKTISKAKGQPREPQVYTLPPSQEEMTKNQVSLWCLVKGFYPSDIAVEWESNGQPENNYKTTPPVLDSDGSFFLYSRLTVDKSRWQEGNVFSCSVMHEALHNHYTQKSLSLSLG

SEQ ID NO: 46 - protein, 229 aa, Artificial Sequence
  source: /note="Description of Artificial Sequence: Synthetic polypeptide"
ESKYGPPCPPCPAPEAAGGPSVFLFPPKPKDTLMISRTPEVTCVVVDVSQEDPEVQFNWYVDGVEVHNAKTKPREEQFNSTYRVVSVLTVLHQDWLNGKEYKCKVSNKGLPSSIEKTISKAKGQPREPQVYTLPPSQEEMTKNQVSLSCAVKGFYPSDIAVEWESNGQPENNYKTTPPVLDSDGSFFLVSRLTVDKSRWQEGNVFSCSVMHEALHNRFTQKSLSLSLGK

SEQ ID NO: 47 - protein, 228 aa, Artificial Sequence
  source: /note="Description of Artificial Sequence: Synthetic polypeptide"
ESKYGPPCPPCPAPEAAGGPSVFLFPPKPKDTLMISRTPEVTCVVVDVSQEDPEVQFNWYVDGVEVHNAKTKPREEQFNSTYRVVSVLTVLHQDWLNGKEYKCKVSNKGLPSSIEKTISKAKGQPREPQVYTLPPSQEEMTKNQVSLSCAVKGFYPSDIAVEWESNGQPENNYKTTPPVLDSDGSFFLVSRLTVDKSRWQEGNVFSCSVMHEALHNRFTQKSLSLSLG

SEQ ID NO: 48 - protein, 229 aa, Artificial Sequence
  source: /note="Description of Artificial Sequence: Synthetic polypeptide"
ESKYGPPCPPCPAPEAAGGPSVFLFPPKPKDTLMISRTPEVTCVVVDVSQEDPEVQFNWYVDGVEVHNAKTKPREEQFNSTYRVVSVLTVLHQDWLNGKEYKCKVSNKGLPSSIEKTISKAKGQPREPQVYTLPPSQEEMTKNQVSLWCLVKGFYPSDIAVEWESNGQPENNYKTTPPVLDSDGSFFLYSRLTVDKSRWQEGNVFSCSVMHEALHNHYTQKSLSLSLGK

SEQ ID NO: 49 - protein, 228 aa, Artificial Sequence
  source: /note="Description of Artificial Sequence: Synthetic polypeptide"
ESKYGPPCPPCPAPEAAGGPSVFLFPPKPKDTLYITREPEVTCVVVDVSQEDPEVQFNWYVDGVEVHNAKTKPREEQFNSTYRVVSVLTVLHQDWLNGKEYKCKVSNKGLPSSIEKTISKAKGQPREPQVYTLPPSQEEMTKNQVSLWCLVKGFYPSDIAVEWESNGQPENNYKTTPPVLDSDGSFFLYSRLTVDKSRWQEGNVFSCSVMHEALHNHYTQKSLSLSLG

SEQ ID NO: 50 - protein, 229 aa, Artificial Sequence
  source: /note="Description of Artificial Sequence: Synthetic polypeptide"
ESKYGPPCPPCPAPEAAGGPSVFLFPPKPKDTLMISRTPEVTCVVVDVSQEDPEVQFNWYVDGVEVHNAKTKPREEQFNSTYRVVSVLTVLHQDWLNGKEYKCKVSNKGLPSSIEKTISKAKGQPREPQVYTLPPSQEEMTKNQVSLWCLVKGFYPSDIAVEWESNGQPENNYKTTPPVLDSDGSFFLYSRLTVDKSRWQEGNVFSCSVLHEALHSHYTQKSLSLSLGK

SEQ ID NO: 51 - protein, 229 aa, Artificial Sequence
  source: /note="Description of Artificial Sequence: Synthetic polypeptide"
ESKYGPPCPPCPAPEAAGGPSVFLFPPKPKDTLYITREPEVTCVVVDVSQEDPEVQFNWYVDGVEVHNAKTKPREEQFNSTYRVVSVLTVLHQDWLNGKEYKCKVSNKGLPSSIEKTISKAKGQPREPQVYTLPPSQEEMTKNQVSLSCAVKGFYPSDIAVEWESNGQPENNYKTTPPVLDSDGSFFLVSRLTVDKSRWQEGNVFSCSVMHEALHNRFTQKSLSLSLGK

SEQ ID NO: 52 - protein, 228 aa, Artificial Sequence
  source: /note="Description of Artificial Sequence: Synthetic polypeptide"
ESKYGPPCPPCPAPEAAGGPSVFLFPPKPKDTLYITREPEVTCVVVDVSQEDPEVQFNWYVDGVEVHNAKTKPREEQFNSTYRVVSVLTVLHQDWLNGKEYKCKVSNKGLPSSIEKTISKAKGQPREPQVYTLPPSQEEMTKNQVSLSCAVKGFYPSDIAVEWESNGQPENNYKTTPPVLDSDGSFFLVSRLTVDKSRWQEGNVFSCSVMHEALHNRFTQKSLSLSLG

SEQ ID NO: 53 - protein, 229 aa, Artificial Sequence
  source: /note="Description of Artificial Sequence: Synthetic polypeptide"
ESKYGPPCPPCPAPEAAGGPSVFLFPPKPKDTLYITREPEVTCVVVDVSQEDPEVQFNWYVDGVEVHNAKTKPREEQFNSTYRVVSVLTVLHQDWLNGKEYKCKVSNKGLPSSIEKTISKAKGQPREPQVYTLPPSQEEMTKNQVSLWCLVKGFYPSDIAVEWESNGQPENNYKTTPPVLDSDGSFFLYSRLTVDKSRWQEGNVFSCSVMHEALHNHYTQKSLSLSLGK

SEQ ID NO: 54 - protein, 228 aa, Artificial Sequence
  source: /note="Description of Artificial Sequence: Synthetic polypeptide"
ESKYGPPCPPCPAPEAAGGPSVFLFPPKPKDTLMISRTPEVTCVVVDVSQEDPEVQFNWYVDGVEVHNAKTKPREEQFNSTYRVVSVLTVLHQDWLNGKEYKCKVSNKGLPSSIEKTISKAKGQPREPQVYTLPPSQEEMTKNQVSLWCLVKGFYPSDIAVEWESNGQPENNYKTTPPVLDSDGSFFLYSRLTVDKSRWQEGNVFSCSVLHEALHSHYTQKSLSLSLG

SEQ ID NO: 55 - protein, 229 aa, Artificial Sequence
  source: /note="Description of Artificial Sequence: Synthetic polypeptide"
ESKYGPPCPPCPAPEAAGGPSVFLFPPKPKDTLMISRTPEVTCVVVDVSQEDPEVQFNWYVDGVEVHNAKTKPREEQFNSTYRVVSVLTVLHQDWLNGKEYKCKVSNKGLPSSIEKTISKAKGQPREPQVYTLPPSQEEMTKNQVSLSCAVKGFYPSDIAVEWESNGQPENNYKTTPPVLDSDGSFFLVSRLTVDKSRWQEGNVFSCSVLHEALHSRFTQKSLSLSLGK

SEQ ID NO: 56 - protein, 228 aa, Artificial Sequence
  source: /note="Description of Artificial Sequence: Synthetic polypeptide"
ESKYGPPCPPCPAPEAAGGPSVFLFPPKPKDTLMISRTPEVTCVVVDVSQEDPEVQFNWYVDGVEVHNAKTKPREEQFNSTYRVVSVLTVLHQDWLNGKEYKCKVSNKGLPSSIEKTISKAKGQPREPQVYTLPPSQEEMTKNQVSLSCAVKGFYPSDIAVEWESNGQPENNYKTTPPVLDSDGSFFLVSRLTVDKSRWQEGNVFSCSVLHEALHSRFTQKSLSLSLG

SEQ ID NO: 57 - protein, 231 aa, Artificial Sequence
  source: /note="Description of Artificial Sequence: Synthetic polypeptide"
EPKSSDKTHTCPPCPAPEAAGGPSVFLFPPKPKDTLMISRTPEVTCVVVDVSHEDPEVKFNWYVDGVEVHNAKTKPREEQYNSTYRVVSVLTVLHQDWLNGKEYKCKVSNKALPASIEKTISKAKGQPREPQVYTLPPSREEMTKNQVSLWCLVKGFYPSDIAVEWESNGQPENNYKTTPPVLDSDGSFFLYSKLTVDKSRWQQGNVFSCSVMHEALHNHYTQKSLSLSPG

SEQ ID NO: 58 - protein, 232 aa, Artificial Sequence
  source: /note="Description of Artificial Sequence: Synthetic polypeptide"
EPKSCDKTHTCPPCPAPEAAGGPSVFLFPPKPKDTLMISRTPEVTCVVVDVSHEDPEVKFNWYVDGVEVHNAKTKPREEQYNSTYRVVSVLTVLHQDWLNGKEYKCKVSNKALPASIEKTISKAKGQPREPQVYTLPPSREEMTKNQVSLSCAVKGFYPSDIAVEWESNGQPENNYKTTPPVLDSDGSFFLVSKLTVDKSRWQQGNVFSCSVMHEALHNRFTQKSLSLSPGK

SEQ ID NO: 59 - protein, 231 aa, Artificial Sequence
  source: /note="Description of Artificial Sequence: Synthetic polypeptide"
EPKSCDKTHTCPPCPAPEAAGGPSVFLFPPKPKDTLMISRTPEVTCVVVDVSHEDPEVKFNWYVDGVEVHNAKTKPREEQYNSTYRVVSVLTVLHQDWLNGKEYKCKVSNKALPASIEKTISKAKGQPREPQVYTLPPSREEMTKNQVSLSCAVKGFYPSDIAVEWESNGQPENNYKTTPPVLDSDGSFFLVSKLTVDKSRWQQGNVFSCSVMHEALHNRFTQKSLSLSPG

SEQ ID NO: 60 - protein, 232 aa, Artificial Sequence
  source: /note="Description of Artificial Sequence: Synthetic polypeptide"
EPKSSDKTHTCPPCPAPEAAGGPSVFLFPPKPKDTLMISRTPEVTCVVVDVSHEDPEVKFNWYVDGVEVHNAKTKPREEQYNSTYRVVSVLTVLHQDWLNGKEYKCKVSNKALPASIEKTISKAKGQPREPQVYTLPPSREEMTKNQVSLWCLVKGFYPSDIAVEWESNGQPENNYKTTPPVLDSDGSFFLYSKLTVDKSRWQQGNVFSCSVMHEALHNHYTQKSLSLSPGK

SEQ ID NO: 61 - protein, 231 aa, Artificial Sequence
  source: /note="Description of Artificial Sequence: Synthetic polypeptide"
EPKSSDKTHTCPPCPAPEAAGGPSVFLFPPKPKDTLYITREPEVTCVVVDVSHEDPEVKFNWYVDGVEVHNAKTKPREEQYNSTYRVVSVLTVLHQDWLNGKEYKCKVSNKALPASIEKTISKAKGQPREPQVYTLPPSREEMTKNQVSLWCLVKGFYPSDIAVEWESNGQPENNYKTTPPVLDSDGSFFLYSKLTVDKSRWQQGNVFSCSVMHEALHNHYTQKSLSLSPG

SEQ ID NO: 62 - protein, 232 aa, Artificial Sequence
  source: /note="Description of Artificial Sequence: Synthetic polypeptide"
EPKSCDKTHTCPPCPAPEAAGGPSVFLFPPKPKDTLYITREPEVTCVVVDVSHEDPEVKFNWYVDGVEVHNAKTKPREEQYNSTYRVVSVLTVLHQDWLNGKEYKCKVSNKALPASIEKTISKAKGQPREPQVYTLPPSREEMTKNQVSLSCAVKGFYPSDIAVEWESNGQPENNYKTTPPVLDSDGSFFLVSKLTVDKSRWQQGNVFSCSVMHEALHNRFTQKSLSLSPGK

SEQ ID NO: 63 - protein, 231 aa, Artificial Sequence
  source: /note="Description of Artificial Sequence: Synthetic polypeptide"
EPKSCDKTHTCPPCPAPEAAGGPSVFLFPPKPKDTLYITREPEVTCVVVDVSHEDPEVKFNWYVDGVEVHNAKTKPREEQYNSTYRVVSVLTVLHQDWLNGKEYKCKVSNKALPASIEKTISKAKGQPREPQVYTLPPSREEMTKNQVSLSCAVKGFYPSDIAVEWESNGQPENNYKTTPPVLDSDGSFFLVSKLTVDKSRWQQGNVFSCSVMHEALHNHYTQKSLSLSPG

SEQ ID NO: 64 - protein, 232 aa, Artificial Sequence
  source: /note="Description of Artificial Sequence: Synthetic polypeptide"
EPKSSDKTHTCPPCPAPEAAGGPSVFLFPPKPKDTLYITREPEVTCVVVDVSHEDPEVKFNWYVDGVEVHNAKTKPREEQYNSTYRVVSVLTVLHQDWLNGKEYKCKVSNKALPASIEKTISKAKGQPREPQVYTLPPSREEMTKNQVSLWCLVKGFYPSDIAVEWESNGQPENNYKTTPPVLDSDGSFFLYSKLTVDKSRWQQGNVFSCSVMHEALHNRFTQKSLSLSPGK

SEQ ID NO: 65 - protein, 231 aa, Artificial Sequence
  source: /note="Description of Artificial Sequence: Synthetic polypeptide"
EPKSCDKTHTCPPCPAPEAAGGPSVFLFPPKPKDTLYITREPEVTCVVVDVSHEDPEVKFNWYVDGVEVHNAKTKPREEQYNSTYRVVSVLTVLHQDWLNGKEYKCKVSNKALPASIEKTISKAKGQPREPQVYTLPPSREEMTKNQVSLSCAVKGFYPSDIAVEWESNGQPENNYKTTPPVLDSDGSFFLVSKLTVDKSRWQQGNVFSCSVMHEALHNRFTQKSLSLSPG

SEQ ID NO: 66 - protein, 232 aa, Artificial Sequence
  source: /note="Description of Artificial Sequence: Synthetic polypeptide"
EPKSSDKTHTCPPCPAPEAAGGPSVFLFPPKPKDTLYITREPEVTCVVVDVSHEDPEVKFNWYVDGVEVHNAKTKPREEQYNSTYRVVSVLTVLHQDWLNGKEYKCKVSNKALPASIEKTISKAKGQPREPQVYTLPPSREEMTKNQVSLWCLVKGFYPSDIAVEWESNGQPENNYKTTPPVLDSDGSFFLYSKLTVDKSRWQQGNVFSCSVMHEALHNHYTQKSLSLSPGK

SEQ ID NO: 67 - protein, 231 aa, Artificial Sequence
  source: /note="Description of Artificial Sequence: Synthetic polypeptide"
EPKSSDKTHTCPPCPAPEAAGGPSVFLFPPKPKDTLYITREPEVTCVVVDVSHEDPEVKFNWYVDGVEVHNAKTKPREEQYNSTYRVVSVLTVLHQDWLNGKEYKCKVSNKALPASIEKTISKAKGQPREPQVYTLPPSREEMTKNQVSLWCLVKGFYPSDIAVEWESNGQPENNYKTTPPVLDSDGSFFLYSKLTVDKSRWQQGNVFSCSVMHEALHNRFTQKSLSLSPG

SEQ ID NO: 68 - protein, 232 aa, Artificial Sequence
  source: /note="Description of Artificial Sequence: Synthetic polypeptide"
EPKSCDKTHTCPPCPAPEAAGGPSVFLFPPKPKDTLYITREPEVTCVVVDVSHEDPEVKFNWYVDGVEVHNAKTKPREEQYNSTYRVVSVLTVLHQDWLNGKEYKCKVSNKALPASIEKTISKAKGQPREPQVYTLPPSREEMTKNQVSLSCAVKGFYPSDIAVEWESNGQPENNYKTTPPVLDSDGSFFLVSKLTVDKSRWQQGNVFSCSVMHEALHNHYTQKSLSLSPGK

SEQ ID NO: 69 - protein, 231 aa, Artificial Sequence
  source: /note="Description of Artificial Sequence: Synthetic polypeptide"
EPKSSDKTHTCPPCPAPEAAGGPSVFLFPPKPKDTLMISRTPEVTCVVVDVSHEDPEVKFNWYVDGVEVHNAKTKPREEQYNSTYRVVSVLTVLHQDWLNGKEYKCKVSNKALPASIEKTISKAKGQPREPQVYTLPPSREEMTKNQVSLWCLVKGFYPSDIAVEWESNGQPENNYKTTPPVLDSDGSFFLYSKLTVDKSRWQQGNVFSCSVLHEALHSHYTQKSLSLSPG

SEQ ID NO: 70 - protein, 232 aa, Artificial Sequence
  source: /note="Description of Artificial Sequence: Synthetic polypeptide"
EPKSCDKTHTCPPCPAPEAAGGPSVFLFPPKPKDTLMISRTPEVTCVVVDVSHEDPEVKFNWYVDGVEVHNAKTKPREEQYNSTYRVVSVLTVLHQDWLNGKEYKCKVSNKALPASIEKTISKAKGQPREPQVYTLPPSREEMTKNQVSLSCAVKGFYPSDIAVEWESNGQPENNYKTTPPVLDSDGSFFLVSKLTVDKSRWQQGNVFSCSVLHEALHSRFTQKSLSLSPGK

SEQ ID NO: 71 - protein, 231 aa, Artificial Sequence
  source: /note="Description of Artificial Sequence: Synthetic polypeptide"
EPKSCDKTHTCPPCPAPEAAGGPSVFLFPPKPKDTLMISRTPEVTCVVVDVSHEDPEVKFNWYVDGVEVHNAKTKPREEQYNSTYRVVSVLTVLHQDWLNGKEYKCKVSNKALPASIEKTISKAKGQPREPQVYTLPPSREEMTKNQVSLSCAVKGFYPSDIAVEWESNGQPENNYKTTPPVLDSDGSFFLVSKLTVDKSRWQQGNVFSCSVLHEALHSRFTQKSLSLSPG

SEQ ID NO: 72 - protein, 232 aa, Artificial Sequence
  source: /note="Description of Artificial Sequence: Synthetic polypeptide"
EPKSSDKTHTCPPCPAPEAAGGPSVFLFPPKPKDTLMISRTPEVTCVVVDVSHEDPEVKFNWYVDGVEVHNAKTKPREEQYNSTYRVVSVLTVLHQDWLNGKEYKCKVSNKALPASIEKTISKAKGQPREPQVYTLPPSREEMTKNQVSLWCLVKGFYPSDIAVEWESNGQPENNYKTTPPVLDSDGSFFLYSKLTVDKSRWQQGNVFSCSVLHEALHSHYTQKSLSLSPGK

SEQ ID NO: 73 - skipped

SEQ ID NO: 74 - protein, 232 aa, Homo sapiens
EPKSCDKTHTCPPCPAPELLGGPSVFLFPPKPKDTLMISRTPEVTCVVVDVSHEDPEVKFNWYVDGVEVHNAKTKPREEQYNSTYRVVSVLTVLHQDWLNGKEYKCKVSNKALPAPIEKTISKAKGQPREPQVYTLPPSREEMTKNQVSLTCLVKGFYPSDIAVEWESNGQPENNYKTTPPVLDSDGSFFLYSKLTVDKSRWQQGNVFSCSVMHEALHNHYTQKSLSLSPGK

SEQ ID NO: 75 - protein, 376 aa, Artificial Sequence
  source: /note="Description of Artificial Sequence: Synthetic polypeptide"
  VARIANT (281)..(281): /replace="S" or "G" or "A"
  VARIANT (284)..(284): /replace="G" or "A"
  VARIANT (285)..(285): /replace="G" or "A"
  VARIANT (288)..(288): /replace="G" or "A"
  VARIANT (304)..(304): /replace="G" or "A"
  VARIANT (305)..(305): /replace="G" or "A"
  VARIANT (311)..(311): /replace="G" or "A"
  VARIANT (315)..(315): /replace="G" or "A"
  VARIANT (317)..(317): /replace="G" or "A"
  VARIANT (350)..(350): /replace="G" or "A"
  SITE (1)..(376): /note="Variant residues given in the sequence have no preference with respect to those in the annotations for variant positions"
ESKYGPPCPPCPAPEAAGGPSVFLFPPKPKDTLMISRTPEVTCVVVDVSQEDPEVQFNWYVDGVEVHNAKTKPREEQFNSTYRVVSVLTVLHQDWLNGKEYKCKVSNKGLPSSIEKTISKAKGQPREPQVYTLPPSQEEMTKNQVSLWCLVKGFYPSDIAVEWESNGQPENNYKTTPPVLDSDGSFFLYSRLTVDKSRWQEGNVFSCSVMHEALHNHYTQKSLSLSLGGGGGSGGGGSGGGGSGGGGSSTKKTQLQLEHLLLDLQMILNGINNYKNPKLTRMLTFKFYMPKKATELKHLQCLEEELKPLEEVLNLAQSKNFHLRPRDLISNINVIVLELKGSETTFMCEYADETATIVEFLNRWITFSQSIISTLT

SEQ ID NO: 76 - protein, 376 aa, Artificial Sequence; identical to SEQ ID NO: 75
  source: /note="Description of Artificial Sequence: Synthetic polypeptide"
  VARIANT (281)..(281): /replace="S" or "G" or "A"
  VARIANT (285)..(285): /replace="G" or "A"
  VARIANT (288)..(288): /replace="G" or "A"
  VARIANT (304)..(304): /replace="G" or "A"
  VARIANT (305)..(305): /replace="G" or "A"
  VARIANT (315)..(315): /replace="G" or "A"
  SITE (1)..(376): /note="Variant residues given in the sequence have no preference with respect to those in the annotations for variant positions"

SEQ ID NO: 77 - protein, 376 aa, Artificial Sequence; identical to SEQ ID NO: 75
  source: /note="Description of Artificial Sequence: Synthetic polypeptide"
  VARIANT (281)..(281): /replace="S" or "G" or "A"
  VARIANT (285)..(285): /replace="G" or "A"
  VARIANT (288)..(288): /replace="G" or "A"
  VARIANT (304)..(304): /replace="G" or "A"
  VARIANT (305)..(305): /replace="G" or "A"
  SITE (1)..(376): /note="Variant residues given in the sequence have no preference with respect to those in the annotations for variant positions"

SEQ ID NO: 78 - protein, 376 aa, Artificial Sequence; identical to SEQ ID NO: 75
  source: /note="Description of Artificial Sequence: Synthetic polypeptide"
  VARIANT (281)..(281): /replace="S" or "G" or "A"
  VARIANT (285)..(285): /replace="G" or "A"
  VARIANT (288)..(288): /replace="G" or "A"
  VARIANT (305)..(305): /replace="G" or "A"
  SITE (1)..(376): /note="Variant residues given in the sequence have no preference with respect to those in the annotations for variant positions"

SEQ ID NO: 79 - protein, 376 aa, Artificial Sequence; identical to SEQ ID NO: 75
  source: /note="Description of Artificial Sequence: Synthetic polypeptide"
  VARIANT (281)..(281): /replace="S" or "G" or "A"
  VARIANT (285)..(285): /replace="G" or "A"
  VARIANT (305)..(305): /replace="G" or "A"
  SITE (1)..(376): /note="Variant residues given in the sequence have no preference with respect to those in the annotations for variant positions"

SEQ ID NO: 80 - protein, 376 aa, Artificial Sequence
  source: /note="Description of Artificial Sequence: Synthetic polypeptide"
  VARIANT (281)..(281): /replace="S" or "G" or "A"
  SITE (1)..(376): /note="Variant residues given in the sequence have no preference with respect to those in the annotations for variant positions"
ESKYGPPCPPCPAPEAAGGPSVFLFPPKPKDTLMISRTPEVTCVVVDVSQEDPEVQFNWYVDGVEVHNAKTKPREEQFNSTYRVVSVLTVLHQDWLNGKEYKCKVSNKGLPSSIEKTISKAKGQPREPQVYTLPPSQEEMTKNQVSLWCLVKGFYPSDIAVEWESNGQPENNYKTTPPVLDSDGSFFLYSRLTVDKSRWQEGNVFSCSVMHEALHNHYTQKSLSLSLGGGGGSGGGGSGGGGSGGGGSSTKKTQLQLEHLLLDLQMILNGINNYKNPKLTRMLTAKFYMPKKATELKHLQCLEEALKPLEEVLNLAQSKNFHLRPRDLISNINVIVLELKGSETTFMCEYADETATIVEFLNRWITFSQSIISTLT

SEQ ID NO: 81 - protein, 376 aa, Artificial Sequence
  source: /note="Description of Artificial Sequence: Synthetic polypeptide"
ESKYGPPCPPCPAPEAAGGPSVFLFPPKPKDTLMISRTPEVTCVVVDVSQEDPEVQFNWYVDGVEVHNAKTKPREEQFNSTYRVVSVLTVLHQDWLNGKEYKCKVSNKGLPSSIEKTISKAKGQPREPQVYTLPPSQEEMTKNQVSLWCLVKGFYPSDIAVEWESNGQPENNYKTTPPVLDSDGSFFLYSRLTVDKSRWQEGNVFSCSVMHEALHNHYTQKSLSLSLGGGGGSGGGGSGGGGSGGGGSSTKKTQLQLEHLLLDLQMILNGINNYKNPKLTGMLTFKFYMPKKATELKHLQCLEEELKPLEEVLNLAQSKNFHLRPRDLISNINVIVLELKGSETTFMCEYADETATIVEFLNRWITFSQSIISTLT

SEQ ID NO: 82 - protein, 376 aa, Artificial Sequence
  source: /note="Description of Artificial Sequence: Synthetic polypeptide"
ESKYGPPCPPCPAPEAAGGPSVFLFPPKPKDTLMISRTPEVTCVVVDVSQEDPEVQFNWYVDGVEVHNAKTKPREEQFNSTYRVVSVLTVLHQDWLNGKEYKCKVSNKGLPSSIEKTISKAKGQPREPQVYTLPPSQEEMTKNQVSLWCLVKGFYPSDIAVEWESNGQPENNYKTTPPVLDSDGSFFLYSRLTVDKSRWQEGNVFSCSVMHEALHNHYTQKSLSLSLGGGGGSGGGGSGGGGSGGGGSSTKKTQLQLEHLLLDLQMILNGINNYKNPKLTAMLTFKFYMPKKATELKHLQCLEEELKPLEEVLNLAQSKNFHLRPRDLISNINVIVLELKGSETTFMCEYADETATIVEFLNRWITFSQSIISTLT

SEQ ID NO: 83 - protein, 376 aa, Artificial Sequence
  source: /note="Description of Artificial Sequence: Synthetic polypeptide"
ESKYGPPCPPCPAPEAAGGPSVFLFPPKPKDTLMISRTPEVTCVVVDVSQEDPEVQFNWYVDGVEVHNAKTKPREEQFNSTYRVVSVLTVLHQDWLNGKEYKCKVSNKGLPSSIEKTISKAKGQPREPQVYTLPPSQEEMTKNQVSLWCLVKGFYPSDIAVEWESNGQPENNYKTTPPVLDSDGSFFLYSRLTVDKSRWQEGNVFSCSVMHEALHNHYTQKSLSLSLGGGGGSGGGGSGGGGSGGGGSSTKKTQLQLEHLLLDLQMILNGINNYKNPKLTRMLGFKFYMPKKATELKHLQCLEEELKPLEEVLNLAQSKNFHLRPRDLISNINVIVLELKGSETTFMCEYADETATIVEFLNRWITFSQSIISTLT

SEQ ID NO: 84 - protein, 376 aa, Artificial Sequence
  source: /note="Description of Artificial Sequence: Synthetic polypeptide"
ESKYGPPCPPCPAPEAAGGPSVFLFPPKPKDTLMISRTPEVTCVVVDVSQEDPEVQFNWYVDGVEVHNAKTKPREEQFNSTYRVVSVLTVLHQDWLNGKEYKCKVSNKGLPSSIEKTISKAKGQPREPQVYTLPPSQEEMTKNQVSLWCLVKGFYPSDIAVEWESNGQPENNYKTTPPVLDSDGSFFLYSRLTVDKSRWQEGNVFSCSVMHEALHNHYTQKSLSLSLGGGGGSGGGGSGGGGSGGGGSSTKKTQLQLEHLLLDLQMILNGINNYKNPKLTRMLAFKFYMPKKATELKHLQCLEEELKPLEEVLNLAQSKNFHLRPRDLISNINVIVLELKGSETTFMCEYADETATIVEFLNRWITFSQSIISTLT

SEQ ID NO: 85 - protein, 376 aa, Artificial Sequence
  source: /note="Description of Artificial Sequence: Synthetic polypeptide"
ESKYGPPCPPCPAPEAAGGPSVFLFPPKPKDTLMISRTPEVTCVVVDVSQEDPEVQFNWYVDGVEVHNAKTKPREEQFNSTYRVVSVLTVLHQDWLNGKEYKCKVSNKGLPSSIEKTISKAKGQPREPQVYTLPPSQEEMTKNQVSLWCLVKGFYPSDIAVEWESNGQPENNYKTTPPVLDSDGSFFLYSRLTVDKSRWQEGNVFSCSVMHEALHNHYTQKSLSLSLGGGGGSGGGGSGGGGSGGGGSSTKKTQLQLEHLLLDLQMILNGINNYKNPKLTRMLTGKFYMPKKATELKHLQCLEEELKPLEEVLNLAQSKNFHLRPRDLISNINVIVLELKGSETTFMCEYADETATIVEFLNRWITFSQSIISTLT

SEQ ID NO: 86 - protein, 376 aa, Artificial Sequence
  source: /note="Description of Artificial Sequence: Synthetic polypeptide"
ESKYGPPCPPCPAPEAAGGPSVFLFPPKPKDTLMISRTPEVTCVVVDVSQEDPEVQFNWYVDGVEVHNAKTKPREEQFNSTYRVVSVLTVLHQDWLNGKEYKCKVSNKGLPSSIEKTISKAKGQPREPQVYTLPPSQEEMTKNQVSLWCLVKGFYPSDIAVEWESNGQPENNYKTTPPVLDSDGSFFLYSRLTVDKSRWQEGNVFSCSVMHEALHNHYTQKSLSLSLGGGGGSGGGGSGGGGSGGGGSSTKKTQLQLEHLLLDLQMILNGINNYKNPKLTRMLTAKFYMPKKATELKHLQCLEEELKPLEEVLNLAQSKNFHLRPRDLISNINVIVLELKGSETTFMCEYADETATIVEFLNRWITFSQSIISTLT

SEQ ID NO: 87 - protein, 376 aa, Artificial Sequence
  source: /note="Description of Artificial Sequence: Synthetic polypeptide"
ESKYGPPCPPCPAPEAAGGPSVFLFPPKPKDTLMISRTPEVTCVVVDVSQEDPEVQFNWYVDGVEVHNAKTKPREEQFNSTYRVVSVLTVLHQDWLNGKEYKCKVSNKGLPSSIEKTISKAKGQPREPQVYTLPPSQEEMTKNQVSLWCLVKGFYPSDIAVEWESNGQPENNYKTTPPVLDSDGSFFLYSRLTVDKSRWQEGNVFSCSVMHEALHNHYTQKSLSLSLGGGGGSGGGGSGGGGSGGGGSSTKKTQLQLEHLLLDLQMILNGINNYKNPKLTRMLTFKFGMPKKATELKHLQCLEEELKPLEEVLNLAQSKNFHLRPRDLISNINVIVLELKGSETTFMCEYADETATIVEFLNRWITFSQSIISTLT

SEQ ID NO: 88 - protein, 376 aa, Artificial Sequence
  source: /note="Description of Artificial Sequence: Synthetic polypeptide"
ESKYGPPCPPCPAPEAAGGPSVFLFPPKPKDTLMISRTPEVTCVVVDVSQEDPEVQFNWYVDGVEVHNAKTKPREEQFNSTYRVVSVLTVLHQDWLNGKEYKCKVSNKGLPSSIEKTISKAKGQPREPQVYTLPPSQEEMTKNQVSLWCLVKGFYPSDIAVEWESNGQPENNYKTTPPVLDSDGSFFLYSRLTVDKSRWQEGNVFSCSVMHEALHNHYTQKSLSLSLGGGGGSGGGGSGGGGSGGGGSSTKKTQLQLEHLLLDLQMILNGINNYKNPKLTRMLTFKFAMPKKATELKHLQCLEEELKPLEEVLNLAQSKNFHLRPRDLISNINVIVLELKGSETTFMCEYADETATIVEFLNRWITFSQSIISTLT

SEQ ID NO: 89 - protein, 376 aa, Artificial Sequence
  source: /note="Description of Artificial Sequence: Synthetic polypeptide"
ESKYGPPCPPCPAPEAAGGPSVFLFPPKPKDTLMISRTPEVTCVVVDVSQEDPEVQFNWYVDGVEVHNAKTKPREEQFNSTYRVVSVLTVLHQDWLNGKEYKCKVSNKGLPSSIEKTISKAKGQPREPQVYTLPPSQEEMTKNQVSLWCLVKGFYPSDIAVEWESNGQPENNYKTTPPVLDSDGSFFLYSRLTVDKSRWQEGNVFSCSVMHEALHNHYTQKSLSLSLGGGGGSGGGGSGGGGSGGGGSSTKKTQLQLEHLLLDLQMILNGINNYKNPKLTRMLTFKFYMPKKATELKHLQCLEAELKPLEEVLNLAQSKNFHLRPRDLISNINVIVLELKGSETTFMCEYADETATIVEFLNRWITFSQSIISTLT

SEQ ID NO: 90 - protein, 376 aa, Artificial Sequence
  source: /note="Description of Artificial Sequence: Synthetic polypeptide"
ESKYGPPCPPCPAPEAAGGPSVFLFPPKPKDTLMISRTPEVTCVVVDVSQEDPEVQFNWYVDGVEVHNAKTKPREEQFNSTYRVVSVLTVLHQDWLNGKEYKCKVSNKGLPSSIEKTISKAKGQPREPQVYTLPPSQEEMTKNQVSLWCLVKGFYPSDIAVEWESNGQPENNYKTTPPVLDSDGSFFLYSRLTVDKSRWQEGNVFSCSVMHEALHNHYTQKSLSLSLGGGGGSGGGGSGGGGSGGGGSSTKKTQLQLEHLLLDLQMILNGINNYKNPKLTRMLTFKFYMPKKATELKHLQCLEEALKPLEEVLNLAQSKNFHLRPRDLISNINVIVLELKGSETTFMCEYADETATIVEFLNRWITFSQSIISTLT

SEQ ID NO: 91 - protein, 376 aa, Artificial Sequence
  source: /note="Description of Artificial Sequence: Synthetic polypeptide"
ESKYGPPCPPCPAPEAAGGPSVFLFPPKPKDTLMISRTPEVTCVVVDVSQEDPEVQFNWYVDGVEVHNAKTKPREEQFNSTYRVVSVLTVLHQDWLNGKEYKCKVSNKGLPSSIEKTISKAKGQPREPQVYTLPPSQEEMTKNQVSLWCLVKGFYPSDIAVEWESNGQPENNYKTTPPVLDSDGSFFLYSRLTVDKSRWQEGNVFSCSVMHEALHNHYTQKSLSLSLGGGGGSGGGGSGGGGSGGGGSSTKKTQLQLEHLLLDLQMILNGINNYKNPKLTRMLTFKFYMPKKATELKHLQCLEEELKPLEAVLNLAQSKNFHLRPRDLISNINVIVLELKGSETTFMCEYADETATIVEFLNRWITFSQSIISTLT

SEQ ID NO: 92 - protein, 376 aa, Artificial Sequence
  source: /note="Description of Artificial Sequence: Synthetic polypeptide"
ESKYGPPCPPCPAPEAAGGPSVFLFPPKPKDTLMISRTPEVTCVVVDVSQEDPEVQFNWYVDGVEVHNAKTKPREEQFNSTYRVVSVLTVLHQDWLNGKEYKCKVSNKGLPSSIEKTISKAKGQPREPQVYTLPPSQEEMTKNQVSLWCLVKGFYPSDIAVEWESNGQPENNYKTTPPVLDSDGSFFLYSRLTVDKSRWQEGNVFSCSVMHEALHNHYTQKSLSLSLGGGGGSGGGGSGGGGSGGGGSSTKKTQLQLEHLLLDLQMILNGINNYKNPKLTRMLTFKFYMPKKATELKHLQCLEEELKPLEEVLNGAQSKNFHLRPRDLISNINVIVLELKGSETTFMCEYADETATIVEFLNRWITFSQSIISTLT

SEQ ID NO: 93 - protein, 376 aa, Artificial Sequence
  source: /note="Description of Artificial Sequence: Synthetic polypeptide"
ESKYGPPCPPCPAPEAAGGPSVFLFPPKPKDTLMISRTPEVTCVVVDVSQEDPEVQFNWYVDGVEVHNAKTKPREEQFNSTYRVVSVLTVLHQDWLNGKEYKCKVSNKGLPSSIEKTISKAKGQPREPQVYTLPPSQEEMTKNQVSLWCLVKGFYPSDIAVEWESNGQPENNYKTTPPVLDSDGSFFLYSRLTVDKSRWQEGNVFSCSVMHEALHNHYTQKSLSLSLGGGGGSGGGGSGGGGSGGGGSSTKKTQLQLEHLLLDLQMILNGINNYKNPKLTRMLTFKFYMPKKATELKHLQCLEEELKPLEEVLNLAGSKNFHLRPRDLISNINVIVLELKGSETTFMCEYADETATIVEFLNRWITFSQSIISTLT

SEQ ID NO: 94 - protein, 376 aa, Artificial Sequence
  source: /note="Description of Artificial Sequence: Synthetic polypeptide"
ESKYGPPCPPCPAPEAAGGPSVFLFPPKPKDTLMISRTPEVTCVVVDVSQEDPEVQFNWYVDGVEVHNAKTKPREEQFNSTYRVVSVLTVLHQDWLNGKEYKCKVSNKGLPSSIEKTISKAKGQPREPQVYTLPPSQEEMTKNQVSLWCLVKGFYPSDIAVEWESNGQPENNYKTTPPVLDSDGSFFLYSRLTVDKSRWQEGNVFSCSVMHEALHNHYTQKSLSLSLGGGGGSGGGGSGGGGSGGGGSSTKKTQLQLEHLLLDLQMILNGINNYKNPKLTRMLTFKFYMPKKATELKHLQCLEEELKPLEEVLNLAQSKNFHLRPRDLISNINVIVLELKGSETTFMCEGADETATIVEFLNRWITFSQSIISTLT

SEQ ID NO: 95 - protein, 376 aa, Artificial Sequence
  source: /note="Description of Artificial Sequence: Synthetic polypeptide"
ESKYGPPCPPCPAPEAAGGPSVFLFPPKPKDTLMISRTPEVTCVVVDVSQEDPEVQFNWYVDGVEVHNAKTKPREEQFNSTYRVVSVLTVLHQDWLNGKEYKCKVSNKGLPSSIEKTISKAKGQPREPQVYTLPPSQEEMTKNQVSLWCLVKGFYPSDIAVEWESNGQPENNYKTTPPVLDSDGSFFLYSRLTVDKSRWQEGNVFSCSVMHEALHNHYTQKSLSLSLGGGGGSGGGGSGGGGSGGGGSSTKKTQLQLEHLLLDLQMILNGINNYKNPKLTRMLTFKFYMPKKATELKHLQCLEEELKPLEEVLNLAQSKNFHLRPRDLISNINVIVLELKGSETTFMCEAADETATIVEFLNRWITFSQSIISTLT

SEQ ID NO: 96 - protein, 376 aa, Artificial Sequence
  source: /note="Description of Artificial Sequence: Synthetic polypeptide"
ESKYGPPCPPCPAPEAAGGPSVFLFPPKPKDTLMISRTPEVTCVVVDVSQEDPEVQFNWYVDGVEVHNAKTKPREEQFNSTYRVVSVLTVLHQDWLNGKEYKCKVSNKGLPSSIEKTISKAKGQPREPQVYTLPPSQEEMTKNQVSLWCLVKGFYPSDIAVEWESNGQPENNYKTTPPVLDSDGSFFLYSRLTVDKSRWQEGNVFSCSVMHEALHNHYTQKSLSLSLGGGGGSGGGGSGGGGSGGGGSSTKKTQLQLEHLLLDLQMILNGINNYKNPKLTRMLTFKFGMPKKATELKHLQCLEAELKPLEEVLNLAQSKNFHLRPRDLISNINVIVLELKGSETTFMCEYADETATIVEFLNRWITFSQSIISTLT

SEQ ID NO: 97 - protein, 376 aa, Artificial Sequence
  source: /note="Description of Artificial Sequence: Synthetic polypeptide"
ESKYGPPCPPCPAPEAAGGPSVFLFPPKPKDTLMISRTPEVTCVVVDVSQEDPEVQFNWYVDGVEVHNAKTKPREEQFNSTYRVVSVLTVLHQDWLNGKEYKCKVSNKGLPSSIEKTISKAKGQPREPQVYTLPPSQEEMTKNQVSLWCLVKGFYPSDIAVEWESNGQPENNYKTTPPVLDSDGSFFLYSRLTVDKSRWQEGNVFSCSVMHEALHNHYTQKSLSLSLGGGGGSGGGGSGGGGSGGGGSSTKKTQLQLEHLLLDLQMILNGINNYKNPKLTRMLTFKFGMPKKATELKHLQCLEEALKPLEEVLNLAQSKNFHLRPRDLISNINVIVLELKGSETTFMCEYADETATIVEFLNRWITFSQSIISTLT

SEQ ID NO: 98 - protein, 376 aa, Artificial Sequence
  source: /note="Description of Artificial Sequence: Synthetic polypeptide"
ESKYGPPCPPCPAPEAAGGPSVFLFPPKPKDTLMISRTPEVTCVVVDVSQEDPEVQFNWYVDGVEVHNAKTKPREEQFNSTYRVVSVLTVLHQDWLNGKEYKCKVSNKGLPSSIEKTISKAKGQPREPQVYTLPPSQEEMTKNQVSLWCLVKGFYPSDIAVEWESNGQPENNYKTTPPVLDSDGSFFLYSRLTVDKSRWQEGNVFSCSVMHEALHNHYTQKSLSLSLGGGGGSGGGGSGGGGSGGGGSSTKKTQLQLEHLLLDLQMILNGINNYKNPKLTGMLTFKFGMPKKATELKHLQCLEEELKPLEEVLNLAQSKNFHLRPRDLISNINVIVLELKGSETTFMCEYADETATIVEFLNRWITFSQSIISTLT

SEQ ID NO: 99 - protein, 376 aa, Artificial Sequence
  source: /note="Description of Artificial Sequence: Synthetic polypeptide"
ESKYGPPCPPCPAPEAAGGPSVFLFPPKPKDTLMISRTPEVTCVVVDVSQEDPEVQFNWYVDGVEVHNAKTKPREEQFNSTYRVVSVLTVLHQDWLNGKEYKCKVSNKGLPSSIEKTISKAKGQPREPQVYTLPPSQEEMTKNQVSLWCLVKGFYPSDIAVEWESNGQPENNYKTTPPVLDSDGSFFLYSRLTVDKSRWQEGNVFSCSVMHEALHNHYTQKSLSLSLGGGGGSGGGGSGGGGSGGGGSSTKKTQLQLEHLLLDLQMILNGINNYKNPKLTGMLTFKFYMPKKATELKHLQCLEAELKPLEEVLNLAQSKNFHLRPRDLISNINVIVLELKGSETTFMCEYADETATIVEFLNRWITFSQSIISTLT

SEQ ID NO: 100 - protein, 376 aa, Artificial Sequence
  source: /note="Description of Artificial Sequence: Synthetic polypeptide"
ESKYGPPCPPCPAPEAAGGPSVFLFPPKPKDTLMISRTPEVTCVVVDVSQEDPEVQFNWYVDGVEVHNAKTKPREEQFNSTYRVVSVLTVLHQDWLNGKEYKCKVSNKGLPSSIEKTISKAKGQPREPQVYTLPPSQEEMTKNQVSLWCLVKGFYPSDIAVEWESNGQPENNYKTTPPVLDSDGSFFLYSRLTVDKSRWQEGNVFSCSVMHEALHNHYTQKSLSLSLGGGGGSGGGGSGGGGSGGGGSSTKKTQLQLEHLLLDLQMILNGINNYKNPKLTRMLTAKFYMPKKATELKHLQCLEAELKPLEEVLNLAQSKNFHLRPRDLISNINVIVLELKGSETTFMCEYADETATIVEFLNRWITFSQSIISTLT

SEQ ID NO: 101 - protein, 376 aa, Artificial Sequence
  source: /note="Description of Artificial Sequence: Synthetic polypeptide"
ESKYGPPCPPCPAPEAAGGPSVFLFPPKPKDTLMISRTPEVTCVVVDVSQEDPEVQFNWYVDGVEVHNAKTKPREEQFNSTYRVVSVLTVLHQDWLNGKEYKCKVSNKGLPSSIEKTISKAKGQPREPQVYTLPPSQEEMTKNQVSLWCLVKGFYPSDIAVEWESNGQPENNYKTTPPVLDSDGSFFLYSRLTVDKSRWQEGNVFSCSVMHEALHNHYTQKSLSLSLGGGGGSGGGGSGGGGSGGGGSSTKKTQLQLEHLLLDLQMILNGINNYKNPKLTRMLTAKFGMPKKATELKHLQCLEEELKPLEEVLNLAQSKNFHLRPRDLISNINVIVLELKGSETTFMCEYADETATIVEFLNRWITFSQSIISTLT

SEQ ID NO: 102 - protein, 376 aa, Artificial Sequence
  source: /note="Description of Artificial Sequence: Synthetic polypeptide"
ESKYGPPCPPCPAPEAAGGPSVFLFPPKPKDTLMISRTPEVTCVVVDVSQEDPEVQFNWYVDGVEVHNAKTKPREEQFNSTYRVVSVLTVLHQDWLNGKEYKCKVSNKGLPSSIEKTISKAKGQPREPQVYTLPPSQEEMTKNQVSLWCLVKGFYPSDIAVEWESNGQPENNYKTTPPVLDSDGSFFLYSRLTVDKSRWQEGNVFSCSVMHEALHNHYTQKSLSLSLGGGGGSGGGGSGGGGSGGGGSSTKKTQLQLEHLLLDLQMILNGINNYKNPKLTRMLTFKFGMPKKATELKHLQCLEAALKPLEEVLNLAQSKNFHLRPRDLISNINVIVLELKGSETTFMCEYADETATIVEFLNRWITFSQSIISTLT

SEQ ID NO: 103 - protein, 376 aa, Artificial Sequence
  source: /note="Description of Artificial Sequence: Synthetic polypeptide"
ESKYGPPCPPCPAPEAAGGPSVFLFPPKPKDTLMISRTPEVTCVVVDVSQEDPEVQFNWYVDGVEVHNAKTKPREEQFNSTYRVVSVLTVLHQDWLNGKEYKCKVSNKGLPSSIEKTISKAKGQPREPQVYTLPPSQEEMTKNQVSLWCLVKGFYPSDIAVEWESNGQPENNYKTTPPVLDSDGSFFLYSRLTVDKSRWQEGNVFSCSVMHEALHNHYTQKSLSLSLGGGGGSGGGGSGGGGSGGGGSSTKKTQLQLEHLLLDLQMILNGINNYKNPKLTRMLTFKFYMPKKATELKHLQCLEAALKPLEEVLNLAQSKNFHLRPRDLISNINVIVLELKGSETTFMCEYADETATIVEFLNRWITFSQSIISTLT

SEQ ID NO: 104 - protein, 376 aa, Artificial Sequence
  source: /note="Description of Artificial Sequence: Synthetic polypeptide"
ESKYGPPCPPCPAPEAAGGPSVFLFPPKPKDTLMISRTPEVTCVVVDVSQEDPEVQFNWYVDGVEVHNAKTKPREEQFNSTYRVVSVLTVLHQDWLNGKEYKCKVSNKGLPSSIEKTISKAKGQPREPQVYTLPPSQEEMTKNQVSLWCLVKGFYPSDIAVEWESNGQPENNYKTTPPVLDSDGSFFLYSRLTVDKSRWQEGNVFSCSVMHEALHNHYTQKSLSLSLGGGGGSGGGGSGGGGSGGGGSSTKKTQLQLEHLLLDLQMILNGINNYKNPKLTGMLTAKFYMPKKATELKHLQCLEEELKPLEEVLNLAQSKNFHLRPRDLISNINVIVLELKGSETTFMCEYADETATIVEFLNRWITFSQSIISTLT

SEQ ID NO: 105 - protein, 376 aa, Artificial Sequence
  source: /note="Description of Artificial Sequence: Synthetic polypeptide"
ESKYGPPCPPCPAPEAAGGPSVFLFPPKPKDTLMISRTPEVTCVVVDVSQEDPEVQFNWYVDGVEVHNAKTKPREEQFNSTYRVVSVLTVLHQDWLNGKEYKCKVSNKGLPSSIEKTISKAKGQPREPQVYTLPPSQEEMTKNQVSLWCLVKGFYPSDIAVEWESNGQPENNYKTTPPVLDSDGSFFLYSRLTVDKSRWQEGNVFSCSVMHEALHNHYTQKSLSLSLGGGGGSGGGGSGGGGSGGGGSSTKKTQLQLEHLLLDLQMILNGINNYKNPKLTRMLTAKFAMPKKATELKHLQCLEEELKPLEEVLNGAQSKNFHLRPRDLISNINVIVLELKGSETTFMCEYADETATIVEFLNRWITFSQSIISTLT

SEQ ID NO: 106 - protein, 376 aa, Artificial Sequence
  source: /note="Description of Artificial Sequence: Synthetic polypeptide"
ESKYGPPCPPCPAPEAAGGPSVFLFPPKPKDTLMISRTPEVTCVVVDVSQEDPEVQFNWYVDGVEVHNAKTKPREEQFNSTYRVVSVLTVLHQDWLNGKEYKCKVSNKGLPSSIEKTISKAKGQPREPQVYTLPPSQEEMTKNQVSLWCLVKGFYPSDIAVEWESNGQPENNYKTTPPVLDSDGSFFLYSRLTVDKSRWQEGNVFSCSVMHEALHNHYTQKSLSLSLGGGGGSGGGGSGGGGSGGGGSSTKKTQLQLEHLLLDLQMILNGINNYKNPKLTGMLTAKFGMPKKATELKHLQCLEEELKPLEEVLNLAQSKNFHLRPRDLISNINVIVLELKGSETTFMCEYADETATIVEFLNRWITFSQSIISTLT

SEQ ID NO: 107 - protein, 376 aa, Artificial Sequence; identical to SEQ ID NO: 80
  source: /note="Description of Artificial Sequence: Synthetic polypeptide"

SEQ ID NO: 108 - protein, 376 aa, Artificial Sequence
  source: /note="Description of Artificial Sequence: Synthetic polypeptide"
ESKYGPPCPPCPAPEAAGGPSVFLFPPKPKDTLMISRTPEVTCVVVDVSQEDPEVQFNWYVDGVEVHNAKTKPREEQFNSTYRVVSVLTVLHQDWLNGKEYKCKVSNKGLPSSIEKTISKAKGQPREPQVYTLPPSQEEMTKNQVSLWCLVKGFYPSDIAVEWESNGQPENNYKTTPPVLDSDGSFFLYSRLTVDKSRWQEGNVFSCSVMHEALHNHYTQKSLSLSLGGGGGSGGGGSGGGGSGGGGSSTKKTQLQLEHLLLDLQMILNGINNYKNPKLTRMLTAKFGMPKKATELKHLQCLEEALKPLEEVLNLAQSKNFHLRPRDLISNINVIVLELKGSETTFMCEYADETATIVEFLNRWITFSQSIISTLT

SEQ ID NO: 109 - protein, 376 aa, Artificial Sequence
  source: /note="Description of Artificial Sequence: Synthetic polypeptide"
ESKYGPPCPPCPAPEAAGGPSVFLFPPKPKDTLMISRTPEVTCVVVDVSQEDPEVQFNWYVDGVEVHNAKTKPREEQFNSTYRVVSVLTVLHQDWLNGKEYKCKVSNKGLPSSIEKTISKAKGQPREPQVYTLPPSQEEMTKNQVSLWCLVKGFYPSDIAVEWESNGQPENNYKTTPPVLDSDGSFFLYSRLTVDKSRWQEGNVFSCSVMHEALHNHYTQKSLSLSLGGGGGSGGGGSGGGGSGGGGSSTKKTQLQLEHLLLDLQMILNGINNYKNPKLTRMLTAKFGMPKKATELKHLQCLEAELKPLEEVLNLAQSKNFHLRPRDLISNINVIVLELKGSETTFMCEYADETATIVEFLNRWITFSQSIISTLT

SEQ ID NO: 110 - protein, 376 aa, Artificial Sequence
  source: /note="Description of Artificial Sequence: Synthetic polypeptide"
ESKYGPPCPPCPAPEAAGGPSVFLFPPKPKDTLMISRTPEVTCVVVDVSQEDPEVQFNWYVDGVEVHNAKTKPREEQFNSTYRVVSVLTVLHQDWLNGKEYKCKVSNKGLPSSIEKTISKAKGQPREPQVYTLPPSQEEMTKNQVSLWCLVKGFYPSDIAVEWESNGQPENNYKTTPPVLDSDGSFFLYSRLTVDKSRWQEGNVFSCSVMHEALHNHYTQKSLSLSLGGGGGSGGGGSGGGGSGGGGSSTKKTQLQLEHLLLDLQMILNGINNYKNPKLTGMLTFKFGMPKKATELKHLQCLEAELKPLEEVLNLAQSKNFHLRPRDLISNINVIVLELKGSETTFMCEYADETATIVEFLNRWITFSQSIISTLT

SEQ ID NO: 111 - protein, 376 aa, Artificial Sequence
  source: /note="Description of Artificial Sequence: Synthetic polypeptide"
ESKYGPPCPPCPAPEAAGGPSVFLFPPKPKDTLMISRTPEVTCVVVDVSQEDPEVQFNWYVDGVEVHNAKTKPREEQFNSTYRVVSVLTVLHQDWLNGKEYKCKVSNKGLPSSIEKTISKAKGQPREPQVYTLPPSQEEMTKNQVSLWCLVKGFYPSDIAVEWESNGQPENNYKTTPPVLDSDGSFFLYSRLTVDKSRWQEGNVFSCSVMHEALHNHYTQKSLSLSLGGGGGSGGGGSGGGGSGGGGSSTKKTQLQLEHLLLDLQMILNGINNYKNPKLTGMLTAKFYMPKKATELKHLQCLEAELKPLEEVLNLAQSKNFHLRPRDLISNINVIVLELKGSETTFMCEYADETATIVEFLNRWITFSQSIISTLT

SEQ ID NO: 112 - protein, 376 aa, Artificial Sequence
  source: /note="Description of Artificial Sequence: Synthetic polypeptide"
ESKYGPPCPPCPAPEAAGGPSVFLFPPKPKDTLMISRTPEVTCVVVDVSQEDPEVQFNWYVDGVEVHNAKTKPREEQFNSTYRVVSVLTVLHQDWLNGKEYKCKVSNKGLPSSIEKTISKAKGQPREPQVYTLPPSQEEMTKNQVSLWCLVKGFYPSDIAVEWESNGQPENNYKTTPPVLDSDGSFFLYSRLTVDKSRWQEGNVFSCSVMHEALHNHYTQKSLSLSLGGGGGSGGGGSGGGGSGGGGSSTKKTQLQLEHLLLDLQMILNGINNYKNPKLTGMLTFKFGMPKKATELKHLQCLEEALKPLEEVLNLAQSKNFHLRPRDLISNINVIVLELKGSETTFMCEYADETATIVEFLNRWITFSQSIISTLT

SEQ ID NO: 113 - protein, 376 aa, Artificial Sequence
  source: /note="Description of Artificial Sequence: Synthetic polypeptide"
ESKYGPPCPPCPAPEAAGGPSVFLFPPKPKDTLMISRTPEVTCVVVDVSQEDPEVQFNWYVDGVEVHNAKTKPREEQFNSTYRVVSVLTVLHQDWLNGKEYKCKVSNKGLPSSIEKTISKAKGQPREPQVYTLPPSQEEMTKNQVSLWCLVKGFYPSDIAVEWESNGQPENNYKTTPPVLDSDGSFFLYSRLTVDKSRWQEGNVFSCSVMHEALHNHYTQKSLSLSLGGGGGSGGGGSGGGGSGGGGSSTKKTQLQLEHLLLDLQMILNGINNYKNPKLTGMLTFKFYMPKKATELKHLQCLEEALKPLEEVLNLAQSKNFHLRPRDLISNINVIVLELKGSETTFMCEYADETATIVEFLNRWITFSQSIISTLT

SEQ ID NO: 114 - protein, 376 aa, Artificial Sequence
  source: /note="Description of Artificial Sequence: Synthetic polypeptide"
ESKYGPPCPPCPAPEAAGGPSVFLFPPKPKDTLMISRTPEVTCVVVDVSQEDPEVQFNWYVDGVEVHNAKTKPREEQFNSTYRVVSVLTVLHQDWLNGKEYKCKVSNKGLPSSIEKTISKAKGQPREPQVYTLPPSQEEMTKNQVSLWCLVKGFYPSDIAVEWESNGQPENNYKTTPPVLDSDGSFFLYSRLTVDKSRWQEGNVFSCSVMHEALHNHYTQKSLSLSLGGGGGSGGGGSGGGGSGGGGSSTKKTQLQLEHLLLDLQMILNGINNYKNPKLTGMLTAKFYMPKKATELKHLQCLEEALKPLEEVLNLAQSKNFHLRPRDLISNINVIVLELKGSETTFMCEYADETATIVEFLNRWITFSQSIISTLT

SEQ ID NO: 115 - protein, 376 aa, Artificial Sequence
  source: /note="Description of Artificial Sequence: Synthetic polypeptide"
ESKYGPPCPPCPAPEAAGGPSVFLFPPKPKDTLMISRTPEVTCVVVDVSQEDPEVQFNWYVDGVEVHNAKTKPREEQFNSTYRVVSVLTVLHQDWLNGKEYKCKVSNKGLPSSIEKTISKAKGQPREPQVYTLPPSQEEMTKNQVSLWCLVKGFYPSDIAVEWESNGQPENNYKTTPPVLDSDGSFFLYSRLTVDKSRWQEGNVFSCSVMHEALHNHYTQKSLSLSLGGGGGSGGGGSGGGGSGGGGSSTKKTQLQLEHLLLDLQMILNGINNYKNPKLTRMLTAKFYMPKKATELKHLQCLEAALKPLEEVLNLAQSKNFHLRPRDLISNINVIVLELKGSETTFMCEYADETATIVEFLNRWITFSQSIISTLT

SEQ ID NO: 116 - protein, 376 aa, Artificial Sequence
  source: /note="Description of Artificial Sequence: Synthetic polypeptide"
ESKYGPPCPPCPAPEAAGGPSVFLFPPKPKDTLMISRTPEVTCVVVDVSQEDPEVQFNWYVDGVEVHNAKTKPREEQFNSTYRVVSVLTVLHQDWLNGKEYKCKVSNKGLPSSIEKTISKAKGQPREPQVYTLPPSQEEMTKNQVSLWCLVKGFYPSDIAVEWESNGQPENNYKTTPPVLDSDGSFFLYSRLTVDKSRWQEGNVFSCSVMHEALHNHYTQKSLSLSLGGGGGSGGGGSGGGGSGGGGSSTKKTQLQLEHLLLDLQMILNGINNYKNPKLTGMLTFKFYMPKKATELKHLQCLEAALKPLEEVLNLAQSKNFHLRPRDLISNINVIVLELKGSETTFMCEYADETATIVEFLNRWITFSQSIISTLT

SEQ ID NO: 117 - protein, 376 aa, Artificial Sequence; identical to SEQ ID NO: 75
  source: /note="Description of Artificial Sequence: Synthetic polypeptide"

SEQ ID NO: 118 - protein, 381 aa, Artificial Sequence
  source: /note="Description of Artificial Sequence: Synthetic polypeptide"
ESKYGPPCPPCPAPEAAGGPSVFLFPPKPKDTLMISRTPEVTCVVVDVSQEDPEVQFNWYVDGVEVHNAKTKPREEQFNSTYRVVSVLTVLHQDWLNGKEYKCKVSNKGLPSSIEKTISKAKGQPREPQVYTLPPSQEEMTKNQVSLWCLVKGFYPSDIAVEWESNGQPENNYKTTPPVLDSDGSFFLYSRLTVDKSRWQEGNVFSCSVMHEALHNHYTQKSLSLSLGGGGGSGGGGSGGGGSGGGGSAPASSSTKKTQLQLEHLLLDLQMILNGINNYKNPKLTRMLTFKFYMPKKATELKHLQCLEEELKPLEEVLNLAQSKNFHLRPRDLISNINVIVLELKGSETTFMCEYADETATIVEFLNRWITFSQSIISTLT

SEQ ID NO: 119 - protein, 379 aa, Artificial Sequence
  source: /note="Description of Artificial Sequence: Synthetic polypeptide"
  VARIANT (284)..(284): /replace="S" or "G" or "A"
  VARIANT (287)..(287): /replace="G" or "A"
  VARIANT (288)..(288): /replace="G" or "A"
  VARIANT (291)..(291): /replace="G" or "A"
  VARIANT (307)..(307): /replace="G" or "A"
  VARIANT (308)..(308): /replace="G" or "A"
  VARIANT (314)..(314): /replace="G" or "A"
  VARIANT (318)..(318): /replace="G" or "A"
  VARIANT (320)..(320): /replace="G" or "A"
  VARIANT (353)..(353): /replace="G" or "A"
  SITE (1)..(379): /note="Variant residues given in the sequence have no preference with respect to those in the annotations for variant positions"
EPKSSDKTHTCPPCPAPEAAGGPSVFLFPPKPKDTLMISRTPEVTCVVVDVSHEDPEVKFNWYVDGVEVHNAKTKPREEQYNSTYRVVSVLTVLHQDWLNGKEYKCKVSNKALPASIEKTISKAKGQPREPQVYTLPPSREEMTKNQVSLWCLVKGFYPSDIAVEWESNGQPENNYKTTPPVLDSDGSFFLYSKLTVDKSRWQQGNVFSCSVMHEALHNHYTQKSLSLSPGGGGGSGGGGSGGGGSGGGGSSTKKTQLQLEHLLLDLQMILNGINNYKNPKLTRMLTFKFYMPKKATELKHLQCLEEELKPLEEVLNLAQSKNFHLRPRDLISNINVIVLELKGSETTFMCEYADETATIVEFLNRWITFSQSIISTLT

SEQ ID NO: 120 - protein, 379 aa, Artificial Sequence; identical to SEQ ID NO: 119
  source: /note="Description of Artificial Sequence: Synthetic polypeptide"
  VARIANT (284)..(284): /replace="S" or "G" or "A"
  VARIANT (288)..(288): /replace="G" or "A"
  VARIANT (291)..(291): /replace="G" or "A"
  VARIANT (307)..(307): /replace="G" or "A"
  VARIANT (308)..(308): /replace="G" or "A"
  VARIANT (318)..(318): /replace="G" or "A"
  SITE (1)..(379): /note="Variant residues given in the sequence have no preference with respect to those in the annotations for variant positions"

SEQ ID NO: 121 - protein, 379 aa, Artificial Sequence; identical to SEQ ID NO: 119
  source: /note="Description of Artificial Sequence: Synthetic polypeptide"
  VARIANT (284)..(284): /replace="S" or "G" or "A"
  VARIANT (288)..(288): /replace="G" or "A"
  VARIANT (291)..(291): /replace="G" or "A"
  VARIANT (307)..(307): /replace="G" or "A"
  VARIANT (308)..(308): /replace="G" or "A"
  SITE (1)..(379): /note="Variant residues given in the sequence have no preference with respect to those in the annotations for variant positions"

SEQ ID NO: 122 - protein, 379 aa, Artificial Sequence; identical to SEQ ID NO: 119
  source: /note="Description of Artificial Sequence: Synthetic polypeptide"
  VARIANT (284)..(284): /replace="S" or "G" or "A"
  VARIANT (288)..(288): /replace="G" or "A"
  VARIANT (291)..(291): /replace="G" or "A"
  VARIANT (308)..(308): /replace="G" or "A"
  SITE (1)..(379): /note="Variant residues given in the sequence have no preference with respect to those in the annotations for variant positions"

SEQ ID NO: 123 - protein, 379 aa, Artificial Sequence; identical to SEQ ID NO: 119
  source: /note="Description of Artificial Sequence: Synthetic polypeptide"
  VARIANT (284)..(284): /replace="S" or "G" or "A"
  VARIANT (288)..(288): /replace="G" or "A"
  VARIANT (308)..(308): /replace="G" or "A"
  SITE (1)..(379): /note="Variant residues given in the sequence have no preference with respect to those in the annotations for variant positions"

SEQ ID NO: 124 - protein, 379 aa, Artificial Sequence
  source: /note="Description of Artificial Sequence: Synthetic polypeptide"
  VARIANT (284)..(284): /replace="S" or "G" or "A"
  SITE (1)..(379): /note="Variant residues given in the sequence have no preference with respect to those in the annotations for variant positions"
EPKSSDKTHTCPPCPAPEAAGGPSVFLFPPKPKDTLMISRTPEVTCVVVDVSHEDPEVKFNWYVDGVEVHNAKTKPREEQYNSTYRVVSVLTVLHQDWLNGKEYKCKVSNKALPASIEKTISKAKGQPREPQVYTLPPSREEMTKNQVSLWCLVKGFYPSDIAVEWESNGQPENNYKTTPPVLDSDGSFFLYSKLTVDKSRWQQGNVFSCSVMHEALHNHYTQKSLSLSPGGGGGSGGGGSGGGGSGGGGSSTKKTQLQLEHLLLDLQMILNGINNYKNPKLTRMLTAKFYMPKKATELKHLQCLEEALKPLEEVLNLAQSKNFHLRPRDLISNINVIVLELKGSETTFMCEYADETATIVEFLNRWITFSQSIISTLT

SEQ ID NO: 125 - protein, 379 aa, Artificial Sequence
  source: /note="Description of Artificial Sequence: Synthetic polypeptide"
EPKSSDKTHTCPPCPAPEAAGGPSVFLFPPKPKDTLMISRTPEVTCVVVDVSHEDPEVKFNWYVDGVEVHNAKTKPREEQYNSTYRVVSVLTVLHQDWLNGKEYKCKVSNKALPASIEKTISKAKGQPREPQVYTLPPSREEMTKNQVSLWCLVKGFYPSDIAVEWESNGQPENNYKTTPPVLDSDGSFFLYSKLTVDKSRWQQGNVFSCSVMHEALHNHYTQKSLSLSPGGGGGSGGGGSGGGGSGGGGSSTKKTQLQLEHLLLDLQMILNGINNYKNPKLTGMLTFKFYMPKKATELKHLQCLEEELKPLEEVLNLAQSKNFHLRPRDLISNINVIVLELKGSETTFMCEYADETATIVEFLNRWITFSQSIISTLT

SEQ ID NO: 126 - protein, 379 aa, Artificial Sequence
  source: /note="Description of Artificial Sequence: Synthetic polypeptide"
EPKSSDKTHTCPPCPAPEAAGGPSVFLFPPKPKDTLMISRTPEVTCVVVDVSHEDPEVKFNWYVDGVEVHNAKTKPREEQYNSTYRVVSVLTVLHQDWLNGKEYKCKVSNKALPASIEKTISKAKGQPREPQVYTLPPSREEMTKNQVSLWCLVKGFYPSDIAVEWESNGQPENNYKTTPPVLDSDGSFFLYSKLTVDKSRWQQGNVFSCSVMHEALHNHYTQKSLSLSPGGGGGSGGGGSGGGGSGGGGSSTKKTQLQLEHLLLDLQMILNGINNYKNPKLTAMLTFKFYMPKKATELKHLQCLEEELKPLEEVLNLAQSKNFHLRPRDLISNINVIVLELKGSETTFMCEYADETATIVEFLNRWITFSQSIISTLT

SEQ ID NO: 127 - protein, 379 aa, Artificial Sequence
  source: /note="Description of Artificial Sequence: Synthetic polypeptide"
EPKSSDKTHTCPPCPAPEAAGGPSVFLFPPKPKDTLMISRTPEVTCVVVDVSHEDPEVKFNWYVDGVEVHNAKTKPREEQYNSTYRVVSVLTVLHQDWLNGKEYKCKVSNKALPASIEKTISKAKGQPREPQVYTLPPSREEMTKNQVSLWCLVKGFYPSDIAVEWESNGQPENNYKTTPPVLDSDGSFFLYSKLTVDKSRWQQGNVFSCSVMHEALHNHYTQKSLSLSPGGGGGSGGGGSGGGGSGGGGSSTKKTQLQLEHLLLDLQMILNGINNYKNPKLTRMLGFKFYMPKKATELKHLQCLEEELKPLEEVLNLAQSKNFHLRPRDLISNINVIVLELKGSETTFMCEYADETATIVEFLNRWITFSQSIISTLT

SEQ ID NO: 128 - protein, 379 aa, Artificial Sequence
  source: /note="Description of Artificial Sequence: Synthetic polypeptide"
EPKSSDKTHTCPPCPAPEAAGGPSVFLFPPKPKDTLMISRTPEVTCVVVDVSHEDPEVKFNWYVDGVEVHNAKTKPREEQYNSTYRVVSVLTVLHQDWLNGKEYKCKVSNKALPASIEKTISKAKGQPREPQVYTLPPSREEMTKNQVSLWCLVKGFYPSDIAVEWESNGQPENNYKTTPPVLDSDGSFFLYSKLTVDKSRWQQGNVFSCSVMHEALHNHYTQKSLSLSPGGGGGSGGGGSGGGGSGGGGSSTKKTQLQLEHLLLDLQMILNGINNYKNPKLTRMLAFKFYMPKKATELKHLQCLEEELKPLEEVLNLAQSKNFHLRPRDLISNINVIVLELKGSETTFMCEYADETATIVEFLNRWITFSQSIISTLT

SEQ ID NO: 129 - protein, 379 aa, Artificial Sequence
  source: /note="Description of Artificial Sequence: Synthetic polypeptide"
EPKSSDKTHTCPPCPAPEAAGGPSVFLFPPKPKDTLMISRTPEVTCVVVDVSHEDPEVKFNWYVDGVEVHNAKTKPREEQYNSTYRVVSVLTVLHQDWLNGKEYKCKVSNKALPASIEKTISKAKGQPREPQVYTLPPSREEMTKNQVSLWCLVKGFYPSDIAVEWESNGQPENNYKTTPPVLDSDGSFFLYSKLTVDKSRWQQGNVFSCSVMHEALHNHYTQKSLSLSPGGGGGSGGGGSGGGGSGGGGSSTKKTQLQLEHLLLDLQMILNGINNYKNPKLTRMLTGKFYMPKKATELKHLQCLEEELKPLEEVLNLAQSKNFHLRPRDLISNINVIVLELKGSETTFMCEYADETATIVEFLNRWITFSQSIISTLT

SEQ ID NO: 130 - protein, 379 aa, Artificial Sequence
  source: /note="Description of Artificial Sequence: Synthetic polypeptide"
EPKSSDKTHTCPPCPAPEAAGGPSVFLFPPKPKDTLMISRTPEVTCVVVDVSHEDPEVKFNWYVDGVEVHNAKTKPREEQYNSTYRVVSVLTVLHQDWLNGKEYKCKVSNKALPASIEKTISKAKGQPREPQVYTLPPSREEMTKNQVSLWCLVKGFYPSDIAVEWESNGQPENNYKTTPPVLDSDGSFFLYSKLTVDKSRWQQGNVFSCSVMHEALHNHYTQKSLSLSPGGGGGSGGGGSGGGGSGGGGSSTKKTQLQLEHLLLDLQMILNGINNYKNPKLTRMLTAKFYMPKKATELKHLQCLEEELKPLEEVLNLAQSKNFHLRPRDLISNINVIVLELKGSETTFMCEYADETATIVEFLNRWITFSQSIISTLT

SEQ ID NO: 131 - protein, 379 aa, Artificial Sequence
  source: /note="Description of Artificial Sequence: Synthetic polypeptide"
EPKSSDKTHTCPPCPAPEAAGGPSVFLFPPKPKDTLMISRTPEVTCVVVDVSHEDPEVKFNWYVDGVEVHNAKTKPREEQYNSTYRVVSVLTVLHQDWLNGKEYKCKVSNKALPASIEKTISKAKGQPREPQVYTLPPSREEMTKNQVSLWCLVKGFYPSDIAVEWESNGQPENNYKTTPPVLDSDGSFFLYSKLTVDKSRWQQGNVFSCSVMHEALHNHYTQKSLSLSPGGGGGSGGGGSGGGGSGGGGSSTKKTQLQLEHLLLDLQMILNGINNYKNPKLTRMLTFKFGMPKKATELKHLQCLEEELKPLEEVLNLAQSKNFHLRPRDLISNINVIVLELKGSETTFMCEYADETATIVEFLNRWITFSQSIISTLT

SEQ ID NO: 132 - protein, 379 aa, Artificial Sequence
  source: /note="Description of Artificial Sequence: Synthetic polypeptide"
EPKSSDKTHTCPPCPAPEAAGGPSVFLFPPKPKDTLMISRTPEVTCVVVDVSHEDPEVKFNWYVDGVEVHNAKTKPREEQYNSTYRVVSVLTVLHQDWLNGKEYKCKVSNKALPASIEKTISKAKGQPREPQVYTLPPSREEMTKNQVSLWCLVKGFYPSDIAVEWESNGQPENNYKTTPPVLDSDGSFFLYSKLTVDKSRWQQGNVFSCSVMHEALHNHYTQKSLSLSPGGGGGSGGGGSGGGGSGGGGSSTKKTQLQLEHLLLDLQMILNGINNYKNPKLTRMLTFKFAMPKKATELKHLQCLEEELKPLEEVLNLAQSKNFHLRPRDLISNINVIVLELKGSETTFMCEYADETATIVEFLNRWITFSQSIISTLT

SEQ ID NO: 133 - protein, 379 aa, Artificial Sequence
  source: /note="Description of Artificial Sequence: Synthetic polypeptide"
EPKSSDKTHTCPPCPAPEAAGGPSVFLFPPKPKDTLMISRTPEVTCVVVDVSHEDPEVKFNWYVDGVEVHNAKTKPREEQYNSTYRVVSVLTVLHQDWLNGKEYKCKVSNKALPASIEKTISKAKGQPREPQVYTLPPSREEMTKNQVSLWCLVKGFYPSDIAVEWESNGQPENNYKTTPPVLDSDGSFFLYSKLTVDKSRWQQGNVFSCSVMHEALHNHYTQKSLSLSPGGGGGSGGGGSGGGGSGGGGSSTKKTQLQLEHLLLDLQMILNGINNYKNPKLTRMLTFKFYMPKKATELKHLQCLEAELKPLEEVLNLAQSKNFHLRPRDLISNINVIVLELKGSETTFMCEYADETATIVEFLNRWITFSQSIISTLT

SEQ ID NO: 134 - protein, 379 aa, Artificial Sequence
  source: /note="Description of Artificial Sequence: Synthetic polypeptide"
EPKSSDKTHTCPPCPAPEAAGGPSVFLFPPKPKDTLMISRTPEVTCVVVDVSHEDPEVKFNWYVDGVEVHNAKTKPREEQYNSTYRVVSVLTVLHQDWLNGKEYKCKVSNKALPASIEKTISKAKGQPREPQVYTLPPSREEMTKNQVSLWCLVKGFYPSDIAVEWESNGQPENNYKTTPPVLDSDGSFFLYSKLTVDKSRWQQGNVFSCSVMHEALHNHYTQKSLSLSPGGGGGSGGGGSGGGGSGGGGSSTKKTQLQLEHLLLDLQMILNGINNYKNPKLTRMLTFKFYMPKKATELKHLQCLEEALKPLEEVLNLAQSKNFHLRPRDLISNINVIVLELKGSETTFMCEYADETATIVEFLNRWITFSQSIISTLT

SEQ ID NO: 135 - protein, 379 aa, Artificial Sequence
  source: /note="Description of Artificial Sequence: Synthetic polypeptide"
EPKSSDKTHTCPPCPAPEAAGGPSVFLFPPKPKDTLMISRTPEVTCVVVDVSHEDPEVKFNWYVDGVEVHNAKTKPREEQYNSTYRVVSVLTVLHQDWLNGKEYKCKVSNKALPASIEKTISKAKGQPREPQVYTLPPSREEMTKNQVSLWCLVKGFYPSDIAVEWESNGQPENNYKTTPPVLDSDGSFFLYSKLTVDKSRWQQGNVFSCSVMHEALHNHYTQKSLSLSPGGGGGSGGGGSGGGGSGGGGSSTKKTQLQLEHLLLDLQMILNGINNYKNPKLTRMLTFKFYMPKKATELKHLQCLEEELKPLEAVLNLAQSKNFHLRPRDLISNINVIVLELKGSETTFMCEYADETATIVEFLNRWITFSQSIISTLT

SEQ ID NO: 136 - protein, 379 aa, Artificial Sequence
  source: /note="Description of Artificial Sequence: Synthetic polypeptide"
EPKSSDKTHTCPPCPAPEAAGGPSVFLFPPKPKDTLMISRTPEVTCVVVDVSHEDPEVKFNWYVDGVEVHNAKTKPREEQYNSTYRVVSVLTVLHQDWLNGKEYKCKVSNKALPASIEKTISKAKGQPREPQVYTLPPSREEMTKNQVSLWCLVKGFYPSDIAVEWESNGQPENNYKTTPPVLDSDGSFFLYSKLTVDKSRWQQGNVFSCSVMHEALHNHYTQKSLSLSPGGGGGSGGGGSGGGGSGGGGSSTKKTQLQLEHLLLDLQMILNGINNYKNPKLTRMLTFKFYMPKKATELKHLQCLEEELKPLEEVLNGAQSKNFHLRPRDLISNINVIVLELKGSETTFMCEYADETATIVEFLNRWITFSQSIISTLT

SEQ ID NO: 137 - protein, 379 aa, Artificial Sequence
  source: /note="Description of Artificial Sequence: Synthetic polypeptide"
EPKSSDKTHTCPPCPAPEAAGGPSVFLFPPKPKDTLMISRTPEVTCVVVDVSHEDPEVKFNWYVDGVEVHNAKTKPREEQYNSTYRVVSVLTVLHQDWLNGKEYKCKVSNKALPASIEKTISKAKGQPREPQVYTLPPSREEMTKNQVSLWCLVKGFYPSDIAVEWESNGQPENNYKTTPPVLDSDGSFFLYSKLTVDKSRWQQGNVFSCSVMHEALHNHYTQKSLSLSPGGGGGSGGGGSGGGGSGGGGSSTKKTQLQLEHLLLDLQMILNGINNYKNPKLTRMLTFKFYMPKKATELKHLQCLEEELKPLEEVLNLAGSKNFHLRPRDLISNINVIVLELKGSETTFMCEYADETATIVEFLNRWITFSQSIISTLT

SEQ ID NO: 138 - protein, 379 aa, Artificial Sequence
  source: /note="Description of Artificial Sequence: Synthetic polypeptide"
EPKSSDKTHTCPPCPAPEAAGGPSVFLFPPKPKDTLMISRTPEVTCVVVDVSHEDPEVKFNWYVDGVEVHNAKTKPREEQYNSTYRVVSVLTVLHQDWLNGKEYKCKVSNKALPASIEKTISKAKGQPREPQVYTLPPSREEMTKNQVSLWCLVKGFYPSDIAVEWESNGQPENNYKTTPPVLDSDGSFFLYSKLTVDKSRWQQGNVFSCSVMHEALHNHYTQKSLSLSPGGGGGSGGGGSGGGGSGGGGSSTKKTQLQLEHLLLDLQMILNGINNYKNPKLTRMLTFKFYMPKKATELKHLQCLEEELKPLEEVLNLAQSKNFHLRPRDLISNINVIVLELKGSETTFMCEGADETATIVEFLNRWITFSQSIISTLT

SEQ ID NO: 139 - protein, 379 aa, Artificial Sequence
  source: /note="Description of Artificial Sequence: Synthetic polypeptide"
EPKSSDKTHTCPPCPAPEAAGGPSVFLFPPKPKDTLMISRTPEVTCVVVDVSHEDPEVKFNWYVDGVEVHNAKTKPREEQYNSTYRVVSVLTVLHQDWLNGKEYKCKVSNKALPASIEKTISKAKGQPREPQVYTLPPSREEMTKNQVSLWCLVKGFYPSDIAVEWESNGQPENNYKTTPPVLDSDGSFFLYSKLTVDKSRWQQGNVFSCSVMHEALHNHYTQKSLSLSPGGGGGSGGGGSGGGGSGGGGSSTKKTQLQLEHLLLDLQMILNGINNYKNPKLTRMLTFKFYMPKKATELKHLQCLEEELKPLEEVLNLAQSKNFHLRPRDLISNINVIVLELKGSETTFMCEAADETATIVEFLNRWITFSQSIISTLT

SEQ ID NO: 140 - protein, 379 aa, Artificial Sequence
  source: /note="Description of Artificial Sequence: Synthetic polypeptide"
EPKSSDKTHTCPPCPAPEAAGGPSVFLFPPKPKDTLMISRTPEVTCVVVDVSHEDPEVKFNWYVDGVEVHNAKTKPREEQYNSTYRVVSVLTVLHQDWLNGKEYKCKVSNKALPASIEKTISKAKGQPREPQVYTLPPSREEMTKNQVSLWCLVKGFYPSDIAVEWESNGQPENNYKTTPPVLDSDGSFFLYSKLTVDKSRWQQGNVFSCSVMHEALHNHYTQKSLSLSPGGGGGSGGGGSGGGGSGGGGSSTKKTQLQLEHLLLDLQMILNGINNYKNPKLTRMLTFKFGMPKKATELKHLQCLEAELKPLEEVLNLAQSKNFHLRPRDLISNINVIVLELKGSETTFMCEYADETATIVEFLNRWITFSQSIISTLT

SEQ ID NO: 141 - protein, 379 aa, Artificial Sequence
  source: /note="Description of Artificial Sequence: Synthetic polypeptide"
EPKSSDKTHTCPPCPAPEAAGGPSVFLFPPKPKDTLMISRTPEVTCVVVDVSHEDPEVKFNWYVDGVEVHNAKTKPREEQYNSTYRVVSVLTVLHQDWLNGKEYKCKVSNKALPASIEKTISKAKGQPREPQVYTLPPSREEMTKNQVSLWCLVKGFYPSDIAVEWESNGQPENNYKTTPPVLDSDGSFFLYSKLTVDKSRWQQGNVFSCSVMHEALHNHYTQKSLSLSPGGGGGSGGGGSGGGGSGGGGSSTKKTQLQLEHLLLDLQMILNGINNYKNPKLTRMLTFKFGMPKKATELKHLQCLEEALKPLEEVLNLAQSKNFHLRPRDLISNINVIVLELKGSETTFMCEYADETATIVEFLNRWITFSQSIISTLT

SEQ ID NO: 142 - protein, 379 aa, Artificial Sequence
  source: /note="Description of Artificial Sequence: Synthetic polypeptide"
EPKSSDKTHTCPPCPAPEAAGGPSVFLFPPKPKDTLMISRTPEVTCVVVDVSHEDPEVKFNWYVDGVEVHNAKTKPREEQYNSTYRVVSVLTVLHQDWLNGKEYKCKVSNKALPASIEKTISKAKGQPREPQVYTLPPSREEMTKNQVSLWCLVKGFYPSDIAVEWESNGQPENNYKTTPPVLDSDGSFFLYSKLTVDKSRWQQGNVFSCSVMHEALHNHYTQKSLSLSPGGGGGSGGGGSGGGGSGGGGSSTKKTQLQLEHLLLDLQMILNGINNYKNPKLTGMLTFKFGMPKKATELKHLQCLEEELKPLEEVLNLAQSKNFHLRPRDLISNINVIVLELKGSETTFMCEYADETATIVEFLNRWITFSQSIISTLT

SEQ ID NO: 143 - protein, 379 aa, Artificial Sequence
  source: /note="Description of Artificial Sequence: Synthetic polypeptide"
EPKSSDKTHTCPPCPAPEAAGGPSVFLFPPKPKDTLMISRTPEVTCVVVDVSHEDPEVKFNWYVDGVEVHNAKTKPREEQYNSTYRVVSVLTVLHQDWLNGKEYKCKVSNKALPASIEKTISKAKGQPREPQVYTLPPSREEMTKNQVSLWCLVKGFYPSDIAVEWESNGQPENNYKTTPPVLDSDGSFFLYSKLTVDKSRWQQGNVFSCSVMHEALHNHYTQKSLSLSPGGGGGSGGGGSGGGGSGGGGSSTKKTQLQLEHLLLDLQMILNGINNYKNPKLTGMLTFKFYMPKKATELKHLQCLEAELKPLEEVLNLAQSKNFHLRPRDLISNINVIVLELKGSETTFMCEYADETATIVEFLNRWITFSQSIISTLT

SEQ ID NO: 144 - protein, 379 aa, Artificial Sequence
  source: /note="Description of Artificial Sequence: Synthetic polypeptide"
EPKSSDKTHTCPPCPAPEAAGGPSVFLFPPKPKDTLMISRTPEVTCVVVDVSHEDPEVKFNWYVDGVEVHNAKTKPREEQYNSTYRVVSVLTVLHQDWLNGKEYKCKVSNKALPASIEKTISKAKGQPREPQVYTLPPSREEMTKNQVSLWCLVKGFYPSDIAVEWESNGQPENNYKTTPPVLDSDGSFFLYSKLTVDKSRWQQGNVFSCSVMHEALHNHYTQKSLSLSPGGGGGSGGGGSGGGGSGGGGSSTKKTQLQLEHLLLDLQMILNGINNYKNPKLTRMLTAKFYMPKKATELKHLQCLEAELKPLEEVLNLAQSKNFHLRPRDLISNINVIVLELKGSETTFMCEYADETATIVEFLNRWITFSQSIISTLT

SEQ ID NO: 145 - protein, 379 aa, Artificial Sequence
  source: /note="Description of Artificial Sequence: Synthetic polypeptide"
EPKSSDKTHTCPPCPAPEAAGGPSVFLFPPKPKDTLMISRTPEVTCVVVDVSHEDPEVKFNWYVDGVEVHNAKTKPREEQYNSTYRVVSVLTVLHQDWLNGKEYKCKVSNKALPASIEKTISKAKGQPREPQVYTLPPSREEMTKNQVSLWCLVKGFYPSDIAVEWESNGQPENNYKTTPPVLDSDGSFFLYSKLTVDKSRWQQGNVFSCSVMHEALHNHYTQKSLSLSPGGGGGSGGGGSGGGGSGGGGSSTKKTQLQLEHLLLDLQMILNGINNYKNPKLTRMLTAKFGMPKKATELKHLQCLEEELKPLEEVLNLAQSKNFHLRPRDLISNINVIVLELKGSETTFMCEYADETATIVEFLNRWITFSQSIISTLT

SEQ ID NO: 146 - protein, 379 aa, Artificial Sequence
  source: /note="Description of Artificial Sequence: Synthetic polypeptide"
EPKSSDKTHTCPPCPAPEAAGGPSVFLFPPKPKDTLMISRTPEVTCVVVDVSHEDPEVKFNWYVDGVEVHNAKTKPREEQYNSTYRVVSVLTVLHQDWLNGKEYKCKVSNKALPASIEKTISKAKGQPREPQVYTLPPSREEMTKNQVSLWCLVKGFYPSDIAVEWESNGQPENNYKTTPPVLDSDGSFFLYSKLTVDKSRWQQGNVFSCSVMHEALHNHYTQKSLSLSPGGGGGSGGGGSGGGGSGGGGSSTKKTQLQLEHLLLDLQMILNGINNYKNPKLTRMLTFKFGMPKKATELKHLQCLEAALKPLEEVLNLAQSKNFHLRPRDLISNINVIVLELKGSETTFMCEYADETATIVEFLNRWITFSQSIISTLT

SEQ ID NO: 147 - protein, 379 aa, Artificial Sequence
  source: /note="Description of Artificial Sequence: Synthetic polypeptide"
EPKSSDKTHTCPPCPAPEAAGGPSVFLFPPKPKDTLMISRTPEVTCVVVDVSHEDPEVKFNWYVDGVEVHNAKTKPREEQYNSTYRVVSVLTVLHQDWLNGKEYKCKVSNKALPASIEKTISKAKGQPREPQVYTLPPSREEMTKNQVSLWCLVKGFYPSDIAVEWESNGQPENNYKTTPPVLDSDGSFFLYSKLTVDKSRWQQGNVFSCSVMHEALHNHYTQKSLSLSPGGGGGSGGGGSGGGGSGGGGSSTKKTQLQLEHLLLDLQMILNGINNYKNPKLTRMLTFKFYMPKKATELKHLQCLEAALKPLEEVLNLAQSKNFHLRPRDLISNINVIVLELKGSETTFMCEYADETATIVEFLNRWITFSQSIISTLT

SEQ ID NO: 148 - protein, 379 aa, Artificial Sequence
  source: /note="Description of Artificial Sequence: Synthetic polypeptide"
EPKSSDKTHTCPPCPAPEAAGGPSVFLFPPKPKDTLMISRTPEVTCVVVDVSHEDPEVKFNWYVDGVEVHNAKTKPREEQYNSTYRVVSVLTVLHQDWLNGKEYKCKVSNKALPASIEKTISKAKGQPREPQVYTLPPSREEMTKNQVSLWCLVKGFYPSDIAVEWESNGQPENNYKTTPPVLDSDGSFFLYSKLTVDKSRWQQGNVFSCSVMHEALHNHYTQKSLSLSPGGGGGSGGGGSGGGGSGGGGSSTKKTQLQLEHLLLDLQMILNGINNYKNPKLTGMLTAKFYMPKKATELKHLQCLEEELKPLEEVLNLAQSKNFHLRPRDLISNINVIVLELKGSETTFMCEYADETATIVEFLNRWITFSQSIISTLT

SEQ ID NO: 149 - protein, 379 aa, Artificial Sequence
  source: /note="Description of Artificial Sequence: Synthetic polypeptide"
EPKSSDKTHTCPPCPAPEAAGGPSVFLFPPKPKDTLMISRTPEVTCVVVDVSHEDPEVKFNWYVDGVEVHNAKTKPREEQYNSTYRVVSVLTVLHQDWLNGKEYKCKVSNKALPASIEKTISKAKGQPREPQVYTLPPSREEMTKNQVSLWCLVKGFYPSDIAVEWESNGQPENNYKTTPPVLDSDGSFFLYSKLTVDKSRWQQGNVFSCSVMHEALHNHYTQKSLSLSPGGGGGSGGGGSGGGGSGGGGSSTKKTQLQLEHLLLDLQMILNGINNYKNPKLTRMLTAKFAMPKKATELKHLQCLEEELKPLEEVLNGAQSKNFHLRPRDLISNINVIVLELKGSETTFMCEYADETATIVEFLNRWITFSQSIISTLT

SEQ ID NO: 150 - protein, 379 aa, Artificial Sequence
  source: /note="Description of Artificial Sequence: Synthetic polypeptide"
EPKSSDKTHTCPPCPAPEAAGGPSVFLFPPKPKDTLMISRTPEVTCVVVDVSHEDPEVKFNWYVDGVEVHNAKTKPREEQYNSTYRVVSVLTVLHQDWLNGKEYKCKVSNKALPASIEKTISKAKGQPREPQVYTLPPSREEMTKNQVSLWCLVKGFYPSDIAVEWESNGQPENNYKTTPPVLDSDGSFFLYSKLTVDKSRWQQGNVFSCSVMHEALHNHYTQKSLSLSPGGGGGSGGGGSGGGGSGGGGSSTKKTQLQLEHLLLDLQMILNGINNYKNPKLTGMLTAKFGMPKKATELKHLQCLEEELKPLEEVLNLAQSKNFHLRPRDLISNINVIVLELKGSETTFMCEYADETATIVEFLNRWITFSQSIISTLT

SEQ ID NO: 151 - protein, 379 aa, Artificial Sequence; identical to SEQ ID NO: 124
  source: /note="Description of Artificial Sequence: Synthetic polypeptide"

SEQ ID NO: 152 - protein, 379 aa, Artificial Sequence
  source: /note="Description of Artificial Sequence: Synthetic polypeptide"
EPKSSDKTHTCPPCPAPEAAGGPSVFLFPPKPKDTLMISRTPEVTCVVVDVSHEDPEVKFNWYVDGVEVHNAKTKPREEQYNSTYRVVSVLTVLHQDWLNGKEYKCKVSNKALPASIEKTISKAKGQPREPQVYTLPPSREEMTKNQVSLWCLVKGFYPSDIAVEWESNGQPENNYKTTPPVLDSDGSFFLYSKLTVDKSRWQQGNVFSCSVMHEALHNHYTQKSLSLSPGGGGGSGGGGSGGGGSGGGGSSTKKTQLQLEHLLLDLQMILNGINNYKNPKLTRMLTAKFGMPKKATELKHLQCLEEALKPLEEVLNLAQSKNFHLRPRDLISNINVIVLELKGSETTFMCEYADETATIVEFLNRWITFSQSIISTLT

SEQ ID NO: 153 - protein, 379 aa, Artificial Sequence
  source: /note="Description of Artificial Sequence: Synthetic polypeptide"
EPKSSDKTHTCPPCPAPEAAGGPSVFLFPPKPKDTLMISRTPEVTCVVVDVSHEDPEVKFNWYVDGVEVHNAKTKPREEQYNSTYRVVSVLTVLHQDWLNGKEYKCKVSNKALPASIEKTISKAKGQPREPQVYTLPPSREEMTKNQVSLWCLVKGFYPSDIAVEWESNGQPENNYKTTPPVLDSDGSFFLYSKLTVDKSRWQQGNVFSCSVMHEALHNHYTQKSLSLSPGGGGGSGGGGSGGGGSGGGGSSTKKTQLQLEHLLLDLQMILNGINNYKNPKLTRMLTAKFGMPKKATELKHLQCLEAELKPLEEVLNLAQSKNFHLRPRDLISNINVIVLELKGSETTFMCEYADETATIVEFLNRWITFSQSIISTLT

SEQ ID NO: 154 - protein, 379 aa, Artificial Sequence
  source: /note="Description of Artificial Sequence: Synthetic polypeptide"
EPKSSDKTHTCPPCPAPEAAGGPSVFLFPPKPKDTLMISRTPEVTCVVVDVSHEDPEVKFNWYVDGVEVHNAKTKPREEQYNSTYRVVSVLTVLHQDWLNGKEYKCKVSNKALPASIEKTISKAKGQPREPQVYTLPPSREEMTKNQVSLWCLVKGFYPSDIAVEWESNGQPENNYKTTPPVLDSDGSFFLYSKLTVDKSRWQQGNVFSCSVMHEALHNHYTQKSLSLSPGGGGGSGGGGSGGGGSGGGGSSTKKTQLQLEHLLLDLQMILNGINNYKNPKLTGMLTFKFGMPKKATELKHLQCLEAELKPLEEVLNLAQSKNFHLRPRDLISNINVIVLELKGSETTFMCEYADETATIVEFLNRWITFSQSIISTLT

SEQ ID NO: 155 - protein, 379 aa, Artificial Sequence
  source: /note="Description of Artificial Sequence: Synthetic polypeptide"
EPKSSDKTHTCPPCPAPEAAGGPSVFLFPPKPKDTLMISRTPEVTCVVVDVSHEDPEVKFNWYVDGVEVHNAKTKPREEQYNSTYRVVSVLTVLHQDWLNGKEYKCKVSNKALPASIEKTISKAKGQPREPQVYTLPPSREEMTKNQVSLWCLVKGFYPSDIAVEWESNGQPENNYKTTPPVLDSDGSFFLYSKLTVDKSRWQQGNVFSCSVMHEALHNHYTQKSLSLSPGGGGGSGGGGSGGGGSGGGGSSTKKTQLQLEHLLLDLQMILNGINNYKNPKLTGMLTAKFYMPKKATELKHLQCLEAELKPLEEVLNLAQSKNFHLRPRDLISNINVIVLELKGSETTFMCEYADETATIVEFLNRWITFSQSIISTLT

SEQ ID NO: 156 - protein, 379 aa, Artificial Sequence
  source: /note="Description of Artificial Sequence: Synthetic polypeptide"
EPKSSDKTHTCPPCPAPEAAGGPSVFLFPPKPKDTLMISRTPEVTCVVVDVSHEDPEVKFNWYVDGVEVHNAKTKPREEQYNSTYRVVSVLTVLHQDWLNGKEYKCKVSNKALPASIEKTISKAKGQPREPQVYTLPPSREEMTKNQVSLWCLVKGFYPSDIAVEWESNGQPENNYKTTPPVLDSDGSFFLYSKLTVDKSRWQQGNVFSCSVMHEALHNHYTQKSLSLSPGGGGGSGGGGSGGGGSGGGGSSTKKTQLQLEHLLLDLQMILNGINNYKNPKLTGMLTFKFGMPKKATELKHLQCLEEALKPLEEVLNLAQSKNFHLRPRDLISNINVIVLELKGSETTFMCEYADETATIVEFLNRWITFSQSIISTLT

SEQ ID NO: 157 - protein, 379 aa, Artificial Sequence
  source: /note="Description of Artificial Sequence: Synthetic polypeptide"
EPKSSDKTHTCPPCPAPEAAGGPSVFLFPPKPKDTLMISRTPEVTCVVVDVSHEDPEVKFNWYVDGVEVHNAKTKPREEQYNSTYRVVSVLTVLHQDWLNGKEYKCKVSNKALPASIEKTISKAKGQPREPQVYTLPPSREEMTKNQVSLWCLVKGFYPSDIAVEWESNGQPENNYKTTPPVLDSDGSFFLYSKLTVDKSRWQQGNVFSCSVMHEALHNHYTQKSLSLSPGGGGGSGGGGSGGGGSGGGGSSTKKTQLQLEHLLLDLQMILNGINNYKNPKLTGMLTFKFYMPKKATELKHLQCLEEALKPLEEVLNLAQSKNFHLRPRDLISNINVIVLELKGSETTFMCEYADETATIVEFLNRWITFSQSIISTLT

SEQ ID NO: 158 - protein, 379 aa, Artificial Sequence
  source: /note="Description of Artificial Sequence: Synthetic polypeptide"
EPKSSDKTHTCPPCPAPEAAGGPSVFLFPPKPKDTLMISRTPEVTCVVVDVSHEDPEVKFNWYVDGVEVHNAKTKPREEQYNSTYRVVSVLTVLHQDWLNGKEYKCKVSNKALPASIEKTISKAKGQPREPQVYTLPPSREEMTKNQVSLWCLVKGFYPSDIAVEWESNGQPENNYKTTPPVLDSDGSFFLYSKLTVDKSRWQQGNVFSCSVMHEALHNHYTQKSLSLSPGGGGGSGGGGSGGGGSGGGGSSTKKTQLQLEHLLLDLQMILNGINNYKNPKLTGMLTAKFYMPKKATELKHLQCLEEALKPLEEVLNLAQSKNFHLRPRDLISNINVIVLELKGSETTFMCEYADETATIVEFLNRWITFSQSIISTLT

SEQ ID NO: 159 - protein, 379 aa, Artificial Sequence
  source: /note="Description of Artificial Sequence: Synthetic polypeptide"
EPKSSDKTHTCPPCPAPEAAGGPSVFLFPPKPKDTLMISRTPEVTCVVVDVSHEDPEVKFNWYVDGVEVHNAKTKPREEQYNSTYRVVSVLTVLHQDWLNGKEYKCKVSNKALPASIEKTISKAKGQPREPQVYTLPPSREEMTKNQVSLWCLVKGFYPSDIAVEWESNGQPENNYKTTPPVLDSDGSFFLYSKLTVDKSRWQQGNVFSCSVMHEALHNHYTQKSLSLSPGGGGGSGGGGSGGGGSGGGGSSTKKTQLQLEHLLLDLQMILNGINNYKNPKLTRMLTAKFYMPKKATELKHLQCLEAALKPLEEVLNLAQSKNFHLRPRDLISNINVIVLELKGSETTFMCEYADETATIVEFLNRWITFSQSIISTLT

SEQ ID NO: 160 - protein, 379 aa, Artificial Sequence
  source: /note="Description of Artificial Sequence: Synthetic polypeptide"
EPKSSDKTHTCPPCPAPEAAGGPSVFLFPPKPKDTLMISRTPEVTCVVVDVSHEDPEVKFNWYVDGVEVHNAKTKPREEQYNSTYRVVSVLTVLHQDWLNGKEYKCKVSNKALPASIEKTISKAKGQPREPQVYTLPPSREEMTKNQVSLWCLVKGFYPSDIAVEWESNGQPENNYKTTPPVLDSDGSFFLYSKLTVDKSRWQQGNVFSCSVMHEALHNHYTQKSLSLSPGGGGGSGGGGSGGGGSGGGGSSTKKTQLQLEHLLLDLQMILNGINNYKNPKLTGMLTFKFYMPKKATELKHLQCLEAALKPLEEVLNLAQSKNFHLRPRDLISNINVIVLELKGSETTFMCEYADETATIVEFLNRWITFSQSIISTLT

SEQ ID NO: 161 - protein, 379 aa, Artificial Sequence; identical to SEQ ID NO: 119
  source: /note="Description of Artificial Sequence: Synthetic polypeptide"

SEQ ID NO: 162 - protein, 379 aa, Artificial Sequence
  source: /note="Description of Artificial Sequence: Synthetic polypeptide"
EPKSSDKTHTCPPCPAPEAAGGPSVFLFPPKPKDTLMISRTPEVTCVVVDVSHEDPEVKFNWYVDGVEVHNAKTKPREEQYNSTYRVVSVLTVLHQDWLNGKEYKCKVSNKALPASIEKTISKAKGQPREPQVYTLPPSREEMTKNQVSLWCLVKGFYPSDIAVEWESNGQPENNYKTTPPVLDSDGSFFLYSKLTVDKSRWQQGNVFSCSVMHEALHNHYTQKSLSLSPGGGGGSGGGGSGGGGSGGGGSSTKKTQLQLEHLLLDLQMILNGINNYKNPKLTRMLTFKFYMPKKATELKHLQCLEEELKPLEEVLNLAQSKNFHLRPRDLISNINVIVLELKGSETTFMCEYADETATIVEFLNRWITFCQSIISTLT

SEQ ID NO: 163 - protein, 5 aa, Artificial Sequence
  source: /note="Description of Artificial Sequence: Synthetic peptide"
APTSS

SEQ ID NO: 164 - skipped

SEQ ID NO: 165 - protein, 375 aa, Artificial Sequence
  source: /note="Description of Artificial Sequence: Synthetic polypeptide"
GPTIKPCPPCKCPAPNAAGGPSVFIFPPKIKDVLMISLSPIVTCVVVDVSEDDPDVQISWFVNNVEVHTAQTQTHREDYNSTLRVVSALPIQHQDWMSGKEFKCKVNNKDLGAPIERTISKPKGSVRAPQVYVLPPPEEEMTKKQVTLWCMVTDFMPEDIYVEWTNNGKTELNYKNTEPVLDSDGSYFMYSKLRVEKKNWVERNSYSCSVVHEGLHNHHTTKSFSRTPGGGGGSGGGGSGGGGSGGGGSQQQHLEQLLMDLQELLSRMENYRNLKLPRMLTFKFYLPKQATELKDLQCLEDELGPLRHVLDLTQSKSFQLEDAENFISNIRVTVVKLKGSDNTFECQFDDESATVVDFLRRWIAFAQSIISTSPQ

SEQ ID NO: 166 - protein, 375 aa, Artificial Sequence
  source: /note="Description of Artificial Sequence: Synthetic polypeptide"
GPTIKPCPPCKCPAPNAAGGPSVFIFPPKIKDVLMISLSPIVTCVVVDVSEDDPDVQISWFVNNVEVHTAQTQTHREDYNSTLRVVSALPIQHQDWMSGKEFKCKVNNKDLGAPIERTISKPKGSVRAPQVYVLPPPEEEMTKKQVTLWCMVTDFMPEDIYVEWTNNGKTELNYKNTEPVLDSDGSYFMYSKLRVEKKNWVERNSYSCSVVHEGLHNHHTTKSFSRTPGGGGGSGGGGSGGGGSGGGGSQQQHLEQLLMDLQELLSRMENYRNLKLPRMLTAKFALPKQATELKDLQCLEDELGPLRHVLDGTQSKSFQLEDAENFISNIRVTVVKLKGSDNTFECQFDDESATVVDFLRRWIAFAQSIISTSPQ

SEQ ID NO: 167 - protein, 375 aa, Artificial Sequence
  source: /note="Description of Artificial Sequence: Synthetic polypeptide"
GPTIKPCPPCKCPAPNAAGGPSVFIFPPKIKDVLMISLSPIVTCVVVDVSEDDPDVQISWFVNNVEVHTAQTQTHREDYNSTLRVVSALPIQHQDWMSGKEFKCKVNNKDLGAPIERTISKPKGSVRAPQVYVLPPPEEEMTKKQVTLWCMVTDFMPEDIYVEWTNNGKTELNYKNTEPVLDSDGSYFMYSKLRVEKKNWVERNSYSCSVVHEGLHNHHTTKSFSRTPGGGGGSGGGGSGGGGSGGGGSQQQHLEQLLMDLQELLSRMENYRNLKLPRMLTAKFYLPKQATELKDLQCLEDELGPLRHVLDLTQSKSFQLEDAENFISNIRVTVVKLKGSDNTFECQFDDESATVVDFLRRWIAFAQSIISTSPQ

SEQ ID NO: 168 - protein, 375 aa, Artificial Sequence
  source: /note="Description of Artificial Sequence: Synthetic polypeptide"
GPTIKPCPPCKCPAPNAAGGPSVFIFPPKIKDVLMISLSPIVTCVVVDVSEDDPDVQISWFVNNVEVHTAQTQTHREDYNSTLRVVSALPIQHQDWMSGKEFKCKVNNKDLGAPIERTISKPKGSVRAPQVYVLPPPEEEMTKKQVTLWCMVTDFMPEDIYVEWTNNGKTELNYKNTEPVLDSDGSYFMYSKLRVEKKNWVERNSYSCSVVHEGLHNHHTTKSFSRTPGGGGGSGGGGSGGGGSGGGGSQQQHLEQLLMDLQELLSRMENYRNLKLPRMLTAKFYLPKQATELKDLQCLEDALGPLRHVLDLTQSKSFQLEDAENFISNIRVTVVKLKGSDNTFECQFDDESATVVDFLRRWIAFAQSIISTSPQ

SEQ ID NO: 169 - protein, 375 aa, Artificial Sequence
  source: /note="Description of Artificial Sequence: Synthetic polypeptide"
GPTIKPCPPCKCPAPNAAGGPSVFIFPPKIKDVLMISLSPIVTCVVVDVSEDDPDVQISWFVNNVEVHTAQTQTHREDYNSTLRVVSALPIQHQDWMSGKEFKCKVNNKDLGAPIERTISKPKGSVRAPQVYVLPPPEEEMTKKQVTLWCMVTDFMPEDIYVEWTNNGKTELNYKNTEPVLDSDGSYFMYSKLRVEKKNWVERNSYSCSVVHEGLHNHHTTKSFSRTPGGGGGSGGGGSGGGGSGGGGSQQQHLEQLLMDLQELLSRMENYRNLKLPRMLTAKFGLPKQATELKDLQCLEDALGPLRHVLDLTQSKSFQLEDAENFISNIRVTVVKLKGSDNTFECQFDDESATVVDFLRRWIAFAQSIISTSPQ

SEQ ID NO: 170 - protein, 375 aa, Artificial Sequence
  source: /note="Description of Artificial Sequence: Synthetic polypeptide"
GPTIKPCPPCKCPAPNAAGGPSVFIFPPKIKDVLMISLSPIVTCVVVDVSEDDPDVQISWFVNNVEVHTAQTQTHREDYNSTLRVVSALPIQHQDWMSGKEFKCKVNNKDLGAPIERTISKPKGSVRAPQVYVLPPPEEEMTKKQVTLWCMVTDFMPEDIYVEWTNNGKTELNYKNTEPVLDSDGSYFMYSKLRVEKKNWVERNSYSCSVVHEGLHNHHTTKSFSRTPGGGGGSGGGGSGGGGSGGGGSQQQHLEQLLMDLQELLSRMENYRNLKLPGMLTFKFYLPKQATELKDLQCLEDALGPLRHVLDLTQSKSFQLEDAENFISNIRVTVVKLKGSDNTFECQFDDESATVVDFLRRWIAFAQSIISTSPQ

SEQ ID NO: 171 - protein, 375 aa, Artificial Sequence
  source: /note="Description of Artificial Sequence: Synthetic polypeptide"
GPTIKPCPPCKCPAPNAAGGPSVFIFPPKIKDVLMISLSPIVTCVVVDVSEDDPDVQISWFVNNVEVHTAQTQTHREDYNSTLRVVSALPIQHQDWMSGKEFKCKVNNKDLGAPIERTISKPKGSVRAPQVYVLPPPEEEMTKKQVTLWCMVTDFMPEDIYVEWTNNGKTELNYKNTEPVLDSDGSYFMYSKLRVEKKNWVERNSYSCSVVHEGLHNHHTTKSFSRTPGGGGGSGGGGSGGGGSGGGGSQQQHLEQLLMDLQELLSRMENYRNLKLPGMLTAKFYLPKQATELKDLQCLEDALGPLRHVLDLTQSKSFQLEDAENFISNIRVTVVKLKGSDNTFECQFDDESATVVDFLRRWIAFAQSIISTSPQ

SEQ ID NO: 172 - protein, 230 aa, Artificial Sequence
  source: /note="Description of Artificial Sequence: Synthetic polypeptide"
GPTIKPCPPCKCPAPNAAGGPSVFIFPPKIKDVLMISLSPIVTCVVVDVSEDDPDVQISWFVNNVEVHTAQTQTHREDYNSTLRVVSALPIQHQDWMSGKEFKCKVNNKDLGAPIERTISKPKGSVRAPQVYVLPPPEEEMTKKQVTLWCMVTDFMPEDIYVEWTNNGKTELNYKNTEPVLDSDGSYFMYSKLRVEKKNWVERNSYSCSVVHEGLHNHHTTKSFSRTPGK

SEQ ID NO: 173 - protein, 230 aa, Artificial Sequence
  source: /note="Description of Artificial Sequence: Synthetic polypeptide"
GPTIKPCPPCKCPAPNAAGGPSVFIFPPKIKDVLMISLSPIVTCVVVDVSEDDPDVQISWFVNNVEVHTAQTQTHREDYNSTLRVVSALPIQHQDWMSGKEFKCKVNNKDLGAPIERTISKPKGSVRAPQVYVLPPPEEEMTKKQVTLSCAVTDFMPEDIYVEWTNNGKTELNYKNTEPVLDSDGSYFMVSKLRVEKKNWVERNSYSCSVVHEGLHNHHTTKSFSRTPGK

SEQ ID NO: 174 - protein, 4 aa, Artificial Sequence
  source: /note="Description of Artificial Sequence: Synthetic peptide"
KLIC

SEQ ID NO: 175 - DNA, 1128 bp, Artificial Sequence
  source: /note="Description of Artificial Sequence: Synthetic polynucleotide"
gagtctaagtacggccctccttgtcctccatgtcctgctccagaagctgctggcggcccttccgtgtttctgttccctccaaagcctaaggacaccctgatgatctctcggacccctgaagtgacctgcgtggtggtggatgtgtcccaagaggatcccgaggtgcagttcaattggtacgtggacggcgtggaagtgcacaacgccaagaccaagcctagagaggaacagttcaactccacctacagagtggtgtccgtgctgaccgtgctgcaccaggattggctgaacggcaaagagtacaagtgcaaggtgtccaacaagggcctgccttccagcatcgaaaagaccatctccaaggccaagggccagcctagggaaccccaggtttacaccctgcctccaagccaagaggaaatgaccaagaaccaggtgtccctgtggtgcctggtcaagggcttctacccttccgatatcgccgtggaatgggagagcaatggccagcctgagaacaactacaagaccacacctcctgtgctggactccgacggctccttctttctgtactcccgcctgaccgtggacaagtccagatggcaagagggcaacgtgttctcctgctccgtgatgcacgaggccctgcacaatcactacacccagaagtccctgtctctgtctcttggcggaggcggaggaagtggtggcggaggttctggtggcggtggatcaggcggtggcggaagctctacaaagaaaacccagctgcaactggaacatctgctgctggacctgcagatgatcctgaacggcatcaacaactacaagaaccccaagctgaccggcatgctgaccttcaagttctacatgcccaagaaggccaccgagctgaagcacctccagtgcctggaagaggaactgaagcccctggaagaagtgctgaatctggcccagagcaagaacttccacctgaggcctagggacctgatcagcaacatcaacgtgatcgtgctggaactgaaaggcagcgagacaaccttcatgtgcgagtacgccgacgagacagccaccatcgtggaatttctgaacagatggatcaccttcagccagagcatcatcagcaccctgacc

SEQ ID NO: 176 - DNA, 1128 bp, Artificial Sequence
  source: /note="Description of Artificial Sequence: Synthetic polynucleotide"
gagtctaagtacggccctccttgtcctccatgtcctgctccagaagctgctggcggcccttccgtgtttctgttccctccaaagcctaaggacaccctgatgatctctcggacccctgaagtgacctgcgtggtggtggatgtgtcccaagaggatcccgaggtgcagttcaattggtacgtggacggcgtggaagtgcacaacgccaagaccaagcctagagaggaacagttcaactccacctacagagtggtgtccgtgctgaccgtgctgcaccaggattggctgaacggcaaagagtacaagtgcaaggtgtccaacaagggcctgccttccagcatcgaaaagaccatctccaaggccaagggccagcctagggaaccccaggtttacaccctgcctccaagccaagaggaaatgaccaagaaccaggtgtccctgtggtgcctggtcaagggcttctacccttccgatatcgccgtggaatgggagagcaatggccagcctgagaacaactacaagaccacacctcctgtgctggactccgacggctccttctttctgtactcccgcctgaccgtggacaagtccagatggcaagagggcaacgtgttctcctgctccgtgatgcacgaggccctgcacaatcactacacccagaagtccctgtctctgtctcttggcggaggcggaggaagtggtggcggaggttctggtggcggtggatcaggcggtggcggaagctctacaaagaaaacccagctgcaactggaacatctgctgctggacctgcagatgatcctgaacggcatcaacaactacaagaaccccaagctgaccgccatgctgaccttcaagttctacatgcccaagaaggccaccgagctgaagcacctccagtgcctggaagaggaactgaagcccctggaagaagtgctgaatctggcccagagcaagaacttccacctgaggcctagggacctgatcagcaacatcaacgtgatcgtgctggaactgaaaggcagcgagacaaccttcatgtgcgagtacgccgacgagacagccaccatcgtggaatttctgaacagatggatcaccttcagccagagcatcatcagcaccctgacc

SEQ ID NO: 177 - DNA, 1128 bp, Artificial Sequence
  source: /note="Description of Artificial Sequence: Synthetic polynucleotide"
gagtctaagtacggccctccttgtcctccatgtcctgctccagaagctgctggcggcccttccgtgtttctgttccctccaaagcctaaggacaccctgatgatctctcggacccctgaagtgacctgcgtggtggtggatgtgtcccaagaggatcccgaggtgcagttcaattggtacgtggacggcgtggaagtgcacaacgccaagaccaagcctagagaggaacagttcaactccacctacagagtggtgtccgtgctgaccgtgctgcaccaggattggctgaacggcaaagagtacaagtgcaaggtgtccaacaagggcctgccttccagcatcgaaaagaccatctccaaggccaagggccagcctagggaaccccaggtttacaccctgcctccaagccaagaggaaatgaccaagaaccaggtgtccctgtggtgcctggtcaagggcttctacccttccgatatcgccgtggaatgggagagcaatggccagcctgagaacaactacaagaccacacctcctgtgctggactccgacggctccttctttctgtactcccgcctgaccgtggacaagtccagatggcaagagggcaacgtgttctcctgctccgtgatgcacgaggccctgcacaatcactacacccagaagtccctgtctctgtctcttggcggaggcggaggaagtggtggcggaggttctggtggcggtggatcaggcggtggcggaagctctacaaagaaaacccagctgcaactggaacatctgctgctggacctgcagatgatcctgaacggcatcaacaactacaagaaccccaagctgacccggatgctgggcttcaagttctacatgcccaagaaggccaccgagctgaagcacctccagtgcctggaagaggaactgaagcccctggaagaagtgctgaatctggcccagagcaagaacttccacctgaggcctagggacctgatcagcaacatcaacgtgatcgtgctggaactgaaaggcagcgagacaaccttcatgtgcgagtacgccgacgagacagccaccatcgtggaatttctgaacagatggatcaccttcagccagagcatcatcagcaccctgacc

SEQ ID NO: 178 - DNA, 1128 bp, Artificial Sequence
  source: /note="Description of Artificial Sequence: Synthetic polynucleotide"
gagtctaagtacggccctccttgtcctccatgtcctgctccagaagctgctggcggcccttccgtgtttctgttccctccaaagcctaaggacaccctgatgatctctcggacccctgaagtgacctgcgtggtggtggatgtgtcccaagaggatcccgaggtgcagttcaattggtacgtggacggcgtggaagtgcacaacgccaagaccaagcctagagaggaacagttcaactccacctacagagtggtgtccgtgctgaccgtgctgcaccaggattggctgaacggcaaagagtacaagtgcaaggtgtccaacaagggcctgccttccagcatcgaaaagaccatctccaaggccaagggccagcctagggaaccccaggtttacaccctgcctccaagccaagaggaaatgaccaagaaccaggtgtccctgtggtgcctggtcaagggcttctacccttccgatatcgccgtggaatgggagagcaatggccagcctgagaacaactacaagaccacacctcctgtgctggactccgacggctccttctttctgtactcccgcctgaccgtggacaagtccagatggcaagagggcaacgtgttctcctgctccgtgatgcacgaggccctgcacaatcactacacccagaagtccctgtctctgtctcttggcggaggcggaggaagtggtggcggaggttctggtggcggtggatcaggcggtggcggaagctctacaaagaaaacccagctgcaactggaacatctgctgctggacctgcagatgatcctgaacggcatcaacaactacaagaaccccaagctgacccggatgctggccttcaagttctacatgcccaagaaggccaccgagctgaagcacctccagtgcctggaagaggaactgaagcccctggaagaagtgctgaatctggcccagagcaagaacttccacctgaggcctagggacctgatcagcaacatcaacgtgatcgtgctggaactgaaaggcagcgagacaaccttcatgtgcgagtacgccgacgagacagccaccatcgtggaatttctgaacagatggatcaccttcagccagagcatcatcagcaccctgacc

SEQ ID NO: 179 - DNA, 1128 bp, Artificial Sequence
  source: /note="Description of Artificial Sequence: Synthetic polynucleotide"
gagtctaagtacggccctccttgtcctccatgtcctgctccagaagctgctggcggcccttccgtgtttctgttccctccaaagcctaaggacaccctgatgatctctcggacccctgaagtgacctgcgtggtggtggatgtgtcccaagaggatcccgaggtgcagttcaattggtacgtggacggcgtggaagtgcacaacgccaagaccaagcctagagaggaacagttcaactccacctacagagtggtgtccgtgctgaccgtgctgcaccaggattggctgaacggcaaagagtacaagtgcaaggtgtccaacaagggcctgccttccagcatcgaaaagaccatctccaaggccaagggccagcctagggaaccccaggtttacaccctgcctccaagccaagaggaaatgaccaagaaccaggtgtccctgtggtgcctggtcaagggcttctacccttccgatatcgccgtggaatgggagagcaatggccagcctgagaacaactacaagaccacacctcctgtgctggactccgacggctccttctttctgtactcccgcctgaccgtggacaagtccagatggcaagagggcaacgtgttctcctgctccgtgatgcacgaggccctgcacaatcactacacccagaagtccctgtctctgtctcttggcggaggcggaggaagtggtggcggaggttctggtggcggtggatcaggcggtggcggaagctctacaaagaaaacccagctgcaactggaacatctgctgctggacctgcagatgatcctgaacggcatcaacaactacaagaaccccaagctgacccggatgctgaccggcaagttctacatgcctaagaaggccaccgagctgaagcacctccagtgcctggaagaggaactgaagcccctggaagaagtgctgaatctggcccagagcaagaacttccacctgaggcctagggacctgatcagcaacatcaacgtgatcgtgctggaactgaaaggcagcgagacaaccttcatgtgcgagtacgccgacgagacagccaccatcgtggaatttctgaacagatggatcaccttcagccagagcatcatcagcaccctgacc

SEQ ID NO: 180 - DNA, 1128 bp, Artificial Sequence
  source: /note="Description of Artificial Sequence: Synthetic polynucleotide"
gagtctaagtacggccctccttgtcctccatgtcctgctccagaagctgctggcggcccttccgtgtttctgttccctccaaagcctaaggacaccctgatgatctctcggacccctgaagtgacctgcgtggtggtggatgtgtcccaagaggatcccgaggtgcagttcaattggtacgtggacggcgtggaagtgcacaacgccaagaccaagcctagagaggaacagttcaactccacctacagagtggtgtccgtgctgaccgtgctgcaccaggattggctgaacggcaaagagtacaagtgcaaggtgtccaacaagggcctgccttccagcatcgaaaagaccatctccaaggccaagggccagcctagggaaccccaggtttacaccctgcctccaagccaagaggaaatgaccaagaaccaggtgtccctgtggtgcctggtcaagggcttctacccttccgatatcgccgtggaatgggagagcaatggccagcctgagaacaactacaagaccacacctcctgtgctggactccgacggctccttctttctgtactcccgcctgaccgtggacaagtccagatggcaagagggcaacgtgttctcctgctccgtgatgcacgaggccctgcacaatcactacacccagaagtccctgtctctgtctcttggcggaggcggaggaagtggtggcggaggttctggtggcggtggatcaggcggtggcggaagctctacaaagaaaacccagctgcaactggaacatctgctgctggacctgcagatgatcctgaacggcatcaacaactacaagaaccccaagctgacccggatgctgaccgccaagttctacatgcctaagaaggccaccgagctgaagcacctccagtgcctggaagaggaactgaagcccctggaagaagtgctgaatctggcccagagcaagaacttccacctgaggcctagggacctgatcagcaacatcaacgtgatcgtgctggaactgaaaggcagcgagacaaccttcatgtgcgagtacgccgacgagacagccaccatcgtggaatttctgaacagatggatcaccttcagccagagcatcatcagcaccctgacc

SEQ ID NO: 181 - DNA, 1128 bp, Artificial Sequence
  source: /note="Description of Artificial Sequence: Synthetic polynucleotide"
gagtctaagtacggccctccttgtcctccatgtcctgctccagaagctgctggcggcccttccgtgtttctgttccctccaaagcctaaggacaccctgatgatctctcggacccctgaagtgacctgcgtggtggtggatgtgtcccaagaggatcccgaggtgcagttcaattggtacgtggacggcgtggaagtgcacaacgccaagaccaagcctagagaggaacagttcaactccacctacagagtggtgtccgtgctgaccgtgctgcaccaggattggctgaacggcaaagagtacaagtgcaaggtgtccaacaagggcctgccttccagcatcgaaaagaccatctccaaggccaagggccagcctagggaaccccaggtttacaccctgcctccaagccaagaggaaatgaccaagaaccaggtgtccctgtggtgcctggtcaagggcttctacccttccgatatcgccgtggaatgggagagcaatggccagcctgagaacaactacaagaccacacctcctgtgctggactccgacggctccttctttctgtactcccgcctgaccgtggacaagtccagatggcaagagggcaacgtgttctcctgctccgtgatgcacgaggccctgcacaatcactacacccagaagtccctgtctctgtctcttggcggaggcggaggaagtggtggcggaggttctggtggcggtggatcaggcggtggcggaagctctacaaagaaaacccagctgcaactggaacatctgctgctggacctgcagatgatcctgaacggcatcaacaactacaagaaccccaagctgacccggatgctgaccttcaagttcggcatgcctaagaaggccaccgagctgaaacatctgcagtgcctggaagaggaactgaagcccctggaagaagtgctgaatctggcccagagcaagaacttccacctgaggcctagggacctgatcagcaacatcaacgtgatcgtgctggaactgaaaggcagcgagacaaccttcatgtgcgagtacgccgacgagacagccaccatcgtggaatttctgaacagatggatcaccttcagccagagcatcatcagcaccctgacc

SEQ ID NO: 182 - DNA, 1128 bp, Artificial Sequence
  source: /note="Description of Artificial Sequence: Synthetic polynucleotide"
gagtctaagtacggccctccttgtcctccatgtcctgctccagaagctgctggcggcccttccgtgtttctgttccctccaaagcctaaggacaccctgatgatctctcggacccctgaagtgacctgcgtggtggtggatgtgtcccaagaggatcccgaggtgcagttcaattggtacgtggacggcgtggaagtgcacaacgccaagaccaagcctagagaggaacagttcaactccacctacagagtggtgtccgtgctgaccgtgctgcaccaggattggctgaacggcaaagagtacaagtgcaaggtgtccaacaagggcctgccttccagcatcgaaaagaccatctccaaggccaagggccagcctagggaaccccaggtttacaccctgcctccaagccaagaggaaatgaccaagaaccaggtgtccctgtggtgcctggtcaagggcttctacccttccgatatcgccgtggaatgggagagcaatggccagcctgagaacaactacaagaccacacctcctgtgctggactccgacggctccttctttctgtactcccgcctgaccgtggacaagtccagatggcaagagggcaacgtgttctcctgctccgtgatgcacgaggccctgcacaatcactacacccagaagtccctgtctctgtctcttggcggaggcggaggaagtggtggcggaggttctggtggcggtggatcaggcggtggcggaagctctacaaagaaaacccagctgcaactggaacatctgctgctggacctgcagatgatcctgaacggcatcaacaactacaagaaccccaagctgacccggatgctgaccttcaagttcgccatgcctaagaaggccaccgagctgaaacatctgcagtgcctggaagaggaactgaagcccctggaagaagtgctgaatctggcccagagcaagaacttccacctgaggcctagggacctgatcagcaacatcaacgtgatcgtgctggaactgaaaggcagcgagacaaccttcatgtgcgagtacgccgacgagacagccaccatcgtggaatttctgaacagatggatcaccttcagccagagcatcatcagcaccctgacc

SEQ ID NO: 183 - DNA, 1128 bp, Artificial Sequence
  source: /note="Description of Artificial Sequence: Synthetic polynucleotide"
gagtctaagtacggccctccttgtcctccatgtcctgctccagaagctgctggcggcccttccgtgtttctgttccctccaaagcctaaggacaccctgatgatctctcggacccctgaagtgacctgcgtggtggtggatgtgtcccaagaggatcccgaggtgcagttcaattggtacgtggacggcgtggaagtgcacaacgccaagaccaagcctagagaggaacagttcaactccacctacagagtggtgtccgtgctgaccgtgctgcaccaggattggctgaacggcaaagagtacaagtgcaaggtgtccaacaagggcctgccttccagcatcgaaaagaccatctccaaggccaagggccagcctagggaaccccaggtttacaccctgcctccaagccaagaggaaatgaccaagaaccaggtgtccctgtggtgcctggtcaagggcttctacccttccgatatcgccgtggaatgggagagcaatggccagcctgagaacaactacaagaccacacctcctgtgctggactccgacggctccttctttctgtactcccgcctgaccgtggacaagtccagatggcaagagggcaacgtgttctcctgctccgtgatgcacgaggccctgcacaatcactacacccagaagtccctgtctctgtctcttggcggaggcggaggaagtggtggcggaggttctggtggcggtggatcaggcggtggcggaagctctacaaagaaaacccagctgcaactggaacatctgctgctggacctgcagatgatcctgaacggcatcaacaactacaagaaccccaagctgacccggatgctgaccttcaagttctacatgcccaagaaggccaccgagctgaagcaccttcagtgtctggaagccgaactgaagcccctggaagaggtgctgaatctggcccagagcaagaacttccacctgaggcctagggacctgatcagcaacatcaacgtgatcgtgctggaactgaagggcagcgagacaaccttcatgtgcgagtacgccgacgagacagccaccatcgtggaatttctgaacagatggatcaccttcagccagagcatcatcagcaccctgacc

SEQ ID NO: 184 - DNA, 1128 bp, Artificial Sequence
  source: /note="Description of Artificial Sequence: Synthetic polynucleotide"
gagtctaagtacggccctccttgtcctccatgtcctgctccagaagctgctggcggcccttccgtgtttctgttccctccaaagcctaaggacaccctgatgatctctcggacccctgaagtgacctgcgtggtggtggatgtgtcccaagaggatcccgaggtgcagttcaattggtacgtggacggcgtggaagtgcacaacgccaagaccaagcctagagaggaacagttcaactccacctacagagtggtgtccgtgctgaccgtgctgcaccaggattggctgaacggcaaagagtacaagtgcaaggtgtccaacaagggcctgccttccagcatcgaaaagaccatctccaaggccaagggccagcctagggaaccccaggtttacaccctgcctccaagccaagaggaaatgaccaagaaccaggtgtccctgtggtgcctggtcaagggcttctacccttccgatatcgccgtggaatgggagagcaatggccagcctgagaacaactacaagaccacacctcctgtgctggactccgacggctccttctttctgtactcccgcctgaccgtggacaagtccagatggcaagagggcaacgtgttctcctgctccgtgatgcacgaggccctgcacaatcactacacccagaagtccctgtctctgtctcttggcggaggcggaggaagtggtggcggaggttctggtggcggtggatcaggcggtggcggaagctctacaaagaaaacccagctgcaactggaacatctgctgctggacctgcagatgatcctgaacggcatcaacaactacaagaaccccaagctgacccggatgctgaccttcaagttctacatgcccaagaaggccaccgagctgaagcacctccagtgtctggaagaggccctgaagcctctggaagaagtgctgaatctggcccagagcaagaacttccacctgaggcctagggacctgatcagcaacatcaacgtgatcgtgctggaactgaagggcagcgagacaaccttcatgtgcgagtacgccgacgagacagccaccatcgtggaatttctgaacagatggatcaccttcagccagagcatcatcagcaccctgacc

SEQ ID NO: 185 - DNA, 1128 bp, Artificial Sequence
  source: /note="Description of Artificial Sequence: Synthetic polynucleotide"
gagtctaagtacggccctccttgtcctccatgtcctgctccagaagctgctggcggcccttccgtgtttctgttccctccaaagcctaaggacaccctgatgatctctcggacccctgaagtgacctgcgtggtggtggatgtgtcccaagaggatcccgaggtgcagttcaattggtacgtggacggcgtggaagtgcacaacgccaagaccaagcctagagaggaacagttcaactccacctacagagtggtgtccgtgctgaccgtgctgcaccaggattggctgaacggcaaagagtacaagtgcaaggtgtccaacaagggcctgccttccagcatcgaaaagaccatctccaaggccaagggccagcctagggaaccccaggtttacaccctgcctccaagccaagaggaaatgaccaagaaccaggtgtccctgtggtgcctggtcaagggcttctacccttccgatatcgccgtggaatgggagagcaatggccagcctgagaacaactacaagaccacacctcctgtgctggactccgacggctccttctttctgtactcccgcctgaccgtggacaagtccagatggcaagagggcaacgtgttctcctgctccgtgatgcacgaggccctgcacaatcactacacccagaagtccctgtctctgtctcttggcggaggcggaggaagtggtggcggaggttctggtggcggtggatcaggcggtggcggaagctctacaaagaaaacccagctgcaactggaacatctgctgctggacctgcagatgatcctgaacggcatcaacaactacaagaaccccaagctgacccggatgctgaccttcaagttctacatgcccaagaaggccaccgagctgaagcacctccagtgcctggaagaggaactgaagcctctggaagccgtgctgaatctggcccagagcaagaactttcacctgaggcctcgggacctgatcagcaacatcaacgtgatcgtgctggaactgaaaggcagcgagacaaccttcatgtgcgagtacgccgacgagacagccaccatcgtggaatttctgaacagatggatcaccttcagccagagcatcatcagcaccctgacc

SEQ ID NO: 186 - DNA, 1128 bp, Artificial Sequence
  source: /note="Description of Artificial Sequence: Synthetic polynucleotide"
gagtctaagtacggccctccttgtcctccatgtcctgctccagaagctgctggcggcccttccgtgtttctgttccctccaaagcctaaggacaccctgatgatctctcggacccctgaagtgacctgcgtggtggtggatgtgtcccaagaggatcccgaggtgcagttcaattggtacgtggacggcgtggaagtgcacaacgccaagaccaagcctagagaggaacagttcaactccacctacagagtggtgtccgtgctgaccgtgctgcaccaggattggctgaacggcaaagagtacaagtgcaaggtgtccaacaagggcctgccttccagcatcgaaaagaccatctccaaggccaagggccagcctagggaaccccaggtttacaccctgcctccaagccaagaggaaatgaccaagaaccaggtgtccctgtggtgcctggtcaagggcttctacccttccgatatcgccgtggaatgggagagcaatggccagcctgagaacaactacaagaccacacctcctgtgctggactccgacggctccttctttctgtactcccgcctgaccgtggacaagtccagatggcaagagggcaacgtgttctcctgctccgtgatgcacgaggccctgcacaatcactacacccagaagtccctgtctctgtctcttggcggaggcggaggaagtggtggcggaggttctggtggcggtggatcaggcggtggcggaagctctacaaagaaaacccagctgcaactggaacatctgctgctggacctgcagatgatcctgaacggcatcaacaactacaagaaccccaagctgacccggatgctgaccttcaagttctacatgcccaagaaggccaccgagctgaagcacctccagtgcctggaagaggaactgaagcccctggaagaagtgctgaacggcgcccagagcaagaactttcacctgaggcctcgggacctgatcagcaacatcaacgtgatcgtgctggaactgaaaggcagcgagacaaccttcatgtgcgagtacgccgacgagacagccaccatcgtggaatttctgaacagatggatcaccttcagccagagcatcatcagcaccctgacc

SEQ ID NO: 187 - DNA, 1128 bp, Artificial Sequence
  source: /note="Description of Artificial Sequence: Synthetic polynucleotide"
gagtctaagtacggccctccttgtcctccatgtcctgctccagaagctgctggcggcccttccgtgtttctgttccctccaaagcctaaggacaccctgatgatctctcggacccctgaagtgacctgcgtggtggtggatgtgtcccaagaggatcccgaggtgcagttcaattggtacgtggacggcgtggaagtgcacaacgccaagaccaagcctagagaggaacagttcaactccacctacagagtggtgtccgtgctgaccgtgctgcaccaggattggctgaacggcaaagagtacaagtgcaaggtgtccaacaagggcctgccttccagcatcgaaaagaccatctccaaggccaagggccagcctagggaaccccaggtttacaccctgcctccaagccaagaggaaatgaccaagaaccaggtgtccctgtggtgcctggtcaagggcttctacccttccgatatcgccgtggaatgggagagcaatggccagcctgagaacaactacaagaccacacctcctgtgctggactccgacggctccttctttctgtactcccgcctgaccgtggacaagtccagatggcaagagggcaacgtgttctcctgctccgtgatgcacgaggccctgcacaatcactacacccagaagtccctgtctctgtctcttggcggaggcggaggaagtggtggcggaggttctggtggcggtggatcaggcggtggcggaagctctacaaagaaaacccagctgcaactggaacatctgctgctggacctgcagatgatcctgaacggcatcaacaactacaagaaccccaagctgacccggatgctgaccttcaagttctacatgcccaagaaggccaccgagctgaagcacctccagtgcctggaagaggaactgaagcccctggaagaagtgctgaatctggccggcagcaagaacttccacctgaggcctagagatctgatcagcaacatcaacgtgatcgtgctggaactgaaaggcagcgagacaaccttcatgtgcgagtacgccgacgagacagccaccatcgtggaatttctgaacagatggatcaccttcagccagagcatcatcagcaccctgacc

SEQ ID NO: 188 - DNA, 1128 bp, Artificial Sequence
  source: /note="Description of Artificial Sequence: Synthetic polynucleotide"
gagtctaagtacggccctccttgtcctccatgtcctgctccagaagctgctggcggcccttccgtgtttctgttccctccaaagcctaaggacaccctgatgatctctcggacccctgaagtgacctgcgtggtggtggatgtgtcccaagaggatcccgaggtgcagttcaattggtacgtggacggcgtggaagtgcacaacgccaagaccaagcctagagaggaacagttcaactccacctacagagtggtgtccgtgctgaccgtgctgcaccaggattggctgaacggcaaagagtacaagtgcaaggtgtccaacaagggcctgccttccagcatcgaaaagaccatctccaaggccaagggccagcctagggaaccccaggtttacaccctgcctccaagccaagaggaaatgaccaagaaccaggtgtccctgtggtgcctggtcaagggcttctacccttccgatatcgccgtggaatgggagagcaatggccagcctgagaacaactacaagaccacacctcctgtgctggactccgacggctccttctttctgtactcccgcctgaccgtggacaagtccagatggcaagagggcaacgtgttctcctgctccgtgatgcacgaggccctgcacaatcactacacccagaagtccctgtctctgtctcttggcggaggcggaggaagtggtggcggaggttctggtggcggtggatcaggcggtggcggaagctctacaaagaaaacccagctgcaactggaacatctgctgctggacctgcagatgatcctgaacggcatcaacaactacaagaaccccaagctgacccggatgctgaccttcaagttctacatgcccaagaaggccaccgagctgaagcacctccagtgcctggaagaggaactgaagcccctggaagaagtgctgaatctggcccagagcaagaacttccacctgaggcctagggacctgatcagcaacatcaacgtgatcgtgctggaactgaaaggcagcgagacaacctttatgtgcgagggcgccgacgagacagccaccatcgtggaatttctgaacagatggatcaccttcagccagagcatcatcagcaccctgacc

SEQ ID NO: 189 - DNA, 1128 bp, Artificial Sequence
  source: /note="Description of Artificial Sequence: Synthetic polynucleotide"
gagtctaagtacggccctccttgtcctccatgtcctgctccagaagctgctggcggcccttccgtgtttctgttccctccaaagcctaaggacaccctgatgatctctcggacccctgaagtgacctgcgtggtggtggatgtgtcccaagaggatcccgaggtgcagttcaattggtacgtggacggcgtggaagtgcacaacgccaagaccaagcctagagaggaacagttcaactccacctacagagtggtgtccgtgctgaccgtgctgcaccaggattggctgaacggcaaagagtacaagtgcaaggtgtccaacaagggcctgccttccagcatcgaaaagaccatctccaaggccaagggccagcctagggaaccccaggtttacaccctgcctccaagccaagaggaaatgaccaagaaccaggtgtccctgtggtgcctggtcaagggcttctacccttccgatatcgccgtggaatgggagagcaatggccagcctgagaacaactacaagaccacacctcctgtgctggactccgacggctccttctttctgtactcccgcctgaccgtggacaagtccagatggcaagagggcaacgtgttctcctgctccgtgatgcacgaggccctgcacaatcactacacccagaagtccctgtctctgtctcttggcggaggcggaggaagtggtggcggaggttctggtggcggtggatcaggcggtggcggaagctctacaaagaaaacccagctgcaactggaacatctgctgctggacctgcagatgatcctgaacggcatcaacaactacaagaaccccaagctgacccggatgctgaccttcaagttctacatgcccaagaaggccaccgagctgaagcacctccagtgcctggaagaggaactgaagcccctggaagaagtgctgaatctggcccagagcaagaacttccacctgaggcctagggacctgatcagcaacatcaacgtgatcgtgctggaactgaaaggcagcgagacaacctttatgtgcgaggccgccgacgagacagccaccatcgtggaatttctgaacagatggatcaccttcagccagagcatcatcagcaccctgacc

SEQ ID NO: 190 - DNA, 1128 bp, Artificial Sequence
  source: /note="Description of Artificial Sequence: Synthetic polynucleotide"
gagtctaagtacggccctccttgtcctccatgtcctgctccagaagctgctggcggcccttccgtgtttctgttccctccaaagcctaaggacaccctgatgatctctcggacccctgaagtgacctgcgtggtggtggatgtgtcccaagaggatcccgaggtgcagttcaattggtacgtggacggcgtggaagtgcacaacgccaagaccaagcctagagaggaacagttcaactccacctacagagtggtgtccgtgctgaccgtgctgcaccaggattggctgaacggcaaagagtacaagtgcaaggtgtccaacaagggcctgccttccagcatcgaaaagaccatctccaaggccaagggccagcctagggaaccccaggtttacaccctgcctccaagccaagaggaaatgaccaagaaccaggtgtccctgtggtgcctggtcaagggcttctacccttccgatatcgccgtggaatgggagagcaatggccagcctgagaacaactacaagaccacacctcctgtgctggactccgacggctccttctttctgtactcccgcctgaccgtggacaagtccagatggcaagagggcaacgtgttctcctgctccgtgatgcacgaggccctgcacaatcactacacccagaagtccctgtctctgtctcttggcggaggcggaggaagtggtggcggaggttctggtggcggtggatcaggcggtggcggaagctctacaaagaaaacccagctgcaactggaacatctgctgctggacctgcagatgatcctgaacggcatcaacaactacaagaaccccaagctgacccggatgctgaccttcaagttcggcatgcccaagaaggccaccgagctgaaacatctgcagtgcctggaagctgagctgaagcccctggaagaggtgctgaatctggcccagtccaagaacttccacctgaggcctcgggacctgatctccaacatcaacgtgatcgtgctggaactgaagggctccgagacaaccttcatgtgcgagtacgccgacgagacagctaccatcgtggaatttctgaaccggtggatcaccttcagccagtccatcatcagcaccctgacc

SEQ ID NO: 191 - DNA, 1128 bp, Artificial Sequence
  source: /note="Description of Artificial Sequence: Synthetic polynucleotide"
gagtctaagtacggccctccttgtcctccatgtcctgctccagaagctgctggcggcccttccgtgtttctgttccctccaaagcctaaggacaccctgatgatctctcggacccctgaagtgacctgcgtggtggtggatgtgtcccaagaggatcccgaggtgcagttcaattggtacgtggacggcgtggaagtgcacaacgccaagaccaagcctagagaggaacagttcaactccacctacagagtggtgtccgtgctgaccgtgctgcaccaggattggctgaacggcaaagagtacaagtgcaaggtgtccaacaagggcctgccttccagcatcgaaaagaccatctccaaggccaagggccagcctagggaaccccaggtttacaccctgcctccaagccaagaggaaatgaccaagaaccaggtgtccctgtggtgcctggtcaagggcttctacccttccgatatcgccgtggaatgggagagcaatggccagcctgagaacaactacaagaccacacctcctgtgctggactccgacggctccttctttctgtactcccgcctgaccgtggacaagtccagatggcaagagggcaacgtgttctcctgctccgtgatgcacgaggccctgcacaatcactacacccagaagtccctgtctctgtctcttggcggaggcggaggaagtggtggcggaggttctggtggcggtggatcaggcggtggcggaagctctacaaagaaaacccagctgcaactggaacatctgctgctggacctgcagatgatcctgaacggcatcaacaactacaagaaccccaagctgacccggatgctgaccttcaagttcggcatgcccaagaaggccaccgagctgaaacatctgcagtgcctggaagaggccctgaagcctctggaagaagtgctgaatctggcccagtccaagaacttccacctgaggcctcgggacctgatctccaacatcaacgtgatcgtgctggaactgaagggctccgagacaaccttcatgtgcgagtacgccgacgagacagctaccatcgtggaatttctgaaccggtggatcaccttcagccagtccatcatcagcaccctgacc

SEQ ID NO: 192 - DNA, 1128 bp, Artificial Sequence
  source: /note="Description of Artificial Sequence: Synthetic polynucleotide"
gagtctaagtacggccctccttgtcctccatgtcctgctccagaagctgctggcggcccttccgtgtttctgttccctccaaagcctaaggacaccctgatgatctctcggacccctgaagtgacctgcgtggtggtggatgtgtcccaagaggatcccgaggtgcagttcaattggtacgtggacggcgtggaagtgcacaacgccaagaccaagcctagagaggaacagttcaactccacctacagagtggtgtccgtgctgaccgtgctgcaccaggattggctgaacggcaaagagtacaagtgcaaggtgtccaacaagggcctgccttccagcatcgaaaagaccatctccaaggccaagggccagcctagggaaccccaggtttacaccctgcctccaagccaagaggaaatgaccaagaaccaggtgtccctgtggtgcctggtcaagggcttctacccttccgatatcgccgtggaatgggagagcaatggccagcctgagaacaactacaagaccacacctcctgtgctggactccgacggctccttctttctgtactcccgcctgaccgtggacaagtccagatggcaagagggcaacgtgttctcctgctccgtgatgcacgaggccctgcacaatcactacacccagaagtccctgtctctgtctcttggcggaggcggaggaagtggtggcggaggttctggtggcggtggatcaggcggtggcggaagctctacaaagaaaacccagctgcaactggaacatctgctgctggacctgcagatgatcctgaacggcatcaacaactacaagaaccccaagctgaccggcatgctgaccttcaagttcggcatgcccaagaaggccaccgagctgaaacatctgcagtgcctggaagaggaactgaagcccctggaagaagtgctgaatctggcccagtccaagaacttccacctgaggcctcgggacctgatctccaacatcaacgtgatcgtgctcgagctgaagggctccgagacaaccttcatgtgcgagtacgccgacgagacagctaccatcgtggaatttctgaaccggtggatcaccttcagccagtccatcatcagcaccctgacc

SEQ ID NO: 193 - DNA, 1128 bp, Artificial Sequence
  source: /note="Description of Artificial Sequence: Synthetic polynucleotide"
gagtctaagtacggccctccttgtcctccatgtcctgctccagaagctgctggcggcccttccgtgtttctgttccctccaaagcctaaggacaccctgatgatctctcggacccctgaagtgacctgcgtggtggtggatgtgtcccaagaggatcccgaggtgcagttcaattggtacgtggacggcgtggaagtgcacaacgccaagaccaagcctagagaggaacagttcaactccacctacagagtggtgtccgtgctgaccgtgctgcaccaggattggctgaacggcaaagagtacaagtgcaaggtgtccaacaagggcctgccttccagcatcgaaaagaccatctccaaggccaagggccagcctagggaaccccaggtttacaccctgcctccaagccaagaggaaatgaccaagaaccaggtgtccctgtggtgcctggtcaagggcttctacccttccgatatcgccgtggaatgggagagcaatggccagcctgagaacaactacaagaccacacctcctgtgctggactccgacggctccttctttctgtactcccgcctgaccgtggacaagtccagatggcaagagggcaacgtgttctcctgctccgtgatgcacgaggccctgcacaatcactacacccagaagtccctgtctctgtctcttggcggaggcggaggaagtggtggcggaggttctggtggcggtggatcaggcggtggcggaagctctacaaagaaaacccagctgcaactggaacatctgctgctggacctgcagatgatcctgaacggcatcaacaactacaagaaccccaagctgaccggcatgctgaccttcaagttctacatgcccaagaaggccaccgagctgaaacatctgcagtgcctggaagctgagctgaagcccctggaagaggtgctgaatctggcccagtccaagaacttccacctgaggcctcgggacctgatctccaacatcaacgtgatcgtgctggaactgaagggctccgagacaaccttcatgtgcgagtacgccgacgagacagctaccatcgtggaatttctgaaccggtggatcaccttcagccagtccatcatcagcaccctgacc

SEQ ID NO: 194 - DNA, 1128 bp, Artificial Sequence
  source: /note="Description of Artificial Sequence: Synthetic polynucleotide"
gagtctaagtacggccctccttgtcctccatgtcctgctccagaagctgctggcggcccttccgtgtttctgttccctccaaagcctaaggacaccctgatgatctctcggacccctgaagtgacctgcgtggtggtggatgtgtcccaagaggatcccgaggtgcagttcaattggtacgtggacggcgtggaagtgcacaacgccaagaccaagcctagagaggaacagttcaactccacctacagagtggtgtccgtgctgaccgtgctgcaccaggattggctgaacggcaaagagtacaagtgcaaggtgtccaacaagggcctgccttccagcatcgaaaagaccatctccaaggccaagggccagcctagggaaccccaggtttacaccctgcctccaagccaagaggaaatgaccaagaaccaggtgtccctgtggtgcctggtcaagggcttctacccttccgatatcgccgtggaatgggagagcaatggccagcctgagaacaactacaagaccacacctcctgtgctggactccgacggctccttctttctgtactcccgcctgaccgtggacaagtccagatggcaagagggcaacgtgttctcctgctccgtgatgcacgaggccctgcacaatcactacacccagaagtccctgtctctgtctcttggcggaggcggaggaagtggtggcggaggttctggtggcggtggatcaggcggtggcggaagctctacaaagaaaacccagctgcaactggaacatctgctgctggacctgcagatgatcctgaacggcatcaacaactacaagaaccccaagctgacccggatgctgaccgccaagttctacatgcccaagaaggccaccgagctgaaacatctgcagtgcctggaagctgagctgaagcccctggaagaggtgctgaatctggcccagtccaagaacttccacctgaggcctcgggacctgatctccaacatcaacgtgatcgtgctggaactgaagggctccgagacaaccttcatgtgcgagtacgccgacgagacagctaccatcgtggaatttctgaaccggtggatcaccttcagccagtccatcatcagcaccctgacc

SEQ ID NO: 195 - DNA, 1128 bp, Artificial Sequence
  source: /note="Description of Artificial Sequence: Synthetic polynucleotide"
gagtctaagtacggccctccttgtcctccatgtcctgctccagaagctgctggcggcccttccgtgtttctgttccctccaaagcctaaggacaccctgatgatctctcggacccctgaagtgacctgcgtggtggtggatgtgtcccaagaggatcccgaggtgcagttcaattggtacgtggacggcgtggaagtgcacaacgccaagaccaagcctagagaggaacagttcaactccacctacagagtggtgtccgtgctgaccgtgctgcaccaggattggctgaacggcaaagagtacaagtgcaaggtgtccaacaagggcctgccttccagcatcgaaaagaccatctccaaggccaagggccagcctagggaaccccaggtttacaccctgcctccaagccaagaggaaatgaccaagaaccaggtgtccctgtggtgcctggtcaagggcttctacccttccgatatcgccgtggaatgggagagcaatggccagcctgagaacaactacaagaccacacctcctgtgctggactccgacggctccttctttctgtactcccgcctgaccgtggacaagtccagatggcaagagggcaacgtgttctcctgctccgtgatgcacgaggccctgcacaatcactacacccagaagtccctgtctctgtctcttggcggaggcggaggaagtggtggcggaggttctggtggcggtggatcaggcggtggcggaagctctacaaagaaaacccagctgcaactggaacatctgctgctggacctgcagatgatcctgaacggcatcaacaactacaagaaccccaagctgacccggatgctgaccgccaagtttggcatgcctaagaaggccaccgagctgaaacatctgcagtgcctggaagaggaactgaagcccctggaagaagtgctgaatctggcccagtccaagaacttccacctgaggcctcgggacctgatctccaacatcaacgtgatcgtgctcgagctgaagggctccgagacaaccttcatgtgcgagtacgccgacgagacagctaccatcgtggaatttctgaaccggtggatcaccttcagccagtccatcatcagcaccctgacc

SEQ ID NO: 196 - DNA, 1128 bp, Artificial Sequence
  source: /note="Description of Artificial Sequence: Synthetic polynucleotide"
gagtctaagtacggccctccttgtcctccatgtcctgctccagaagctgctggcggcccttccgtgtttctgttccctccaaagcctaaggacaccctgatgatctctcggacccctgaagtgacctgcgtggtggtggatgtgtcccaagaggatcccgaggtgcagttcaattggtacgtggacggcgtggaagtgcacaacgccaagaccaagcctagagaggaacagttcaactccacctacagagtggtgtccgtgctgaccgtgctgcaccaggattggctgaacggcaaagagtacaagtgcaaggtgtccaacaagggcctgccttccagcatcgaaaagaccatctccaaggccaagggccagcctagggaaccccaggtttacaccctgcctccaagccaagaggaaatgaccaagaaccaggtgtccctgtggtgcctggtcaagggcttctacccttccgatatcgccgtggaatgggagagcaatggccagcctgagaacaactacaagaccacacctcctgtgctggactccgacggctccttctttctgtactcccgcctgaccgtggacaagtccagatggcaagagggcaacgtgttctcctgctccgtgatgcacgaggccctgcacaatcactacacccagaagtccctgtctctgtctcttggcggaggcggaggaagtggtggcggaggttctggtggcggtggatcaggcggtggcggaagctctacaaagaaaacccagctgcaactggaacatctgctgctggacctgcagatgatcctgaacggcatcaacaactacaagaaccccaagctgacccggatgctgaccttcaagttcggcatgcccaagaaggccaccgagctgaagcaccttcagtgtctggaagccgctctgaagcccctggaagaggtgctgaatctggcccagagcaagaacttccacctgaggcctagggacctgatcagcaacatcaacgtgatcgtgctggaactgaagggcagcgagacaaccttcatgtgcgagtacgccgacgagacagccaccatcgtggaatttctgaacagatggatcaccttcagccagagcatcatcagcaccctgacc

SEQ ID NO: 197 - DNA, 1128 bp, Artificial Sequence
  source: /note="Description of Artificial Sequence: Synthetic polynucleotide"
gagtctaagtacggccctccttgtcctccatgtcctgctccagaagctgctggcggcccttccgtgtttctgttccctccaaagcctaaggacaccctgatgatctctcggacccctgaagtgacctgcgtggtggtggatgtgtcccaagaggatcccgaggtgcagttcaattggtacgtggacggcgtggaagtgcacaacgccaagaccaagcctagagaggaacagttcaactccacctacagagtggtgtccgtgctgaccgtgctgcaccaggattggctgaacggcaaagagtacaagtgcaaggtgtccaacaagggcctgccttccagcatcgaaaagaccatctccaaggccaagggccagcctagggaaccccaggtttacaccctgcctccaagccaagaggaaatgaccaagaaccaggtgtccctgtggtgcctggtcaagggcttctacccttccgatatcgccgtggaatgggagagcaatggccagcctgagaacaactacaagaccacacctcctgtgctggactccgacggctccttctttctgtactcccgcctgaccgtggacaagtccagatggcaagagggcaacgtgttctcctgctccgtgatgcacgaggccctgcacaatcactacacccagaagtccctgtctctgtctcttggcggaggcggaggaagtggtggcggaggttctggtggcggtggatcaggcggtggcggaagctctacaaagaaaacccagctgcaactggaacatctgctgctggacctgcagatgatcctgaacggcatcaacaactacaagaaccccaagctgacccggatgctgaccttcaagttctacatgcccaagaaggccaccgagctgaagcaccttcagtgtctggaagccgctctgaagcccctggaagaggtgctgaatctggcccagagcaagaacttccacctgaggcctagggacctgatcagcaacatcaacgtgatcgtgctggaactgaagggcagcgagacaaccttcatgtgcgagtacgccgacgagacagccaccatcgtggaatttctgaacagatggatcaccttcagccagagcatcatcagcaccctgacc

SEQ ID NO: 198 - DNA, 1128 bp, Artificial Sequence
  source: /note="Description of Artificial Sequence: Synthetic polynucleotide"
gagtctaagtacggccctccttgtcctccatgtcctgctccagaagctgctggcggcccttccgtgtttctgttccctccaaagcctaaggacaccctgatgatctctcggacccctgaagtgacctgcgtggtggtggatgtgtcccaagaggatcccgaggtgcagttcaattggtacgtggacggcgtggaagtgcacaacgccaagaccaagcctagagaggaacagttcaactccacctacagagtggtgtccgtgctgaccgtgctgcaccaggattggctgaacggcaaagagtacaagtgcaaggtgtccaacaagggcctgccttccagcatcgaaaagaccatctccaaggccaagggccagcctagggaaccccaggtttacaccctgcctccaagccaagaggaaatgaccaagaaccaggtgtccctgtggtgcctggtcaagggcttctacccttccgatatcgccgtggaatgggagagcaatggccagcctgagaacaactacaagaccacacctcctgtgctggactccgacggctccttctttctgtactcccgcctgaccgtggacaagtccagatggcaagagggcaacgtgttctcctgctccgtgatgcacgaggccctgcacaatcactacacccagaagtccctgtctctgtctcttggcggaggcggaggaagtggtggcggaggttctggtggcggtggatcaggcggtggcggaagctctacaaagaaaacccagctgcaactggaacatctgctgctggacctgcagatgatcctgaacggcatcaacaactacaagaaccccaagctgaccggcatgctgaccgccaagttctacatgcccaagaaggccaccgagctgaaacatctgcagtgcctggaagaggaactgaagcccctggaagaagtgctgaatctggcccagtccaagaacttccacctgaggcctcgggacctgatctccaacatcaacgtgatcgtgctcgagctgaagggctccgagacaaccttcatgtgcgagtacgccgacgagacagctaccatcgtggaatttctgaaccggtggatcaccttcagccagtccatcatcagcaccctgacc

SEQ ID NO: 199 - DNA, 1128 bp, Artificial Sequence
  source: /note="Description of Artificial Sequence: Synthetic polynucleotide"
gagtctaagtacggccctccttgtcctccatgtcctgctccagaagctgctggcggcccttccgtgtttctgttccctccaaagcctaaggacaccctgatgatctctcggacccctgaagtgacctgcgtggtggtggatgtgtcccaagaggatcccgaggtgcagttcaattggtacgtggacggcgtggaagtgcacaacgccaagaccaagcctagagaggaacagttcaactccacctacagagtggtgtccgtgctgaccgtgctgcaccaggattggctgaacggcaaagagtacaagtgcaaggtgtccaacaagggcctgccttccagcatcgaaaagaccatctccaaggccaagggccagcctagggaaccccaggtttacaccctgcctccaagccaagaggaaatgaccaagaaccaggtgtccctgtggtgcctggtcaagggcttctacccttccgatatcgccgtggaatgggagagcaatggccagcctgagaacaactacaagaccacacctcctgtgctggactccgacggctccttctttctgtactcccgcctgaccgtggacaagtccagatggcaagagggcaacgtgttctcctgctccgtgatgcacgaggccctgcacaatcactacacccagaagtccctgtctctgtctcttggcggaggcggaggatctggtggtggtggatctggcggcggaggtagcggtggtggcggttcttctaccaagaaaacccagctgcagttggagcatctgctgctggacctgcagatgatcctgaacggcatcaacaactacaagaaccccaagctgacccggatgctgaccgccaagtttgccatgcctaagaaggccaccgagctgaaacatctgcagtgcctggaagaggaactgaagcccctggaagaagtgctgaacggcgcccagtccaagaacttccatctgaggcctcgggacctgatctccaacatcaacgtgatcgtgctcgagctgaagggctccgagacaaccttcatgtgcgagtacgccgacgagacagctaccatcgtggaatttctgaaccggtggatcaccttcagccagtccatcatcagcaccctgacc

SEQ ID NO: 200 - DNA, 1128 bp, Artificial Sequence
  source: /note="Description of Artificial Sequence: Synthetic polynucleotide"
gagtctaagtacggccctccttgtcctccatgtcctgctccagaagctgctggcggcccttccgtgtttctgttccctccaaagcctaaggacaccctgatgatctctcggacccctgaagtgacctgcgtggtggtggatgtgtcccaagaggatcccgaggtgcagttcaattggtacgtggacggcgtggaagtgcacaacgccaagaccaagcctagagaggaacagttcaactccacctacagagtggtgtccgtgctgaccgtgctgcaccaggattggctgaacggcaaagagtacaagtgcaaggtgtccaacaagggcctgccttccagcatcgaaaagaccatctccaaggccaagggccagcctagggaaccccaggtttacaccctgcctccaagccaagaggaaatgaccaagaaccaggtgtccctgtggtgcctggtcaagggcttctacccttccgatatcgccgtggaatgggagagcaatggccagcctgagaacaactacaagaccacacctcctgtgctggactccgacggctccttctttctgtactcccgcctgaccgtggacaagtccagatggcaagagggcaacgtgttctcctgctccgtgatgcacgaggccctgcacaatcactacacccagaagtccctgtctctgtctcttggcggaggcggaggaagtggtggcggaggttctggtggcggtggatcaggcggtggcggaagctctacaaagaaaacccagctgcaactggaacatctgctgctggacctgcagatgatcctgaacggcatcaacaactacaagaaccccaagctgaccggcatgctgaccgccaagtttggcatgcctaagaaggccaccgagctgaaacatctgcagtgcctggaagaggaactgaagcccctggaagaagtgctgaatctggcccagtccaagaacttccacctgaggcctcgggacctgatctccaacatcaacgtgatcgtgctcgagctgaagggctccgagacaaccttcatgtgcgagtacgccgacgagacagctaccatcgtggaatttctgaaccggtggatcaccttcagccagtccatcatcagcaccctgacc

SEQ ID NO: 201 - DNA, 1128 bp, Artificial Sequence
  source: /note="Description of Artificial Sequence: Synthetic polynucleotide"
gagtctaagtacggccctccttgtcctccatgtcctgctccagaagctgctggcggcccttccgtgtttctgttccctccaaagcctaaggacaccctgatgatctctcggacccctgaagtgacctgcgtggtggtggatgtgtcccaagaggatcccgaggtgcagttcaattggtacgtggacggcgtggaagtgcacaacgccaagaccaagcctagagaggaacagttcaactccacctacagagtggtgtccgtgctgaccgtgctgcaccaggattggctgaacggcaaagagtacaagtgcaaggtgtccaacaagggcctgccttccagcatcgaaaagaccatctccaaggccaagggccagcctagggaaccccaggtttacaccctgcctccaagccaagaggaaatgaccaagaaccaggtgtccctgtggtgcctggtcaagggcttctacccttccgatatcgccgtggaatgggagagcaatggccagcctgagaacaactacaagaccacacctcctgtgctggactccgacggctccttctttctgtactcccgcctgaccgtggacaagtccagatggcaagagggcaacgtgttctcctgctccgtgatgcacgaggccctgcacaatcactacacccagaagtccctgtctctgtctcttggcggaggcggaggaagtggtggcggaggttctggtggcggtggatcaggcggtggcggaagctctacaaagaaaacccagctgcaactggaacatctgctgctggacctgcagatgatcctgaacggcatcaacaactacaagaaccccaagctgacccggatgctgaccgccaagttctacatgcccaagaaggccaccgagctgaaacatctgcagtgcctggaagaggccctgaagcctctggaagaagtgctgaatctggcccagtccaagaacttccacctgaggcctcgggacctgatctccaacatcaacgtgatcgtgctggaactgaagggctccgagacaaccttcatgtgcgagtacgccgacgagacagctaccatcgtggaatttctgaaccggtggatcaccttcagccagtccatcatcagcaccctgacc

SEQ ID NO: 202 - DNA, 1128 bp, Artificial Sequence
  source: /note="Description of Artificial Sequence: Synthetic polynucleotide"
gagtctaagtacggccctccttgtcctccatgtcctgctccagaagctgctggcggcccttccgtgtttctgttccctccaaagcctaaggacaccctgatgatctctcggacccctgaagtgacctgcgtggtggtggatgtgtcccaagaggatcccgaggtgcagttcaattggtacgtggacggcgtggaagtgcacaacgccaagaccaagcctagagaggaacagttcaactccacctacagagtggtgtccgtgctgaccgtgctgcaccaggattggctgaacggcaaagagtacaagtgcaaggtgtccaacaagggcctgccttccagcatcgaaaagaccatctccaaggccaagggccagcctagggaaccccaggtttacaccctgcctccaagccaagaggaaatgaccaagaaccaggtgtccctgtggtgcctggtcaagggcttctacccttccgatatcgccgtggaatgggagagcaatggccagcctgagaacaactacaagaccacacctcctgtgctggactccgacggctccttctttctgtactcccgcctgaccgtggacaagtccagatggcaagagggcaacgtgttctcctgctccgtgatgcacgaggccctgcacaatcactacacccagaagtccctgtctctgtcccttggcggaggcggaggatctggtggtggcggatctggcggcggaggtagcggtggcggtggatcttctaccaagaaaacccagctgcagttggagcatctgctgctggacctgcagatgatcctgaatggcatcaacaattacaagaaccccaagctgacccggatgctgaccgccaagttctacatgcccaagaaggccaccgagctgaaacatctgcagtgcctggaagaggccctgaagcctctggaagaagtgctgaatctggcccagtccaagaacttccacctgaggcctcgggacctgatctccaacatcaacgtgatcgtgctggaactgaagggctccgagacaaccttcatgtgcgagtacgccgacgagacagctaccatcgtggaatttctgaaccggtggatcaccttcagccagtccatcatcagcaccctgacc

SEQ ID NO: 203 - DNA, 1128 bp, Artificial Sequence
  source: /note="Description of Artificial Sequence: Synthetic polynucleotide"
gagtctaagtacggccctccttgtcctccatgtcctgctccagaagctgctggcggcccttccgtgtttctgttccctccaaagcctaaggacaccctgatgatctctcggacccctgaagtgacctgcgtggtggtggatgtgtcccaagaggatcccgaggtgcagttcaattggtacgtggacggcgtggaagtgcacaacgccaagaccaagcctagagaggaacagttcaactccacctacagagtggtgtccgtgctgaccgtgctgcaccaggattggctgaacggcaaagagtacaagtgcaaggtgtccaacaagggcctgccttccagcatcgaaaagaccatctccaaggccaagggccagcctagggaaccccaggtttacaccctgcctccaagccaagaggaaatgaccaagaaccaggtgtccctgtggtgcctggtcaagggcttctacccttccgatatcgccgtggaatgggagagcaatggccagcctgagaacaactacaagaccacacctcctgtgctggactccgacggctccttctttctgtactcccgcctgaccgtggacaagtccagatggcaagagggcaacgtgttctcctgctccgtgatgcacgaggccctgcacaatcactacacccagaagtccctgtctctgtctcttggcggaggcggaggaagtggtggcggaggttctggtggcggtggatcaggcggtggcggaagctctacaaagaaaacccagctgcaactggaacatctgctgctggacctgcagatgatcctgaacggcatcaacaactacaagaaccccaagctgacccggatgctgaccgccaagtttggcatgcctaagaaggccaccgagctgaaacatctgcagtgcctggaagaggccctgaagcctctggaagaagtgctgaatctggcccagtccaagaacttccacctgaggcctcgggacctgatctccaacatcaacgtgatcgtgctggaactgaagggctccgagacaaccttcatgtgcgagtacgccgacgagacagctaccatcgtggaatttctgaaccggtggatcaccttcagccagtccatcatcagcaccctgacc

SEQ ID NO: 204 - DNA, 1128 bp, Artificial Sequence
  source: /note="Description of Artificial Sequence: Synthetic polynucleotide"
gagtctaagtacggccctccttgtcctccatgtcctgctccagaagctgctggcggcccttccgtgtttctgttccctccaaagcctaaggacaccctgatgatctctcggacccctgaagtgacctgcgtggtggtggatgtgtcccaagaggatcccgaggtgcagttcaattggtacgtggacggcgtggaagtgcacaacgccaagaccaagcctagagaggaacagttcaactccacctacagagtggtgtccgtgctgaccgtgctgcaccaggattggctgaacggcaaagagtacaagtgcaaggtgtccaacaagggcctgccttccagcatcgaaaagaccatctccaaggccaagggccagcctagggaaccccaggtttacaccctgcctccaagccaagaggaaatgaccaagaaccaggtgtccctgtggtgcctggtcaagggcttctacccttccgatatcgccgtggaatgggagagcaatggccagcctgagaacaactacaagaccacacctcctgtgctggactccgacggctccttctttctgtactcccgcctgaccgtggacaagtccagatggcaagagggcaacgtgttctcctgctccgtgatgcacgaggccctgcacaatcactacacccagaagtccctgtctctgtctcttggcggaggcggaggaagtggtggcggaggttctggtggcggtggatcaggcggtggcggaagctctacaaagaaaacccagctgcaactggaacatctgctgctggacctgcagatgatcctgaacggcatcaacaactacaagaaccccaagctgacccggatgctgaccgccaagtttggcatgcctaagaaggccaccgagctgaaacatctgcagtgcctggaagctgagctgaagcccctggaagaggtgctgaatctggcccagtccaagaacttccacctgaggcctcgggacctgatctccaacatcaacgtgatcgtgctggaactgaagggctccgagacaaccttcatgtgcgagtacgccgacgagacagctaccatcgtggaatttctgaaccggtggatcaccttcagccagtccatcatcagcaccctgacc

SEQ ID NO: 205 - DNA, 1128 bp, Artificial Sequence
  source: /note="Description of Artificial Sequence: Synthetic polynucleotide"
gagtctaagtacggccctccttgtcctccatgtcctgctccagaagctgctggcggcccttccgtgtttctgttccctccaaagcctaaggacaccctgatgatctctcggacccctgaagtgacctgcgtggtggtggatgtgtcccaagaggatcccgaggtgcagttcaattggtacgtggacggcgtggaagtgcacaacgccaagaccaagcctagagaggaacagttcaactccacctacagagtggtgtccgtgctgaccgtgctgcaccaggattggctgaacggcaaagagtacaagtgcaaggtgtccaacaagggcctgccttccagcatcgaaaagaccatctccaaggccaagggccagcctagggaaccccaggtttacaccctgcctccaagccaagaggaaatgaccaagaaccaggtgtccctgtggtgcctggtcaagggcttctacccttccgatatcgccgtggaatgggagagcaatggccagcctgagaacaactacaagaccacacctcctgtgctggactccgacggctccttctttctgtactcccgcctgaccgtggacaagtccagatggcaagagggcaacgtgttctcctgctccgtgatgcacgaggccctgcacaatcactacacccagaagtccctgtctctgtctcttggcggaggcggaggaagtggtggcggaggttctggtggcggtggatcaggcggtggcggaagctctacaaagaaaacccagctgcaactggaacatctgctgctggacctgcagatgatcctgaacggcatcaacaactacaagaaccccaagctgaccggcatgctgaccttcaagttcggcatgcccaagaaggccaccgagctgaaacatctgcagtgcctggaagctgagctgaagcccctggaagaggtgctgaatctggcccagtccaagaacttccacctgaggcctcgggacctgatctccaacatcaacgtgatcgtgctggaactgaagggctccgagacaaccttcatgtgcgagtacgccgacgagacagctaccatcgtggaatttctgaaccggtggatcaccttcagccagtccatcatcagcaccctgacc

SEQ ID NO: 206 - DNA, 1128 bp, Artificial Sequence
  source: /note="Description of Artificial Sequence: Synthetic polynucleotide"
gagtctaagtacggccctccttgtcctccatgtcctgctccagaagctgctggcggcccttccgtgtttctgttccctccaaagcctaaggacaccctgatgatctctcggacccctgaagtgacctgcgtggtggtggatgtgtcccaagaggatcccgaggtgcagttcaattggtacgtggacggcgtggaagtgcacaacgccaagaccaagcctagagaggaacagttcaactccacctacagagtggtgtccgtgctgaccgtgctgcaccaggattggctgaacggcaaagagtacaagtgcaaggtgtccaacaagggcctgccttccagcatcgaaaagaccatctccaaggccaagggccagcctagggaaccccaggtttacaccctgcctccaagccaagaggaaatgaccaagaaccaggtgtccctgtggtgcctggtcaagggcttctacccttccgatatcgccgtggaatgggagagcaatggccagcctgagaacaactacaagaccacacctcctgtgctggactccgacggctccttctttctgtactcccgcctgaccgtggacaagtccagatggcaagagggcaacgtgttctcctgctccgtgatgcacgaggccctgcacaatcactacacccagaagtccctgtctctgtctcttggcggaggcggaggaagtggtggcggaggttctggtggcggtggatcaggcggtggcggaagctctacaaagaaaacccagctgcaactggaacatctgctgctggacctgcagatgatcctgaacggcatcaacaactacaagaaccccaagctgaccggcatgctgaccgccaagttctacatgcccaagaaggccaccgagctgaaacatctgcagtgcctggaagctgagctgaagcccctggaagaggtgctgaatctggcccagtccaagaacttccacctgaggcctcgggacctgatctccaacatcaacgtgatcgtgctggaactgaagggctccgagacaaccttcatgtgcgagtacgccgacgagacagctaccatcgtggaatttctgaaccggtggatcaccttcagccagtccatcatcagcaccctgacc

SEQ ID NO: 207 - DNA, 1128 bp, Artificial Sequence
  source: /note="Description of Artificial Sequence: Synthetic polynucleotide"
gagtctaagtacggccctccttgtcctccatgtcctgctccagaagctgctggcggcccttccgtgtttctgttccctccaaagcctaaggacaccctgatgatctctcggacccctgaagtgacctgcgtggtggtggatgtgtcccaagaggatcccgaggtgcagttcaattggtacgtggacggcgtggaagtgcacaacgccaagaccaagcctagagaggaacagttcaactccacctacagagtggtgtccgtgctgaccgtgctgcaccaggattggctgaacggcaaagagtacaagtgcaaggtgtccaacaagggcctgccttccagcatcgaaaagaccatctccaaggccaagggccagcctagggaaccccaggtttacaccctgcctccaagccaagaggaaatgaccaagaaccaggtgtccctgtggtgcctggtcaagggcttctacccttccgatatcgccgtggaatgggagagcaatggccagcctgagaacaactacaagaccacacctcctgtgctggactccgacggctccttctttctgtactcccgcctgaccgtggacaagtccagatggcaagagggcaacgtgttctcctgctccgtgatgcacgaggccctgcacaatcactacacccagaagtccctgtctctgtctcttggcggaggcggaggaagtggtggcggaggttctggtggcggtggatcaggcggtggcggaagctctacaaagaaaacccagctgcaactggaacatctgctgctggacctgcagatgatcctgaacggcatcaacaactacaagaaccccaagctgaccggcatgctgaccttcaagttcggcatgcccaagaaggccaccgagctgaaacatctgcagtgcctggaagaggccctgaagcctctggaagaagtgctgaatctggcccagtccaagaacttccacctgaggcctcgggacctgatctccaacatcaacgtgatcgtgctggaactgaagggctccgagacaaccttcatgtgcgagtacgccgacgagacagctaccatcgtggaatttctgaaccggtggatcaccttcagccagtccatcatcagcaccctgacc

SEQ ID NO: 208 - DNA, 1128 bp, Artificial Sequence
  source: /note="Description of Artificial Sequence: Synthetic polynucleotide"
gagtctaagtacggccctccttgtcctccatgtcctgctccagaagctgctggcggcccttccgtgtttctgttccctccaaagcctaaggacaccctgatgatctctcggacccctgaagtgacctgcgtggtggtggatgtgtcccaagaggatcccgaggtgcagttcaattggtacgtggacggcgtggaagtgcacaacgccaagaccaagcctagagaggaacagttcaactccacctacagagtggtgtccgtgctgaccgtgctgcaccaggattggctgaacggcaaagagtacaagtgcaaggtgtccaacaagggcctgccttccagcatcgaaaagaccatctccaaggccaagggccagcctagggaaccccaggtttacaccctgcctccaagccaagaggaaatgaccaagaaccaggtgtccctgtggtgcctggtcaagggcttctacccttccgatatcgccgtggaatgggagagcaatggccagcctgagaacaactacaagaccacacctcctgtgctggactccgacggctccttctttctgtactcccgcctgaccgtggacaagtccagatggcaagagggcaacgtgttctcctgctccgtgatgcacgaggccctgcacaatcactacacccagaagtccctgtctctgtctcttggcggaggcggaggaagtggtggcggaggttctggtggcggtggatcaggcggtggcggaagctctacaaagaaaacccagctgcaactggaacatctgctgctggacctgcagatgatcctgaacggcatcaacaactacaagaaccccaagctgaccggcatgctgaccttcaagttctacatgcccaagaaggccaccgagctgaaacatctgcagtgcctggaagaggccctgaagcctctggaagaagtgctgaatctggcccagtccaagaacttccacctgaggcctcgggacctgatctccaacatcaacgtgatcgtgctggaactgaagggctccgagacaaccttcatgtgcgagtacgccgacgagacagctaccatcgtggaatttctgaaccggtggatcaccttcagccagtccatcatcagcaccctgacc

SEQ ID NO: 209 - DNA, 1128 bp, Artificial Sequence
  source: /note="Description of Artificial Sequence: Synthetic polynucleotide"
gagtctaagtacggccctccttgtcctccatgtcctgctccagaagctgctggcggcccttccgtgtttctgttccctccaaagcctaaggacaccctgatgatctctcggacccctgaagtgacctgcgtggtggtggatgtgtcccaagaggatcccgaggtgcagttcaattggtacgtggacggcgtggaagtgcacaacgccaagaccaagcctagagaggaacagttcaactccacctacagagtggtgtccgtgctgaccgtgctgcaccaggattggctgaacggcaaagagtacaagtgcaaggtgtccaacaagggcctgccttccagcatcgaaaagaccatctccaaggccaagggccagcctagggaaccccaggtttacaccctgcctccaagccaagaggaaatgaccaagaaccaggtgtccctgtggtgcctggtcaagggcttctacccttccgatatcgccgtggaatgggagagcaatggccagcctgagaacaactacaagaccacacctcctgtgctggactccgacggctccttctttctgtactcccgcctgaccgtggacaagtccagatggcaagagggcaacgtgttctcctgctccgtgatgcacgaggccctgcacaatcactacacccagaagtccctgtctctgtctcttggcggaggcggaggaagtggtggcggaggttctggtggcggtggatcaggcggtggcggaagctctacaaagaaaacccagctgcaactggaacatctgctgctggacctgcagatgatcctgaacggcatcaacaactacaagaaccccaagctgaccggcatgctgaccgccaagttctacatgcccaagaaggccaccgagctgaaacatctgcagtgcctggaagaggccctgaagcctctggaagaagtgctgaatctggcccagtccaagaacttccacctgaggcctcgggacctgatctccaacatcaacgtgatcgtgctggaactgaagggctccgagacaaccttcatgtgcgagtacgccgacgagacagctaccatcgtggaatttctgaaccggtggatcaccttcagccagtccatcatcagcaccctgacc

SEQ ID NO: 210 - DNA, 1128 bp, Artificial Sequence
  source: /note="Description of Artificial Sequence: Synthetic polynucleotide"
gagtctaagtacggccctccttgtcctccatgtcctgctccagaagctgctggcggcccttccgtgtttctgttccctccaaagcctaaggacaccctgatgatctctcggacccctgaagtgacctgcgtggtggtggatgtgtcccaagaggatcccgaggtgcagttcaattggtacgtggacggcgtggaagtgcacaacgccaagaccaagcctagagaggaacagttcaactccacctacagagtggtgtccgtgctgaccgtgctgcaccaggattggctgaacggcaaagagtacaagtgcaaggtgtccaacaagggcctgccttccagcatcgaaaagaccatctccaaggccaagggccagcctagggaaccccaggtttacaccctgcctccaagccaagaggaaatgaccaagaaccaggtgtccctgtggtgcctggtcaagggcttctacccttccgatatcgccgtggaatgggagagcaatggccagcctgagaacaactacaagaccacacctcctgtgctggactccgacggctccttctttctgtactcccgcctgaccgtggacaagtccagatggcaagagggcaacgtgttctcctgctccgtgatgcacgaggccctgcacaatcactacacccagaagtccctgtctctgtcccttggcggaggcggaggatctggtggtggcggatctggcggcggaggtagcggtggcggtggatcttctaccaagaaaacccagctgcagttggagcatctgctgctggacctgcagatgatcctgaatggcatcaacaattacaagaaccccaagctgaccggcatgctgaccgccaagttctacatgcccaagaaggccaccgagctgaaacatctgcagtgcctggaagaggccctgaagcctctggaagaagtgctgaatctggcccagtccaagaacttccacctgaggcctcgggacctgatctccaacatcaacgtgatcgtgctggaactgaagggctccgagacaaccttcatgtgcgagtacgccgacgagacagctaccatcgtggaatttctgaaccggtggatcaccttcagccagtccatcatcagcaccctgacc

SEQ ID NO: 211 - DNA, 1128 bp, Artificial Sequence
  source: /note="Description of Artificial Sequence: Synthetic polynucleotide"
gagtctaagtacggccctccttgtcctccatgtcctgctccagaagctgctggcggcccttccgtgtttctgttccctccaaagcctaaggacaccctgatgatctctcggacccctgaagtgacctgcgtggtggtggatgtgtcccaagaggatcccgaggtgcagttcaattggtacgtggacggcgtggaagtgcacaacgccaagaccaagcctagagaggaacagttcaactccacctacagagtggtgtccgtgctgaccgtgctgcaccaggattggctgaacggcaaagagtacaagtgcaaggtgtccaacaagggcctgccttccagcatcgaaaagaccatctccaaggccaagggccagcctagggaaccccaggtttacaccctgcctccaagccaagaggaaatgaccaagaaccaggtgtccctgtggtgcctggtcaagggcttctacccttccgatatcgccgtggaatgggagagcaatggccagcctgagaacaactacaagaccacacctcctgtgctggactccgacggctccttctttctgtactcccgcctgaccgtggacaagtccagatggcaagagggcaacgtgttctcctgctccgtgatgcacgaggccctgcacaatcactacacccagaagtccctgtctctgtctcttggcggaggcggaggaagtggtggcggaggttctggtggcggtggatcaggcggtggcggaagctctacaaagaaaacccagctgcaactggaacatctgctgctggacctgcagatgatcctgaacggcatcaacaactacaagaaccccaagctgacccggatgctgaccgccaagttctacatgcccaagaaggccaccgagctgaagcaccttcagtgtctggaagccgctctgaagcccctggaagaggtgctgaatctggcccagagcaagaacttccacctgaggcctagggacctgatcagcaacatcaacgtgatcgtgctggaactgaagggcagcgagacaaccttcatgtgcgagtacgccgacgagacagccaccatcgtggaatttctgaacagatggatcaccttcagccagagcatcatcagcaccctgacc

SEQ ID NO: 212 - DNA, 1128 bp, Artificial Sequence
  source: /note="Description of Artificial Sequence: Synthetic polynucleotide"
gagtctaagtacggccctccttgtcctccatgtcctgctccagaagctgctggcggcccttccgtgtttctgttccctccaaagcctaaggacaccctgatgatctctcggacccctgaagtgacctgcgtggtggtggatgtgtcccaagaggatcccgaggtgcagttcaattggtacgtggacggcgtggaagtgcacaacgccaagaccaagcctagagaggaacagttcaactccacctacagagtggtgtccgtgctgaccgtgctgcaccaggattggctgaacggcaaagagtacaagtgcaaggtgtccaacaagggcctgccttccagcatcgaaaagaccatctccaaggccaagggccagcctagggaaccccaggtttacaccctgcctccaagccaagaggaaatgaccaagaaccaggtgtccctgtggtgcctggtcaagggcttctacccttccgatatcgccgtggaatgggagagcaatggccagcctgagaacaactacaagaccacacctcctgtgctggactccgacggctccttctttctgtactcccgcctgaccgtggacaagtccagatggcaagagggcaacgtgttctcctgctccgtgatgcacgaggccctgcacaatcactacacccagaagtccctgtctctgtctcttggcggaggcggaggaagtggtggcggaggttctggtggcggtggatcaggcggtggcggaagctctacaaagaaaacccagctgcaactggaacatctgctgctggacctgcagatgatcctgaacggcatcaacaactacaagaaccccaagctgaccggcatgctgaccttcaagttctacatgcccaagaaggccaccgagctgaagcaccttcagtgtctggaagccgctctgaagcccctggaagaggtgctgaatctggcccagagcaagaacttccacctgaggcctagggacctgatcagcaacatcaacgtgatcgtgctggaactgaagggcagcgagacaaccttcatgtgcgagtacgccgacgagacagccaccatcgtggaatttctgaacagatggatcaccttcagccagagcatcatcagcaccctgacc

SEQ ID NO: 213 - DNA, 1128 bp, Artificial Sequence
  source: /note="Description of Artificial Sequence: Synthetic polynucleotide"
gagtctaagtacggccctccttgtcctccatgtcctgctccagaagctgctggcggcccttccgtgtttctgttccctccaaagcctaaggacaccctgatgatctctcggacccctgaagtgacctgcgtggtggtggatgtgtcccaagaggatcccgaggtgcagttcaattggtacgtggacggcgtggaagtgcacaacgccaagaccaagcctagagaggaacagttcaactccacctacagagtggtgtccgtgctgaccgtgctgcaccaggattggctgaacggcaaagagtacaagtgcaaggtgtccaacaagggcctgccttccagcatcgaaaagaccatctccaaggccaagggccagcctagggaaccccaggtttacaccctgcctccaagccaagaggaaatgaccaagaaccaggtgtccctgtggtgcctggtcaagggcttctacccttccgatatcgccgtggaatgggagagcaatggccagcctgagaacaactacaagaccacacctcctgtgctggactccgacggctccttctttctgtactcccgcctgaccgtggacaagtccagatggcaagagggcaacgtgttctcctgctccgtgatgcacgaggccctgcacaatcactacacccagaagtccctgtctctgtcccttggcggaggcggaggatctggtggtggcggatctggcggcggaggtagcggtggcggtggatcttctaccaagaaaacccagctgcagttggagcatctgctgctggacctgcagatgatcctgaatggcatcaacaattacaagaaccccaagctgacccggatgctgaccttcaagttctacatgcccaagaaggccaccgagctgaaacatctgcagtgcctggaagaggaactgaagcccctggaagaagtgctgaatctggcccagtccaagaacttccacctgaggcctcgggacctgatctccaacatcaacgtgatcgtgctcgagctgaagggctccgagacaaccttcatgtgcgagtacgccgacgagacagctaccatcgtggaatttctgaaccggtggatcaccttcagccagtccatcatcagcaccctgacc

SEQ ID NO: 214 - DNA, 687 bp, Artificial Sequence
  source: /note="Description of Artificial Sequence: Synthetic polynucleotide"
gagtctaagtacggccctccttgtcctccatgtcctgctccagaagctgctggcggcccttccgtgtttctgttccctccaaagcctaaggacaccctgatgatcagcagaacccctgaagtgacctgcgtggtggtggacgtgtcccaagaggatcctgaggtgcagttcaattggtacgtggacggcgtggaagtgcacaacgccaagaccaagcctagagaggaacagttcaacagcacctatagagtggtgtccgtgctgaccgtgctgcaccaggattggctgaacggcaaagagtacaagtgcaaggtgtccaacaagggcctgcctagctccatcgagaaaaccatcagcaaggccaagggccagccaagagaaccccaggtgtacacactgcctccaagccaagaggaaatgaccaagaaccaggtgtccctgagctgcgccgtgaagggcttttacccttccgatatcgccgtggaatgggagagcaatggccagcctgagaacaactacaagaccacacctcctgtgctggacagcgacggctcattcttcctggtgtccagactgaccgtggacaagagcagatggcaagagggcaacgtgttcagctgcagcgtgatgcacgaggccctgcacaaccggtttacccagaagtctctgagcctgagcctgggcaaa

SEQ ID NO: 215 - DNA, 687 bp, Artificial Sequence
  source: /note="Description of Artificial Sequence: Synthetic polynucleotide"
gagtctaagtacggccctccttgtcctccatgtcctgctccagaagcagctggcggcccttccgtgtttctgttccctccaaagcctaaggacaccctgatgatctctcggacccctgaagtgacctgcgtggtggtggatgtgtcccaagaggatcccgaggtgcagttcaattggtacgtggacggcgtggaagtgcacaacgccaagaccaagcctagagaggaacagttcaactccacctacagagtggtgtccgtgctgaccgtgctgcaccaggattggctgaacggcaaagagtacaagtgcaaggtgtccaacaagggcctgccttccagcatcgaaaagaccatctccaaggccaagggccagcctagggaaccccaggtttacaccctgcctccaagccaagaggaaatgaccaagaaccaggtgtccctgtcctgcgccgtgaagggcttctacccttctgatatcgccgtggaatgggagagcaacggccagcctgagaacaactacaagaccacacctcctgtgctggactccgacggctctttctttctggtgtcccgcctgaccgtggacaagtctagatggcaagagggcaacgtgttctcctgctccgtgatgcacgaggccctgcacaacagattcacccagaagtccctgtctctgtccctgggcaaa

SEQ ID NO: 216 - protein, 133 aa, Homo sapiens [sequence omitted]

SEQ ID NO: 217 - protein, 134 aa, Macaca mulatta
APTSSSTKKTQLQLEHLLLDLQMILNGINNYKNPKLTRMLTFKFYMPKKATELKHLQCLEEELKPLEEVLNLAQSKNFHLRDTKDLISNINVIVLELKGSETTLMCEYADETATIVEFLNRWITFCQSIISTLT

SEQ ID NO: 218 - protein, 17 aa, Artificial Sequence
  source: /note="Description of Artificial Sequence: Synthetic peptide"
KWVTFISLLFLFSSAYS

SEQ ID NO: 219 - protein, 20 aa, Artificial Sequence
  source: /note="Description of Artificial Sequence: Synthetic peptide"
MYRMQLLSCIALSLALVTNS

SEQ ID NO: 220 - protein, 21 aa, Artificial Sequence
  source: /note="Description of Artificial Sequence: Synthetic peptide"
MPAIAVLAAAAAAWCFLQVES

SEQ ID NO: 221 - protein, 22 aa, Artificial Sequence
  source: /note="Description of Artificial Sequence: Synthetic peptide"
MRAPGCGRLVLPLLLLAAAALA

SEQ ID NO: 222 - protein, 22 aa, Artificial Sequence
  source: /note="Description of Artificial Sequence: Synthetic peptide"
MDMRVPAQLLGLLLLWLSGARC

SEQ ID NO: 223 - protein, 18 aa, Artificial Sequence
  source: /note="Description of Artificial Sequence: Synthetic peptide"
MWLQSLLLLGTVACSISV

SEQ ID NO: 224 - protein, 23 aa, Artificial Sequence
  source: /note="Description of Artificial Sequence: Synthetic peptide"
MDAMKRGLCCVLLLCGAVFVSAR

SEQ ID NO: 225 - protein, 16 aa, Artificial Sequence
  source: /note="Description of Artificial Sequence: Synthetic peptide"
MHRRRSRSCREDQKPV

SEQ ID NO: 226 - protein, 31 aa, Artificial Sequence
  source: /note="Description of Artificial Sequence: Synthetic polypeptide"
MRKAAVSHWQQQSYLDSGIHSGATTTAPSLS

SEQ ID NO: 227 - protein, 23 aa, Artificial Sequence
  source: /note="Description of Artificial Sequence: Synthetic peptide"
MKASAALLCLLLTAAAFSPQGLA

SEQ ID NO: 228 - protein, 76 aa, Artificial Sequence [sequence omitted]

SEQ ID NO: 229 - protein, 17 aa, Artificial Sequence
  source: /note="Description of Artificial Sequence: Synthetic peptide"
MLLSVPLLLGLLGLAVA

SEQ ID NO: 230 - protein, 16 aa, Artificial Sequence
  source: /note="Description of Artificial Sequence: Synthetic peptide"
MKCLLYLAFLFIGVNC

SEQ ID NO: 231 - protein, 21 aa, Artificial Sequence
  source: /note="Description of Artificial Sequence: Synthetic peptide"
MNQTAILICCLIFLTLSGIQG

SEQ ID NO: 232 - protein, 5 aa, Artificial Sequence
  source: /note="Description of Artificial Sequence: Synthetic peptide"
EPKSC

SEQ ID NO: 233 - protein, 227 aa, Artificial Sequence
  source: /note="Description of Artificial Sequence: Synthetic polypeptide"
DKTHTCPPCPAPELLGGPSVFLFPPKPKDTLMISRTPEVTCVVVDVSHEDPEVKFNWYVDGVEVHNAKTKPREEQYNSTYRVVSVLTVLHQDWLNGKEYKCKVSNKALPAPIEKTISKAKGQPREPQVYTLPPSREEMTKNQVSLTCLVKGFYPSDIAVEWESNGQPENNYKTTPPVLDSDGSFFLYSKLTVDKSRWQQGNVFSCSVMHEALHNHYTQKSLSLSPGK

SEQ ID NO: 234 - protein, 149 aa, Mus musculus
APTSSSTSSSTAEAQQQQQQQQQQQQHLEQLLMDLQELLSRMENYRNLKLPRMLTFKFYLPKQATELKDLQCLEDELGPLRHVLDLTQSKSFQLEDAENFISNIRVTVVKLKGSDNTFECQFDDESATVVDFLRRWIAFCQSIISTSPQ

SEQ ID NO: 235 - protein, 23 aa, Mus musculus
APTSSSTSSSTAEAQQQQQQQQQ

SEQ ID NO: 236 - protein, 12 aa, Artificial Sequence
  source: /note="Description of Artificial Sequence: Synthetic peptide"
ESKYGPPCPPCP

SEQ ID NO: 237 - protein, 15 aa, Artificial Sequence
  source: /note="Description of Artificial Sequence: Synthetic peptide"
EPKSCDKTHTCPPCP

SEQ ID NO: 238 - protein, 20 aa, Artificial Sequence
  source: /note="Description of Artificial Sequence: Synthetic peptide"
EPKSCDKTHTCPPCPAPELL

SEQ ID NO: 239 - protein, 212 aa, Artificial Sequence
  source: /note="Description of Artificial Sequence: Synthetic polypeptide"
GGPSVFLFPPKPKDTLMISRTPEVTCVVVDVSHEDPEVKFNWYVDGVEVHNAKTKPREEQYNSTYRVVSVLTVLHQDWLNGKEYKCKVSNKALPAPIEKTISKAKGQPREPQVYTLPPSREEMTKNQVSLTCLVKGFYPSDIAVEWESNGQPENNYKTTPPVLDSDGSFFLYSKLTVDKSRWQQGNVFSCSVMHEALHNHYTQKSLSLSPGK

SEQ ID NO: 240 - protein, 212 aa, Artificial Sequence
  source: /note="Description of Artificial Sequence: Synthetic polypeptide"
GGPSVFLFPPKPKDTLYITREPEVTCVVVDVSHEDPEVKFNWYVDGVEVHNAKTKPREEQYNSTYRVVSVLTVLHQDWLNGKEYKCKVSNKALPAPIEKTISKAKGQPREPQVYTLPPSREEMTKNQVSLTCLVKGFYPSDIAVEWESNGQPENNYKTTPPVLDSDGSFFLYSKLTVDKSRWQQGNVFSCSVMHEALHNHYTQKSLSLSPGK

SEQ ID NO: 241 - protein, 229 aa, Artificial Sequence
  source: /note="Description of Artificial Sequence: Synthetic polypeptide"
ESKYGPPCPPCPAPEFEGGPSVFLFPPKPKDTLMISRTPEVTCVVVDVSQEDPEVQFNWYVDGVEVHNAKTKPREEQFNSTYRVVSVLTVLHQDWLNGKEYKCKVSNKGLPSSIEKTISKAKGQPREPQVYTLPPSQEEMTKNQVSLTCLVKGFYPSDIAVEWESNGQPENNYKTTPPVLDSDGSFFLYSRLTVDKSRWQEGNVFSCSVMHEALHNHYTQKSLSLSLGK

SEQ ID NO: 242 - protein, 229 aa, Artificial Sequence
  source: /note="Description of Artificial Sequence: Synthetic polypeptide"
ESKYGPPCPPCPAPEAAGGPSVFLFPPKPKDTLMISRTPEVTCVVVDVSQEDPEVQFNWYVDGVEVHNAKTKPREEQFNSTYRVVSVLTVLHQDWLNGKEYKCKVSNKGLPSSIEKTISKAKGQPREPQVYTLPPSQEEMTKNQVSLTCLVKGFYPSDIAVEWESNGQPENNYKTTPPVLDSDGSFFLYSRLTVDKSRWQEGNVFSCSVMHEALHNHYTQKSLSLSLGK

SEQ ID NO: 243 - protein, 229 aa, Artificial Sequence
  source: /note="Description of Artificial Sequence: Synthetic polypeptide"
ESKYGPPCPPCPAPEFEGGPSVFLFPPKPKDTLYITREPEVTCVVVDVSQEDPEVQFNWYVDGVEVHNAKTKPREEQFNSTYRVVSVLTVLHQDWLNGKEYKCKVSNKGLPSSIEKTISKAKGQPREPQVYTLPPSQEEMTKNQVSLTCLVKGFYPSDIAVEWESNGQPENNYKTTPPVLDSDGSFFLYSRLTVDKSRWQEGNVFSCSVMHEALHNHYTQKSLSLSLGK

SEQ ID NO: 244 - protein, 20 aa, Artificial Sequence
  source: /note="Description of Artificial Sequence: Synthetic peptide"
  SITE (1)..(20): /note="This sequence may encompass 3-5 'Gly Gly Gly Ser'" repeating units
GGGSGGGSGGGSGGGSGGGS

SEQ ID NO: 245 - protein, 25 aa, Artificial Sequence
  source: /note="Description of Artificial Sequence: Synthetic peptide"
  SITE (1)..(25): /note=" This sequence may encompass 3-5 'Gly Gly Gly Gly Ser'" repeating units
GGGGSGGGGSGGGGSGGGGSGGGGS

SEQ ID NO: 246 - protein, 20 aa, Artificial Sequence
  source: /note="Description of Artificial Sequence: Synthetic peptide"
GGGGSGGGGSGGGGSGGGGS

SEQ ID NO: 247 - protein, 8 aa, Homo sapiens
KPSSPPEE

SEQ ID NO: 248 - protein, 15 aa, Artificial Sequence
  source: /note="Description of Artificial Sequence: Synthetic peptide"
RRCPLYISYDPVCRR

SEQ ID NO: 249 - protein, 19 aa, Artificial Sequence
  source: /note="Description of Artificial Sequence: Synthetic peptide"
RRRRCPLYISYDPVCRRRR

SEQ ID NO: 250 - protein, 230 aa, Artificial Sequence; identical to SEQ ID NO: 173
  source: /note="Description of Artificial Sequence: Synthetic polypeptide"

SEQ ID NO: 251 - protein, 99 aa, Artificial Sequence
  source: /note="Description of Artificial Sequence: Synthetic polypeptide"
KKVVYGKKGDTVELTCTASQKKNIQFHWKNSNQIKILGNQGSFLTKGPSKLNDRVDSRRSLWDQGNFPLIIKNLKPEDSDTYICEVEDQKEEVQLVVVG

SEQ ID NO: 252 - protein, 203 aa, Artificial Sequence
  source: /note="Description of Artificial Sequence: Synthetic polypeptide"
KKVVYGKKGDTVELTCTASQKKNIQFHWKNSNQIKILGNQGSFLTKGPSKLNDRVDSRRSLWDQGNFPLIIKNLKPEDSDTYICEVEDQKEEVQLVVVGGGGSGKKVVYGKKGDTVELTCTASQKKNIQFHWKNSNQIKILGNQGSFLTKGPSKLNDRVDSRRSLWDQGNFPLIIKNLKPEDSDTYICEVEDQKEEVQLVVVG

SEQ ID NO: 253 - protein, 99 aa, Artificial Sequence
  source: /note="Description of Artificial Sequence: Synthetic polypeptide"
KKVVLGKKGDTVELTCTASQKKSIQFHWKNSNQIKILGNQGSFLTKGPSKLNDRADSRRSLWDQGNFPLIIKNLKIEDSDTYICEVEDQKEEVQLLVFG

SEQ ID NO: 254 - protein, 203 aa, Artificial Sequence
  source: /note="Description of Artificial Sequence: Synthetic polypeptide"
KKVVLGKKGDTVELTCTASQKKSIQFHWKNSNQIKILGNQGSFLTKGPSKLNDRADSRRSLWDQGNFPLIIKNLKIEDSDTYICEVEDQKEEVQLLVFGGGGSGKKVVLGKKGDTVELTCTASQKKSIQFHWKNSNQIKILGNQGSFLTKGPSKLNDRADSRRSLWDQGNFPLIIKNLKIEDSDTYICEVEDQKEEVQLLVFG

SEQ ID NO: 255 - protein, 456 aa, Artificial Sequence
  source: /note="Description of Artificial Sequence: Synthetic polypeptide"
AVNGTSQFTCFYNSRANISCVWSQDGALQDTSCQVHAWPDRRRWNQTCELLPVSQASWACNLILGAPDSQKLTTVDIVTLRVLCREGVRWRVMAIQDFKPFENLRLMAPISLQVVHVETHRCNISWEISQASHYFERHLEFEARTLSPGHTWEEAPLLTLKQKQEWICLETLTPDTQYEFQVRVKPLQGEFTTWSPWSQPLAFRTKPAALGKDTGAQDKTHTCPPCPAPELLGGPSVFLFPPKPKDTLMISRTPEVTCVVVDVSHEDPEVKFNWYVDGVEVHNAKTKPREEQYNSTYRVVSVLTVLHQDWLNGKEYKCKVSNKALPAPIEKTISKAKGQPREPQVYTLPPSRDELTKNQVSLSCAVKGFYPSDIAVEWESNGQPENNYKTTPPVLDSDGSFFLVSKLTVDKSRWQQGNVFSCSVMHEALHNRFTQKSLSLSPGKGSGSDYKDDDDK

SEQ ID NO: 256 - protein, 497 aa, Artificial Sequence
  source: /note="Description of Artificial Sequence: Synthetic polypeptide"
LNTTILTPNGNEDTTADFFLTTMPTDSLSVSTLPLPEVQCFVFNVEYMNCTWNSSSEPQPTNLTLHYWYKNSDNDKVQKCSHYLFSEEITSGCQLQKKEIHLYQTFVVQLQDPREPRRQATQMLKLQNLVIPWAPENLTLHKLSESQLELNWNNRFLNHCLEHLVQYRTDWDHSWTEQSVDYRHKFSLPSVDGQKRYTFRVRSRFNPLCGSAQHWSEWSHPIHWGSNTSKENPFLFALEAGAQDKTHTCPPCPAPELLGGPSVFLFPPKPKDTLMISRTPEVTCVVVDVSHEDPEVKFNWYVDGVEVHNAKTKPREEQYNSTYRVVSVLTVLHQDWLNGKEYKCKVSNKALPAPIEKTISKAKGQPREPQVYTLPPSRDELTKNQVSLWCLVKGFYPSDIAVEWESNGQPENNYKTTPPVLDSDGSFFLYSKLTVDKSRWQQGNVFSCSVMHEALHNHYTQKSLSLSPGKGSGSGLNDIFEAQKIEWHEHHHHHHHH

SEQ ID NO: 257 - protein, 8 aa, Artificial Sequence
  source: /note="Description of Artificial Sequence: Synthetic peptide"
DYKDDDDK

SEQ ID NO: 258 - protein, 8 aa, Artificial Sequence
  source: /note="Description of Artificial Sequence: Synthetic 8xHis tag"
HHHHHHHH

SEQ ID NO: 259 - protein, 15 aa, Artificial Sequence
  source: /note="Description of Artificial Sequence: Synthetic peptide"
GLNDIFEAQKIEWHE

SEQ ID NO: 260 - protein, 229 aa, Artificial Sequence; identical to SEQ ID NO: 48
  source: /note="Description of Artificial Sequence: Synthetic polypeptide"

SEQ ID NO: 261 - protein, 229 aa, Artificial Sequence; identical to SEQ ID NO: 46
  source: /note="Description of Artificial Sequence: Synthetic polypeptide"

SEQ ID NO: 262 - protein, 134 aa, Macaca fascicularis
APTSSSTKKTQLQLEHLLLDLQMILNGINNYKNPKLTRMLTFKFYMPKKATELRHLQCLEEELKPLEEVLNLAQSKSFHLRDTKDLISNINVIVLELKGSETTLMCEYADETATIVEFLNRWITFCQSIISTLT

SEQ ID NO: 263 - protein, 9 aa, Artificial Sequence
  source: /note="Description of Artificial Sequence: Synthetic peptide"
KLLEIAPNC

SEQ ID NO: 264 - protein, 5 aa, Artificial Sequence
  source: /note="Description of Artificial Sequence: Synthetic peptide"
GGGGS

SEQ ID NO: 265 - protein, 4 aa, Artificial Sequence
  source: /note="Description of Artificial Sequence: Synthetic peptide"
GGGS